European Patent Specification EP 3 599 829 B1, published October 4, 2023. Title: METHODS FOR IMPROVING TRAITS IN PLANTS. Applicant: PlantArcBio Ltd. The sequence listing filed with the application follows.

SEQUENCE LISTING (333 sequences)

SEQ ID NO: 1 - DNA, 1019 bp, metagenomes purified from environmentally challenged niches
ggactttctcattttcagaattattttctatactctgacaagagcaagcaataccaaacatcttccacatcgaagctttaaccattttgcccttaacatttgaacaagacgaaatggccttcttcccacactacaccactaatctgtcgcctctgctctacttgttggacgacgactatgctgtctaccgctcaacttgtccaaagtccaactaccaccacaagcaacaccacagccgccgtcagccttcgccagttcgttactttagtccgaattttgatatgcgagaggggaatgactcctactaccttgacggagagctccctggtgtcaaccagaatgatgtcgatattgaattctctgaccctcagacactggtgatcaagggtcgagtggagcggaattacaacaatctcgacggcatgaacgaggaaaaccagcaagatgaagaacaattctctgaaactctctctagcaagtcgtaccaacccactgtcgaggacgaggacgaggcgaaccattcaccacccgtggcgacaccaacctactctgagaagtctgttactgagaaaactcagaagcctgcgtacaaataccgaaattctgaacgtgctattggcgaattccaccgagccttcaatctccctacaagagtcgatcaagatgcggtcagggctacattgaggaatggaatcctctcgctggagctcccgaaggagccggcaccgaagatgaagaagattcggattgaatagaggatttcgaataaaatttttgatttgatgagtagttggtgtttattgttatgtctaattatatggggctatgtcatgattgggaaatgggacaccgcatttgtttcctttttccccatttcttcagacgccatctatattacatgtatgttgcatgaactatggtttttgctaggagcggttgcttctgctctgcattttcatgaactattttctttttattaaattaataactagcatatcaattaatgatctgtcatatgg

SEQ ID NO: 2 - DNA, 712 bp, metagenomes purified from environmentally challenged niches
gatcatcaatcaattaatcaatctactctactttccaaaacataactaccaaataaccagaatgcagctcctcagcaccctcaccccccttgccctcctagtcaccgtcgcttccgccaccggcaaagccgtcaataatgccgttggcaacgccgtcgtcacaaaccactgtaaagacccaatctatctctggtccgtcggctcctccgtctccccgaaacacaccatcccctccggctccaactataccgagcccttccgccacgacgacgcatctggcggcatcgcgctgaagatcacccgtaacgacaacgggctgtatgacgggagtgcgcagttagtttactcctacgctttggatggggaacaggtgtggtatgatttgtcgagtgtgtttggggatgcgtttgcaggggaggctgttgctgtgaagccggagaatgaggggtgtgggagtatttgttggcctaagggtaccacgcctggtggaagccaggttaaggtctgtgatgcggagggggatgttggattggttgtttgtgcgaaggggtgttagggggtctgagtgaaggttggtggtggtaatgagcaattgggtatgagaggggaaaggatatgttaatcgtttatgttatttacttgatcaaaatatttgtattgacgtcggttgttttgttattgttgttttaaatgcaaatgtatatgaactttc

SEQ ID NO: 3 - DNA, 580 bp, metagenomes purified from environmentally challenged niches
ggttcgtcaacgcgacgatccgcgggggtccaagctaggacgtggcagttgtgacacaacaagagcatgctatggcaaatgccattcgcgagctcgccactaccctgtgaactgtggccttactcctatacccgccagagtctgacttattcctgtcactggaatctggcttactgctggtgctggagtctggtcccagtattttagtatagtacaattgctagctgaagccataaggcgtggattgttggggtggcgcagggctgaagccaaatggcagcggtgttgctgctggttgagcaccgggcatagcgccagaaagtgcacccgcgaacattccctggtattgcatgaacggctgtccaggaatcgcgccaggcattggcaaggcgttgttgcgctttgcctccgctgccagcagcctctctgcttccgtaccgtgtctttcgcccttaccgtccttcttgaatgcataatcaaccgtcagaggcttgttcatcaagtactggccattcatagccgtgattgcctggtccgagctgtcaaagtcgttgtactggatgaatccatatcctttcaa

SEQ ID NO: 4 - DNA, 580 bp, metagenomes purified from environmentally challenged niches
ttgaaaggatatggattcatccagtacaacgactttgacagctcggaccaggcaatcacggctatgaatggccagtacttgatgaacaagcctctgacggttgattatgcattcaagaaggacggtaagggcgaaagacacggtacggaagcagagaggctgctggcagcggaggcaaagcgcaacaacgccttgccaatgcctggcgcgattcctggacagccgttcatgcaataccagggaatgttcgcgggtgcactttctggcgctatgcccggtgctcaaccagcagcaacaccgctgccatttggcttcagccctgcgccaccccaacaatccacgccttatggcttcagctagcaattgtactatactaaaatactgggaccagactccagcaccagcagtaagccagattccagtgacaggaataagtcagactctggcgggtataggagtaaggccacagttcacagggtagtggcgagctcgcgaatggcatttgccatagcatgctcttgttgtgtcacaactgccacgtcctagcttggacccccgcggatcgtcgcgttgacgaacc

SEQ ID NO: 5 - DNA, 781 bp, metagenomes purified from environmentally challenged niches
gaaaaaaactttagaatacagtttaatcaatcttcacagctacaaggctatatcatttgatatagcatatcaaagtggctttgatttctgtaaatttatatctaataataatagtgtttatatcagctaaatacatatttctatcctatctatatatcaccgacagaccatatttgaaactgctgttgacactattattcatatgttcggatttaattttaatacgacaaaattgttaaaaacaattctcgttgtttgttatttgcaggcaacagtgttagctgatccttatacaagagtatcttgggaagcgtatatgaatcatgtcaatggatccgacgactatcgtactcaaggggatgataccagagctacacgctttccagagactaaacctccaaaacaaggaaaagatttcctgtggtcgagtaaaccagtccccagttcagatctatttctggagttctttatgtatgagggagaaccagatgaattcagcaggacgactgaatcgtatcaatcacttccgagcaacgcgttaactgctaggcaaaatgcccttacttgtcaggacatagagtcatgttcgtatcctccacaggtgaacaactttcaagctttattcgacgacctggggccatcaacttgtaatctcataaaagacgaaactcgtgactggatattgcagcagtggcccgggttagctgtaggagccgttatatcgtttgcggtagccgttgcgggaagctcctgtgatatattatattaatcagctttggca

SEQ ID NO: 6 - DNA, 661 bp, metagenomes purified from environmentally challenged niches
ggtcgagctactttcaaggtcaagcaagatggtccgttacgcacacaatgctgagaacccagagaagaccgccaaggctcgtggtcagcacttgcgtacgcacttcaagaacacccgtgaagtcgctgctgctctgaccggcttgaagctttcaaaggcttacaagtacctcggcgatgtccaagagcacaaggatgtcatcccattccgtcgcttcaacggtggtgttggcagagccgctcaggctaagaaccacggtacgacccaaggtcgttggccagtcaagtcgattggcttcttgctcagacttttgaagaacgctgaggccaacgctgacgccaagtcactcgacacggaagacctcttgatcaagcacattgttgtccaacaagctccaaaaacccgtcgtcgtacttaccgtgctcacggtcgtatcaacccttaccaaggacacccatgccacattgagatcactctggctgtcccagacgagcaagtcgctcgcaacaaggacgttgaggtgaaccaaccaaagaagatccaaggcaacaagcgtcaagtcgctgctcaacgtcgcttgacctctgcataaactggctactcggttgtgtaccactctatacaaattattcagtaaaatgctatccatcttggcttcgaa

SEQ ID NO: 7 - DNA, 713 bp, metagenomes purified from environmentally challenged niches
agccacaaccacatcaatcctccaccactttcagctttcgacttcatcaaacaactccttctaccactactacctcaacaaccttcatcaaaatgactggacgcggcaagggcggcaagggtctcggaaagggcggcgccaagcgtcaccgcaagatcttgcgcgacaacatccagggcatcaccaagcccgccatccgccgtctggcgcgtcgtggcggtgtcaagcgtatctccgccatgatctacgaggagacccgcggtgtcctcaagaccttcctcgagggtgtcatccgcgacgccgtcacctacaccgagcacgccaagcgcaagaccgtcacctccctcgacgtcgtctacgccctcaagaggcaaggccgcaccctctacggtttcggtggttaagcagctcgctcttctctcttcgactgctttgctttcttcaaacacaataacaatcacgacaacaacaacttcatcagatatccacccacaatgcgagagttgggcttgcgggtatggcgcgaatgggcaatgggctatccgggttttttcatttttggggtttttttctcttttcctgtttcgatgctgcgaggtgagcacactgggctgcggctcatgaggctttgagtgtagaataggctcaacatcatcaaagaagcattccacgagacgtggcgctttcttcatcaaccaaatgaatattgcagc

SEQ ID NO: 8 - DNA, 1021 bp, metagenomes purified from environmentally challenged niches
ggacttgcgaccacacacatctttatacctcaaaatgtcgctcgatgtcggagatgtagacgcctggatcgacacgctatcgcagtgcaagcagctatctgaatctgacgtgaagctcctctgcgacaaggccagagaaattcttatagaggagtccaacgtacagccagtcagatgccccgtcaccgtctgcggcgatattcacggtcaattccacgacttgattgagctctttagaataggcggcaactccccatccaccaattacctcttcatgggcgattacgtagacagggggtactactcggtcgaaactgtcaccctcctcgtcgccttgaagctccgctacagggaaagaatcaccatcttgcgcggtaaccacgagtcgagacagatcacccaggtctacggtttctacgacgagtgcttgagaaagtatggaaacgccaacgtctggaagttcttcaccgatctctttgactacctcccactgacggcgcttattgacaatcaaatcttctgtcttcacggtggtttgtctccttccatcgacacgctcgaccacatccgctctatcgaccgtatccaagaggtgcctcacgaaggtcctatgtgcgatctcctctggtccgatccagacgaccgctgcggctggggcatatcccctcgtggtgccggttacaccttcggtcaggacatttcagaggctttcaaccactcaaacggcttgacgctcgtagcccgtgctcaccaacttgtcatggaaggttacaactggtcccaggacaggaatgtcgtcactctcttctctgcgccaaattactgctacagatgcggtaaccaagctgcgatcatggagattgacgagaatctcaagtacactttcctccaattcgatccagcaccaagagctggcgaaccgatggtgtctcgaagagttccggactacttcttataggctcttactcactgtatttatgtttgcactgggtattgtttacttgtacaatgtgtaactacg

SEQ ID NO: 9 - DNA, 715 bp, metagenomes purified from environmentally challenged niches
ggagccacaaccacatcaatcctccaccactttcagctttcgacttcatcaaacaactccttctaccactactacctcaacaaccttcatcaaaatgactggacgcggcaagggcggcaagggtctcggaaagggcggcgccaagcgtcaccgcaagatcttgcgcgacaacatccagggcatcaccaagcccgccatccgccgtctggcgcgtcgtggcggtgtcaagcgtatctccgccatgatctacgaggagacccgcggtgtcctcaagaccttcctcgagggtgtcatccgcgacgccgtcacctacaccgagcacgccaagcgcaagaccgtcacctccctcgacgtcgtctacgccctcaagaggcaaggccgcaccctctacggtttcggtggttaagcagctcgctcttctctcttcgactgctttgctttcttcaaacacaataacaatcacgacaacaacaacttcatcagatatccacccacaatgcgagagttgggcttgcgggtatggcgcgaatgggcaatgggctatccgggttttttcatttttggggtttttttctcttttcctgtttcgatgctgcgaggtgagcacactgggctgcggctcatgaggctttgagtgtagaataggctcaacatcatcaaagaagcattccacgagacgtggcgctttcttcatcaaccaaatgaatattgcagc

SEQ ID NO: 10 - DNA, 503 bp, metagenomes purified from environmentally challenged niches
aatcacccaaatgttctctaaactcatcgccatcgcctctcttgccctcgctgccaacgctgcagtcatcgacccaagtgaccacactgtccaatacgaagctgcaccaggaaaggttgtgactgagcactacgaggttctcagccacgccgaagcatcgcgcataatcgaagccaatccacacatcagcgactatcgctacagatgcaactaccaatgcaacgatagcagcggcaactacatgagaaacctgcagcagggagttccaaaccaagcatgcatcttctctagctgctacgactgtgactggaaattccaaaactgtagctactgtcgcttgtcgactggccacaactaccgtgatatcggtggactcgagagctggtgctacaacaacggcggtactacagtgacgcacaactgtggttatactgatggcgaccaatgctaagagcggccttgtaaagtaaaacttgtactctgaatttgcctttatctttccc

SEQ ID NO: 11 - DNA, 580 bp, metagenomes purified from environmentally challenged niches
atcatctcaaacccaattatcttgaacacctagtttctcaagaacatcctcaaaatgcacttcaaatctctctttattgctggcgccctcttcatggtcggtgccagtgccgttgattgtgccactcctgagattcactgcgagactagtgatggcagcccctggtacgacgatgccgtccaagccactgaatactggaaagaaatccaggacgccggcaaagacagctgcggtgatgctggttgcgcacagccccatggctctggatgccacagcgacggtggtagctatggtaccgccgagatcgttctctgccaggatgactcgtcctcttcaactccccaatgtgccgactgccggtgtgtctacagctacctgaagcctcttctcgaccaatgcaagggtgccaacaacaagattggtggatatgctcatgttgacatgggaggcaactacatcaactatgaatttgttaagaaatgagcggatctcacgtgtgtgagaccatcatatagggttttgaagtctgtttcctttgtatttaacgtcgaaagacaattatgagccaggtttatactcc

SEQ ID NO: 12 - DNA, 607 bp, metagenomes purified from environmentally challenged niches
cgcgccgggggaaattggaccatgatagacgacctcaccactggctcagaggacagcttctccaacagctggatatcgtggttcttatctaccaaagggaacgagtacttctgtgaggtggatgaggagtacatactggacagattcaacctcactggcctcaacaacgacgtgcagaactactcgcaggcgctggagctcatcacagacagcctcgacgacgaggacctcgatgatgagcagagagacgctatcgagaacagtgccaggtatctctatggcttgatccacgccagatacatcattacctcccgcggactggcaaagatgctcttcttggtgtacccgcagcagctgccgtcaaagacgacgaactcagtgccgagcacgaagccggcaacttcagcagacgcagcggtcggggtggacaggtacctgcccaagatattcgggttcccggtgcacgagatgtccaagcacgcgaggtggcaggaggcgcagagggatctgcagatttcgaggctgcagcaaagtgcgagtgacccgtcgtacgtgtagagcgttcaaacatgtattactattggtataataatttaactttactgcc

SEQ ID NO: 13 - DNA, 1406 bp, metagenomes purified from environmentally challenged niches
aagttacccggcttattagtcctagattccgagatgtcgctcactcccgaacaaaccgaaatcatcaaggccaccgtgcctgtcgttaaagaacatggcaagaccatcaccaccgttttctacaagaacatgctcgaagcgcatcctgagctgaacgccattttcaacactaccaatcaggtcaatggtcaccagcccaacgcactcgccggagccctcttcgcctacgcctccaacattgacaaccttggcgccttgggccctgccgtcgaactcatctgcaacaagcatgcttcgctgtatatccaacctgagcactacggcatcgtcggcaagttccttctcgaagcgatgggacaggttttgggtgacgccttgactccgcagatcctcgacgcctgggcagctgcctactggcagctcgccaacctctttattggtcgcgaaagtgctatctacaagcagagtgagggatggacacagtggcgcgagttccgggttgcacagaaggtccctgagtccgcggagatcacatcgttctacctcaagcctgtcgacgagaagcctttgccccgcttccgccccggacagtacatttccgtccaagtgcacgttcctcagcttgaatgcccccaagctcgccaatactccctcagcgacaagccccgcgacgattactaccgcatcagcgtgaagaaggagacgggtctcaacacagcaaagccggaggccaaggtcaacccgggttacgtctcgaatattctgcacgagaacgtcaacgagggcgacgtgatcaaggtgtcgcacccttgcggcgatttcttcttgaccgagcaggaaccgtcgcaccctgtcgtcctcatcgcagccggtgtgggtctgacgccacttacctcgatgctcaacacattggactccacccccgcggactctcagcgcaagattcacttcatccacggtgcgcgcaccacttccgtccgcgctttcaaggaccagattaagtctcgcgctgagcgactcccgaatctccaggccaccttcttcaccagctccccgtcggcagatgaaaagcaaggcgtcgactatgacgtccagggccgtatcgatgtgtccaagatggatgccagcaaggatcttttcctcgacaatgcgcagaccgagttctacatttgtggtcccacttccttcatgaatgatatcgcgaacagcttgaaagctcggggggctacctcggagcgtatccacatggaattgttcggcactggcggcgtgcctgtttagatgatggctcagttagccgtgattgggttttatttctttacgacgatatgactcaggtttctaagttagtatacataatcatgataaattcttatatagatatatcaataatacatctcctctcg

SEQ ID NO: 14 - DNA, 750 bp, metagenomes purified from environmentally challenged niches
gggtctcttccatttgaatttttcaacccacagcatggccttcatgaatctcccatggcccactgaatgcctgcatgccgctctcaagaacggatccttacctttctggggatttgtaatctatcgaacgacctacaccgctcagtcagatgccgcctggccgcagattatcgagcttattgcctcctatatgaaagccttactctaccacgagtataacgacaagaaaaaagatggagatgagcctacagtctacgacgaaatctgggcaaggcatcagttgacgattatggatgatagacaattcaacggagcgtctgtgtttgatatccaacttcacttcgaaaagtgggttgaggcgcagggaaagcgagatgaatctactatgtatcgcatgtgtatggtcattgatgatgaatcaatccagacgttattggaggcgccacccggggaaaataggaaactcggacgacgtatagggggccctgtacgctttgtcaaagtcgtggaggctttccccgagctagacagccttgacgaattccagggatggatgaaatgtgagatcaacgcgttatggccgctgtggaagatgatgtctgacggagatgaaatgaggatgtcatatgatgagatgaaggggaatggaaagcaggtctatggcgcaatttaatcggtttttcttcatgttatcctgatggaaaaaatggcagaacatatgtctgtacatgcagaaaataaggtgattgg

SEQ ID NO: 15 - DNA, 811 bp, metagenomes purified from environmentally challenged niches
gacaccacctctttttcgacaaccacaccccgtttcgcaggaagtccatttccagcagtcaaaatggcccgtcgtcccgcgagatgttaccgctactgcaagaacaagccttaccctaagtcccggttcaaccgtggtgttcccgaccccaagatccgtatcttcgacttgggtcgtaagaaggcttccgtggacgacttccccctgtgcgtccacatggtctccaacgaatacgaacagctttcctccgaagctctcgaagctgcccgtatctgtgccaacaagtacctcgtcaagatcgccggtaaggaaggtttccacctgcgtgtccgcgcccaccccttccacgtcgtccgtatcaacaagatgttgtcgtgcgctggtgccgatcgtctccagaccggtatgcgtggtgccttcggtaagcccaacggtgttgtcgcccgtgtgaacatcggccagatcctcctgtccatccgcacccgtgactccaaccgcgccgccgccgttgaggccatgcgccgctccacctacaagttccctggtcgccaaaagatcattatctccaagaactggggcttcacccccgtccgtcgtgaggagtacgtcaagctccgccaggagggcaagctcaagcaggacggtgcctacgtccagttcctgcgtggccacggtttggtcgaggagaacatgaagcgcttcccccaggcctacgagggcgttgctcagtagattgggatgaattaggtggttttatgtgctggtcgtatttatcgtttttactagggccaaatgagaacaaaaaaaggct

SEQ ID NO: 16 - DNA, 923 bp, metagenomes purified from environmentally challenged niches
gtctttagttggccattgaacactgacagatttgcattgcttatatttgcatctacctcacatctactcaactcctcctctccgtttgtcatgtccttctaccagtctcgtccagacactatcaagggtcctgatcctttgaccgacaattggacttatgatagtgccattgatctcttctcttggaatcccatgatgcccgatccttttacctttgacctgcccgacgatcttatgaaatttgaatctaaggatatgtctgctggcatggtcgctccttcggacattagtggttttgccattggtaaccatttgggcgaggatgctgcctcgatatctgatcccgagagtgatgaccacccatggtccccctccgctcatgctgccttcccggagctctctcccatcacatcgacagagcaagtccatcaagaaactgctcgatactcaactacccccgatgccacctcacctcaagaacaaccctcctcaccaccaacacgatctactcgccgccgatcatccgctgacggtcccgttcgcaacgctgccaaacgagcagcccacaacgtcattgaaaagcgctacagaacaaacatgaatgccaaattcgtggcactcgagaaagcaatgaatggcggtaatggcgtgcaaacatcatcaagaggcggagggtccgcgtcgcttaagaaatccgaaatcctctctaatgctattgcctacatgcatggactgcaagaggaaaatcgctatttacaaaaggagcttgctatcgttaaacagaatcttgtaccggcagggatatggcgaggggctcctagttgtaaacgggagacgagttatcgttaacttgttgatttccctgtggttgtttagattttttttacgatgttacgtgtataataatactctcccctcgggtc

SEQ ID NO: 17 - DNA, 1046 bp, metagenomes purified from environmentally challenged niches
ggacaagcccatcttcaattcgagacagtcgccatgggtcgcgttatccgcaaccagaggaagggccgtggctccattttcacggctcacacccgtctgaacaaggctcccgcccagttccgtaccctcgacttcgctgagcgtcacggatacacccgtggtgttgtcaaggagatcatccacgatgccggccgtggtgctcccctcgccaaggtccagttccgccacccctacaagttcaagatggtgaccgagaccttcatcgccaacgagggcatgtacaccggtcagttcatctacgccggtaagaacgctcagctcaccgtcggcaacgttctgcccctcgcctccatgcccgagggtaccgtcatctccaacgttgaggagaagtccggtgaccgtggtgcgcttggccgtacctccggtaactacgttaccgtcattggccacaaccccgaggacggcaagacccgtgtcaagcttccctccggtgccaaaaaggtcatcaagaacaccgcccgtggtatggttggtatcgtcgccggtggtggtcgtaccgacaagcccctgctcaaggcttcccgcgccaagcacaagttcgccgtcaagcgcaactcttggcccaagactcgtggtgttgccatgaaccccgttgatcaccctcacggtggtggtaaccaccagcatatcggtaaggcctctaccatctcccgctacgccgcccagggtcaaaaggccggtctcattgctgcccggagaaccggtctgctccgtggtacccagaagaccaaggattaagcgtgatattacgtggagttttctttgtgacgggttgaaaatggacttctgctatgagacatatgtacttaggcgagtgcggataagcgtcccatgcgcccttagcgaattaaggttgtggtcaccatccttttctttttattaaatcaaaaaagggtgatggaatggggtccgaggctggcctcaagtcaaggcagaacggaaaagtcaaaaatgccccttggggttttggaaatgatacacctttg

SEQ ID NO: 18 - DNA, 780 bp, metagenomes purified from environmentally challenged niches
ggcgcagaggcctattactccccagtatcatcgctaataggcatgtccacgggtctaaggttcagcactttgccagctgcttccaatccacagtcgtcgtcattgatacccagccctagtgctcccatatcaacttttccatatactttaacactcacgctaactcccttgacgggatccctctcaacctcatactcattacgcgcctctcccaatctgtcatttagctctcggttcggtttcaatgtttacagttgggaaagcgagatggtagcgggatttgaactatggcgacaatcgaaaaagcccaagttggccgcgggaagcgatggcgacgatcttgaatgggcccgcaggaaggtccgtgtctgggatccctcagcttttcccctggcaccccctgaacctgaaatcccacaaccaaaccatgaagatgagtctcaagagtcagtacttaagctacgagtcgaccaatcctggaatgttcgtcttctctgggaaggtcgggtgaaggagcttttggtcagcgctggtgtcgggctcggcccgagttccttctcaccatcgtcatatgcaaatcccccgggtacagccggggctcaaggcagcggtgggggctcaccggcctcatactggaggggcgtggggggtttcggtatcatattcttcatgagggatttcttcggatctatgtacttgaatgagcactgtctagatgtatatagtttatcagattttatgagacaatagacaccatgaatctgcgttattgcgagacgg

SEQ ID NO: 19 - DNA, 896 bp, metagenomes purified from environmentally challenged niches
ggccctggcgtgctttctggctttcaacctcccgacctccctctaattacctcaattgaactcgatttagacgtggtgctgccacctcccgcctgccgcacaatgtttcttcgcaccgtttctcgcgctgtccctcgcagcaccgcggccatccgtgctgcaccgactgcctctgtgaacgccctgcagacccgcgctgcctcggaccatgctatccccaaccctaccctcgccaacattgagaagcgctgggaggtcatgccccctcaggagcaggccgagctctggatgcagctccgtgaccgcatgaaggttgactggcaccagatgaccctgcaggagaagaaggccgcttactacattgccttcggcgcccacggcccccgcgcccagccccccaagggtgagggcatgcgcgtgttcgccaaggtgctccagctcactgccgcctccgttgctgtcttctacgccatccacgccttcgccggcaagcagcccgccaccatgtccaaggagtggcaggaggcctccaacgaatatgccctgaaagagaagatcaaccccatccacggcatcagcaaagagggttacgaaggcaagggcttcgtccagagcccccctgccgagaagtcataggtgtaccagttgcccgaccgggaatgagttgatatctacgccggacggacggcggcacccatcgcacgatctatatgtcgatcttattacaagctactctttccatagccatgttcgacatgtctttgtgtcggaggatgggcctccgcccgtgcgcgcggccgtcgattgttccattctatcttttttggcaagcattggaaaatgcgtgtatcccgtactgtgctataatcaatgtatctcttttgtagccatagagc

SEQ ID NO: 20 - DNA, 641 bp, metagenomes purified from environmentally challenged niches
gtggcgcgccgggggggcatctacctcgacggcaacaacgacctggtcactatgaagggtaactacatctaccacaccagcggccgctctcctaaggttcagggtaacaccttgctgcacgctgtcaacaactactggcacgacaactccggccacgccttcgagatcggtgagggtggttacgttctggccgagggtaacgtcttccaggatgttactacccccgttgaggaccccgttgacggccagctcttcacttcccctgaccccagcaccaacgctcagtgctcgtcataccttggccgggcctgcgaaatcaacggcttcggtaactctggtaccttcaaccaggctgacactagcctgctgtctaaatttaagggtcagaacattgcttctgctgatgcttactctaaggttgcctcgagcgttgccagcaacgccggtcagggacacctgtaaaatggaaagaggaggttcagagcttaatttgctcatgtcggacgacatagccctagcggcttgctggtgaatttggcataatagcgtttctcttctcatacctactttattactccgtttggatccttattaggtaaatattagcccattgtatggttcaattcgattgactttgaggc

SEQ ID NO: 21 - DNA, 591 bp, metagenomes purified from environmentally challenged niches
gtggcgcgccgggattctcatcatcagataaaatcaagattaatcttactggacatcacaacgatccaacacaaagttccttcatacttcaaacaaatctctacaattgaatcaaaatgccatccaaaaccgaagcagcccgtctacaaaacgacttcggcgcagactactgggttagaaatacccaagaacgccgccactcaaccgctggccgcggactattcgccggtctccaggatgtcaagcactataacgtcgaccatggctgggcccgtcgcaagtctagcgataaccccggactccttgcttctttcttcagtcgattcaccgggggatcataccatccgccctcggaatagaattccttttcttaatgtgcgatattgggaggagtgtgatttgaattgggaataagggaaaagagtgcttggaatatttgagtctcagacttaactcgagtcaagtttcatttatgagtatactgaggtttttgtgttagtagcttggagtttgggtggtttattagtattacctattgcattaccatgtttatacatcgtgaatcatcgaatgaataccatgtcttcaatt

SEQ ID NO: 22 - DNA, 639 bp, metagenomes purified from environmentally challenged niches
gtggtatcaacgcagagtgacgagcccaccatccccggaggcgccgctgtcaccatccactcccgtaacgagaagaaggcccgtaaggccattggcaagctcggtctcaagcacgtccccggcatcacccgtgttactctccgccgtcctaagaacatccttttcgttgttaaccagcccgatgtctacaagtcgccttccagcaacacctggatcatcttcggtgaggccaagatcgaggacctgaactcccaggcccaggcttccgctgctcagcagcttgccgccgccgaggctgccgccggaggtgagcacgctggtcacgaccacgagcacgacatcctcggcaagggcaaggcccccgagaccgagggcaagaaggaagaagaggaggacgacggcgaggaggttgacgaggccggcctcgaggccaaggacatcgaccttgtcatggcccaggccaacgtctcccgcaagaaggccgtcaaggccctccgggagaacgacaatgatatcgtgaactcgatcatggctctcagcatatgatttggctgcctgccggcaggatgaatgagtgagctttgggcgcgaggtcacgttgatatccctgttctgggccctctcccttaagtgtatagc

SEQ ID NO: 23 - DNA, 832 bp, metagenomes purified from environmentally challenged niches
gctcccaacgtcaacaccccctccgccttcccctcgaccgttactcctgcccgtccgattacaacaaggagaatgttccttcagcgtacggtatctaccctcgcgaggcgcacccccgtgcggggccttgctgccgcgcgcccgttttcttcgtccgttagccgattcaacaagtacgaggttaaggaggccaagctccgttctcttgacgagatccaaactgaagaagacctcatcccccctggtgctaagcccggtaccgtccctagcgatatcgaacacgccactggtctcgagcgtctcgaactcgtcggtaaaatgcagggaattgacatcttcgacttgaggcctctggatgcttcccgcaagggaaccctcgaaaaccccattgttgtcaacggtgctggtgacgagcagtacgctggttgcactggttaccccgtcgactctcaccaggttaactggttgactgtctctcgtgagcgccccatcgagcgctgcaacgaatgcggtaacgttgtcaagctgaactatgtcggacctgaggaggaccctcacgctcacgaccacggccacggccaccaccctgcccccgaggagcccaagaccttcgccgactacgtcaagcccgagtactggtaccggtaaataccccagcagtacgacgcgagagttttcaaaaaagagaataagaaacaagcaaagggacggatcaagacgggctagtgcgggaatgtcaaacgcaacatatttaagcattgggtctactatatacgggttcattcgtccattgattcctcggtctagtgttttcttgaacgtctttagctgg

SEQ ID NO: 24 - DNA, 832 bp, metagenomes purified from environmentally challenged niches
ccagctaaagacgttcaagaaaacactagaccgaggaatcaatggacgaatgaacccgtatatagtagacccaatgcttaaatatgttgcgtttgacattcccgcactagcccgtcttgatccgtccctttgcttgtttcttattctcttttttgaaaactctcgcgtcgtactgctggggtatttaccggtaccagtactcgggcttgacgtagtcggcgaaggtcttgggctcctcgggggcagggtggtggccgtggccgtggtcgtgagcgtgagggtcctcctcaggtccgacatagttcagcttgacaacgttaccgcattcgttgcagcgctcgatggggcgctcacgagagacagtcaaccagttaacctggtgagagtcgacggggtaaccagtgcaaccagcgtactgctcgtcaccagcaccgttgacaacaatggggttttcgagggttcccttgcgggaagcatccagaggcctcaagtcgaagatgtcaattccctgcattttaccgacgagttcgagacgctcgagaccagtggcgtgttcgatatcgctagggacggtaccgggcttagcaccaggggggatgaggtcttcttcagtttggatctcgtcaagagaacggagcttggcctccttaacctcgtacttgttgaatcggctaacggacgaagaaaacgggcgcgcggcagcaaggccccgcacgggggtgcgcctcgcgagggtagataccgtacgctgaaggaacattctccttgttgtaatcggacgggcaggagtaacggtcgaggggaaggcggagggggtgttgacgttgggagc

SEQ ID NO: 25 - DNA, 1263 bp, metagenomes purified from environmentally challenged niches
acccaaaccctgcgaagcaaaacgcgttactcgatttggtcatttcctccaaagcatcattcctctttgggcactgcctgtttcgtccattaatcaactgtgcttgaatctctaactatcttttgatataccctctttatctctctcccctttaatctttttttctctctctctcttttcctttctttttcggttactcactatcatggccgacatcactgccgtcggtgaggagaacccttctcctacccaggatgagctgcagcaggccgcggccggtaacggcgctcctgataaccgcactcccaagcgtcgcatgagtgacgatgaagaggacgaggagaagcagggtcgcgagcgcagaaagattgagatcaagttcattcaggataagtcgcgtcgccacatcaccttctccaagcggaaggcgggtatcatgaagaaggcatacgaattgtccgtcctcacaggcacccaggtgctgttgctggtcgtgtccgagaccggcctggtctatacctttaccacccctaagctccaaccattggtcaccaaggcggagggcaagaacctgattcaggcttgcctcaacgcccccgaccctaccaccagcgagaatggcgtcgatgcccccgaggtcccagcggagacccccgaggatgtcaaccacgccaacgtcaacgctgccgcagcccagcagaccaacatccctcgtcccaccggaatgcatcccggctacatgaccaacgaacaacagcagcagatggcctactaccaaaaccacctccagcagcaacagcaggccggtgggcagtaccctggcatgtctgtcggtggtcgcatgcctacgcagcaccagcctaccgcataatcttatttactcttatctacgctcccacgcacctcctctttctgatttccctgcatatggtcttgtttttagtagctgaggagtccagagttcagttgtttttgccttctttccgcatctaccctttattttcccctctttcgttattatctctctcccctgacatttgatacccgacaatcctgttgttcaatccatcgtcgcatgaaaacgggtcctataaatataatgcatccccctgtttactttcgactgcgaacgagagcatgcaaatctgaagaacagcatggtcaattgtctcagtaacctcgttaaggcgccgatgagtttggcgtttacatactctgctttggaacgtgtgatgcctttttaccgttcaatgaaagcgactc

SEQ ID NO: 26 - DNA, 1066 bp, metagenomes purified from environmentally challenged niches
aggctttgatggcctcttcaaaggggaacattgttcactcgaccagagttgagtagagccaagaccattccataatctccaggggcatatcgccatgccgtcttgtcaagacgatctccttctcacacatattgatgataggtaccgttagattggactcggttgaaccgagtccaatttggaactacgactcctcccgggcctgattttgcaacgaggattccactcccgtacactacagaactatatcgacaccgtcgctgagattcaatgtattctttcattcgactggcttcttcctccgggtgagacgagctgatatttgggagaaatattggacatcccagataatctcgcgcaaagtctagtttggtctggttgatatcggaaatgatcacttgtttggctccaaacgctgtggccgtcgctgcacagaacagaccgatagtccccgacgcttgtaccaggacagtatgaccgggagtgatacctgccacccgagctccatgaattgcaacactcaacggctcgaccaaaacagtttcttcaagtgagaaattttcgggaatcggatacaccaaatcctcgggtgcgcggaatagatgggtcagagtcccatggttattggggggaggatccgcggcaaagctcatctctggaaaaatatcatatctccctgctttacattgtttacatcgtcgacgagagaaactagctcgatggcaaagcggtcgccaggaatcacttttgtcactgccggtccaattgagtgcacgatacctgatgcctcatgacccatgaccagtggttgctcgtcagagaccattcgaagtaccccgccgtgtttccagaaatgggcctatggaattggaaattagcaaaagagaccctggtgaaaggaagagggatttgtggggactcatatcgctcccatacacacccacatacgcgatgcgaactaatatatcatagggatcactgagggtagggacatcgcggtactcaagtcgagctttcccaggcccgtagagtaggcaggacaaattattctgaaattatgatcaac

SEQ ID NO: 27 - DNA, 1066 bp, metagenomes purified from environmentally challenged niches
gttgatcataatttcagaataatttgtcctgcctactctacgggcctgggaaagctcgacttgagtaccgcgatgtccctaccctcagtgatccctatgatatattagttcgcatcgcgtatgtgggtgtgtatgggagcgatatgagtccccacaaatccctcttcctttcaccagggtctcttttgctaatttccaattccataggcccatttctggaaacacggcggggtacttcgaatggtctctgacgagcaaccactggtcatgggtcatgaggcatcaggtatcgtgcactcaattggaccggcagtgacaaaagtgattcctggcgaccgctttgccatcgagctagtttctctcgtcgacgatgtaaacaatgtaaagcagggagatatgatatttttccagagatgagctttgccgcggatcctccccccaataaccatgggactctgacccatctattccgcgcacccgaggatttggtgtatccgattcccgaaaatttctcacttgaagaaactgttttggtcgagccgttgagtgttgcaattcatggagctcgggtggcaggtatcactcccggtcatactgtcctggtacaagcgtcggggactatcggtctgttctgtgcagcgacggccacagcgtttggagccaaacaagtgatcatttccgatatcaaccagaccaaactagactttgcgcgagattatctgggatgtccaatatttctcccaaatatcagctcgtctcacccggaggaagaagccagtcgaatgaaagaatacattgaatctcagcgacggtgtcgatatagttctgtagtgtacgggagtggaatcctcgttgcaaaatcaggcccgggaggagtcgtagttccaaattggactcggttcaaccgagtccaatctaacggtacctatcatcaatatgtgtgagaaggagatcgtcttgacaagacggcatggcgatatgcccctggagattatggaatggtcttggctctactcaactctggtcgagtgaacaatgttcccctttgaagaggccatcaaagcct

SEQ ID NO: 28 - DNA, 564 bp, metagenomes purified from environmentally challenged niches
agactcaacgataattcaatacccagttgcaacactatttgttttctaaacatatcctcaagaccaattctaccttaatctccccaacacaactcaattgaaaacatacaccatgcctcgcggagccgaatacgccaacggtcctctccagagcgacaatgccatcgaagctggcgaaaataaggcccacggaacctccggtaacaccggcctcaaccgcgtcaacaaggtcgccgaattccccgaaggcgccagaggaaccggtaccgctgctaacccgctcagtggccagggtagcgccggccatcaggatggaaagggtggccatgacccgaagacccttggagagaacaagggactgggtactcaatgatcttatgattcagaagacatgagttatttgcatgagctgggctcgctgcgattctgtgggattctgtgatttgtaatatgatttgcatgggtcaggtcagacttaattaagcatgcgctattgtttccgttatgcttatgatatggatgggtccatggttggagttgataatctaatatggaattgaagtg

SEQ ID NO: 29 - DNA, 39 bp, metagenomes purified from environmentally challenged niches
attccatctaaagctaaatattggcctgagaccgatagc

SEQ ID NO: 30 - DNA, 577 bp, metagenomes purified from environmentally challenged niches
gagactatgacgacgatcacagagttcccgccattctacacgcagcagccgaatgcgagcgcgctgacgcagcagctggggctgtggcagaagcatatactgagcacgtgcaagcagcggcggcagttcaagctgagcgtgagtgatgatatctgggccaacgagaggataaagcgagctgcttctcgtgaatttatttctgtgattatctcctcgctggtgacagaagggctagcgagctatacagacgccaccaaggaggctgtgtgggtgtactggcggagtctatctgattgggcgcaggcggcgtacgcgtacgcggaaagcacagcgcagctgaacacgccgttgacgtactatgagctagtacaaggggagtacagccatctatctgagctgcatgagatgccagtagagctgctcaagcttgctgtgtcgctgctggtgaagcagaacaaagcggtgataatcaaaacgagtcaaggggaaggtgtcaaattcgtctagtatagaataacttaggttacattggaatctggtaatcaattcccttgtcattcagcttctgctgctttcc

SEQ ID NO: 31 - DNA, 606 bp, metagenomes purified from environmentally challenged niches
gggaacaaactctcattctaactaaatactttttactctctgctcccctatcgcattctttttaggacattcagaaggtgatcgcttgaccaaatgtctatcccaaaagcggcagctcataccgacaaggcgcctcagcctttcaaggacctctattcgcaagcagttattgctggtggcgtggtctattgctctggaattgttgccattgaccctgaaaccggtagcctgattgaaggagatgtcaaggctcatacggaacgaattttacaaagcctttctagtactctacaggccgccggtaccagtcttgatcgagctgtaaagatcaatgtttacctagcaaacatggaagacttcacatccatgaactcagtttacgaaaagtattttgtggatggagtgaaaccctgcagaacctgtgtggctgttaagtctctaccttttggcactgatgttgagatggaatgcattgcagtactgtaaatgtttagttttatgcgcaactgagaaagacggaaggatcatcctattactttttcgaatgtgctctttggatttctctgttggatacacaacaatgccacacattgggtacaaccagat

SEQ ID NO: 32 - DNA, 411 bp, metagenomes purified from environmentally challenged niches
ggaaccaattacatccatcaaccaaaccaacaaaatgctgagatctcaattcggtgtaatttcaaacgcagcaaagacagccgcattcctcaagcctgttcaaaccagattgtacgctagtggcgctctctcgaagggcgacatccaaactcgcatttttgatgtcctcaagtcgtttgataaggtgaaggctgataacctcactgaatcggcttctttcaccaacgacctcggcttggatagcttggacgccgttgaagtcgttatggccattgaggaggagtttgccatcgaaattccagacgctgaagctgacgcaatccaaaacgtgaaccaggctatcgaatacatcgccaaaacccctgaagcacactaaacacgctaaataattttatcaattcatttcaaacg

SEQ ID NO: 33 - DNA, 619 bp, metagenomes purified from environmentally challenged niches
gtggtatcaacgcagagtggcgcgccgggaacgaagaaagtttcttcgacctacctatcaaagatatgtaaggagcaacataaatcaatattcttttatctgattgaccttcactctagtgcctcgctacgatcagttacaaccttgcccgcgcgaatggaacgtatacgactttccgaacaggccgcgacgatttgcaaccaaattcgtgaaatgataccagagactgccactttgcccaatcaacctggcaaggatcaagctgaactcatgcatgaagatgaaaacgggaataagatatacggcgggaaacttttaacggagagagctgctcgactgaaagagcacatgaagattgaccaagtgagtgccagatttatctcacagtactttactaatggcattcaggactggacagagcgcttggtatattggacaaagccgacgaaactattgaaccaacggaaacaaggatatatcataccgttatctaaagacatcgttctacaacctgggggacctttagaagcaaataacggctttcgggtcacaaacgagcggattctgagttcaggagctgcccttttcattatgccccaatgatattattttgaaaccc

SEQ ID NO: 34 - DNA, 1647 bp, metagenomes purified from environmentally challenged niches
accgctaccgtcatcactacaaatgctggctcgcagcttacagcaaatcagacgctcaagcaggctgagcttacaattgcgcgcctacgccagcagtccagaccgcagcgcaagcttctctaagctctcagagcaagatctcccatcactcgcctccatcttctcatcccccgacacctccctcctcaccacgctcggcgacaagccaacagccaccagcgacgatctcgagccattcaacgtcgactggatgggcaagtacaagggccactcttccataattgtgaaaccaaagacgacgcaagaagtcagcaaggtgctgcagtggtgcaacgagcgcaacgtagctgttgttccacaaggtggcaacaccggtctcgttggtggatccgtgcctttgcacgacgaggtcgtcttatctctctcctcaatgaacagcatcagacacttcgaccctctttccggttacgtttctgtcgattccggtatcgtgctcgaaaatttggataactacctcgcacaacaaggacacattgtccctctcgatctgggtgctaaaggctcctgtcagattggtggcaacgtcgcaaccaacgctggtggtctgcgcatgttgagatacggtagtttgcacggcaacgtgctcggcctcgaagtcgttctgccagatggtagagtaatcaatggtatgaagggactcaagaaggacaacactggtatcgatctcaagcagctcttcatcggctcggagggtgttctcggtgttatcactggtgtcactctcgccacacccgtcagaccatccgcaactaacgtcgctgtcttcgctttgcctgactatgagtcagtgcagactgccttctcatcagctagacgcgatctcggtgagatcttgtcggcgtttgagttcttcgatgctgcctcatacaagctcgtgcgcagccatggacacgcagctgagcgcaaaaccttcgaagatggggaagacgcaccatttttctgcttggtcgagacgtctggctcgaacaaagaccacgacgatgagaaactgggtgctttcctagagcagctcatggagtcaggtatcgtcaatgacggtgtattggcacaagacgagacgcaaattggccagctgtggtcgctgcgtgagggcattccagaagctgcaggcaaagctggtcgcgtgtacaagtacgacttgagtttaccagtcgagaagatgtactcgctggtgccagagctgcgccaaaagcttgctgagaagggtctgcttgccgctgagtcagagggtggtaatggagatgggccagtcaagacagtcttcggatttggtcaccttggcgatggcaacctgcacatcaacattgttgccgatgcttacagaaaggaggtggaggaagtcgtcgagccatacatttacgagttggtagccaagtacaatggatctatctcagcagagcatggtctcggtctgatgaaggcaccttatgtcgcatacagtcaagacgcgccatcgcttgacctcatgcgcactctcaagaagacactcgatccaaagggcattctcaacccatacaagtgcgtcaccgcggaatagattggagttatagatttacgttatatgcatgcgatcctgttacattatcc

SEQ ID NO: 35 - DNA, 669 bp, metagenomes purified from environmentally challenged niches
gtcatcaacttcattcagcaaaatggctctctattacggcatcgtatttggtatcttaacatttgagattattctctttttcttattcttgttgcctatcccaactcgttggcaaaaaccagtgttccgttggttagctacctcacctaccattgcacatgctcaatatatcatgaaaattgtatttgtattcatctttgtgctcttccttgattccgtcaacactctccgcgctttctacgaagtagtgaacactgaagatgagaatggtggtattccagctgccggtaactctgatttcagagctcaagttggtcaagctgcaaagaagttttatgctcaaagaaatttgtatctcactggattcaccattctgttattactcattttgaacaagatcaagaacatggctatggactatattagattggaagatcaattcattgagcttgaaggatccgtttccaaagatcccgccatcagaaaggcaagcaaagaaatcgacactactcccatcgaagaccatgttacaagactcgagcctgttgaacaagaacaggaaaacaaaaaggatatctaattcacacctgtaactaatatgtaaacatctccctcgctaaaagcgcaataaactaaaatcagcatcattgcgtatctctttcttctcac

SEQ ID NO: 36 - DNA, 873 bp, metagenomes purified from environmentally challenged niches
gtggcgcgccgggaggcgcctaacggtcatgaattgcctcctcgcggttatgatcccggagaaaacacttaccaagcaccacctgatgaacgtagtcaagtagatgttgcgattgaccctaaatccaaccgtcttcagctgttgaagcctttccagaagtgggacggcaaggacatcaccaatgttcctatcttgattaaggtgcaaggcaaatgcactacagatcatatttccatggccggcccttggctcaagtatcgtggtcatttggacaatatcagtaacaatttcctcattggcgccaagagtagcgaaggcaaagtcaacagcatcaagaatgcttttactggtgaatacaagggtgtccagaaacagctcgtgattacaagaaggaaggtgttcgttgggtcgtggtaggtgatgagaactatggcgaaggctcctctcgtgagcatgccgctctagaacctcgattcctcaatggagctgccatcattaccaaatcatttgctcgtatccatgaaaccaatctcaaaaagcaaggaatgcttcctttaacctttgctgatcccaaggactatgacaaggtggacgcctcagataaagttgatattcttggcttgactgatttccaagaaggaaagccattgacccttcgcttgcacaaaaaagatggatcaactgtcgatgttcctttgaaccatacattcaacggtcagcaaattgaatggttcaagcatggatctgccttgaaccttatgaaggaaaatactgccaagaacggaagcttgtaggtgcaccgttacgttatcttcacaagcatttgtatgtcaaataaactcgattagttacttgcacttttgttaagtttat

SEQ ID NO: 37 - DNA, 874 bp, metagenomes purified from environmentally challenged niches
gtggcgcgccgggaggcgcctaacggtcatgaattgcctcctcgcggttatgatcccggagaaaacacttaccaagcaccacctgatgaacgtagtcaagtagatgttgcgattgaccctaaatccaaccgtcttcagctgttgaagcctttccagaagtgggacggcaaggacatcaccaatgttcctatcttgattaaggtgcaaggcaaatgcactacagatcatatttccatggccggcccttggctcaagtatcgtggtcatttggacaatatcagtaacaatttcctcattggcgccaagagtagcgaaggcaaagtcaacagcatcaagaatgcttttactggtgaatacaagggtgtcccagaaacagctcgtgattacaagaaggaaggtgttcgttgggtcgtggtaggtgatgagaactatggcgaaggctcctctcgtgagcatgccgctctagaacctcgattcctcaatggagctgccatcattaccaaatcatttgctcgtatccatgaaaccaatctcaaaaagcaaggaatgcttcctttaacctttgctgatcccaaggactatgacaaggtggacgcctcagataaagttgatattcttggcttgactgatttccaagaaggaaagccattgacccttcgcttgcacaaaaaagatggatcaactgtcgatgttcctttgaaccatacattcaacggtcagcaaattgaatggttcaagcatggatctgccttgaaccttatgaaggaaaatactgccaagaacggaagcttgtaggtgcaccgttacgttatcttcacaagcatttgtatgtcaaataaactcgattagttacttgcacttttgttaagtttat

SEQ ID NO: 38 - DNA, 718 bp, metagenomes purified from environmentally challenged niches
ggcgcgcccttgacacaggagcacgggtttcccgtgcgcgtcatcgttccaggcgtggcgggcgcgagggccgtgaagtggttggatcacatcacagtgcagcgggaaatgagcagcaatcattatatgcatttcgactacaaggtcctaccaccagaagcggtcgatgcggaaagggcacgcaccttctggcataaagtcccgccggtgatcgacatgccagcgaattctgccatcacgtcgccacgaaatgaagacacggtggaagtggatgcagagggatttatcacggtggatgggtacgctttgccggggggagaagatgggccggtgaaaagagtcgaggtctccattgacaaggagagatgggtcgacgcggaactgtttacacatcccatggaaagcaagtggacttggaaaatctggaaggccaaagtgcaggtcgagccgggcgagcgaagatgtctctacagcagaaccactgatgaagcgggcaactcgcagccgcagcgttctcagtggaacctgagaggcgtatgttacaacggctatggagaagtgaggaatttgaaggtggtgaaaggataggcccaatcgttcattccatcatccatcaagatgtgtctgtatgtgtatgaaggcctgaagcgaccacgggaccccagggtggtcactaaacagtactcaaacggactgtttggttcgtttgacactttcg

SEQ ID NO: 39 - DNA, 160 bp, metagenomes purified from environmentally challenged niches
aatcaagttcgactgtcaaaatgccagccaacacgatgtctgccactctcagatccctccacgttcccgggaaaccagtcatcttcgccaatgtctgggacaccgtctccgccaaatcaatcgcacctctggattcatgcaaagctctagcaacggccag

SEQ ID NO: 40 - DNA, 1274 bp, metagenomes purified from environmentally challenged niches
gccttgcccatgctactcatcaaccctcctcgcaacctcatcggccaaagtcagtctggtaccggcaagacggctgcattcaccctcaacatgctctcacgagtcgacccaaacatcatgacccctcaggctatctgtttggcaccgtcgcgagagcttgctcgacagattcaggaagtagtcgacaagattggccagttcacccagatcaagagtttcctcgctgttccgggctcttggtcgcgtaatgtcaagatcgacaagcacattcttgtcggtacgcctggtacactcgtcgacatgctttcgcgaggaggcaggatcttcgacccgaagcagattagagtctttgtgctggatgaagcggacgaaatgatcgctttgcaaggtctgggggaccagacgaagcgcatcaagaggatgctgccgcctggggtccagaacgtcctgttctccgctactttccccgacaacgtccgagactttgcaggcgacttcgcacccgaggcgaaccagatcttcctgaagaaagaggagatcactgtcgacgccatcaagcagctctacctcgagtgtgatggagaggagcagaagtacaacgccctttctgccttgtacgacatcatgtcgatcggtcagagtatcgtattctgcaagcgaaaagacacggccgaccgaattgcggcgagactgacggatgagggtcactctgtcgcttctctacacggtgacaaacagactcgagaccgtgatgacatccttgacgctttccgagatggcaaaaccaaggttctgatcaccaccaacgtcgttgctcgaggtatcgatatccagcaagtgaacatggtggtcaactatgacgttcccgatctcggtccagagggagattggaagcctgatatcgagacctatatccatcgaataggtcgaaccggtcgatttggtcgaaaaggttgttcggtcatctttgcccatgatcagaggtcgatgcaggatgttcagttcatcgccgatacgctcggcaagaaaatgagcagaatcaacgctaccaggcagactgatctcgatcagctcgaagcggctttgaaagccgccatcaagggcaatcaaccgaaagagtgaagagtggcaccgaattcgaagagacgggcgctggaagatatcctgaagcaacagggaggagctccccttatagcatgatcattgacgataaccatctagggcctgaagtacattatgatagatagcagacatcaatgcaacgtcgcgtcgcc

SEQ ID NO: 41 - DNA, 919 bp, metagenomes purified from environmentally challenged niches
cacctccaacctctttctagtttaccttcaaaacacatcggtgtaaggtcttgcccaacatggctaccttctcgacccgcatcaacctcgtccccacctcccgaacgctcgctagcggcgttccattcgcacccaggatcgcccttgttcatcctcccgcgtctcacggtcacggaacgagcggtcccaggagtgatgtcccacccaggtgggctggtgtccagggtggattcgcctcgaactcgagggtcaatgtactccccaccggcaacttccagcaacgattcatgtccaccacgccagcccgcaagatcgaggctcaaccccacgtccgaggtgttcccgattggtcggcatatcagtcttcgggcaagggcgagaacacccgatccctttcgtacttcatggtcggatctctcggtgtcctcgctgcttcaggtgccaagtcgaccgtcagcgacattctgagcaacatggccgcttcggctgatgttttggctttggccaagatcgaagttgagatgggtgctatccctgagggcaagaacctgatcgtcaagtggcgaggaaagcccgtcttcattcgacaccgaacggaagatgagattaacgaggcacgcgcagtcgacatcaagtctttgcgtgatccggagagcgacgaggataggacccaaaggggagagtggcttgtcatgctgggtgtctgcactcacttgggttgtgttcccattggcgaggctggtgattacggaggatggttctgcccctgtcacggatctcactacgatatctctggccgaatccgacgaggtcccgcccctctcaacttggaggttcccgagtacgctttcaacgacgacgaggagaagcttgtcattggttaggtgtagatggacatatgcagtctatggccatagcg

SEQ ID NO: 42 - DNA, 1459 bp, metagenomes purified from environmentally challenged niches
ggggagcatcaccatagtgacagggactgtagctcggtcaagcgcgtattcgcacttgggcgcctggacgttactctggccgtggagtgcgggagtgtcaggacgatgtcccttcgtgacctcgcttgctacactctcacgctcaagccatctaccgagaataccctcctgaccgagctcacggctttggagggaccgagtgaggagccacgattcgcaagagtgcgggagaaggtggaaggagaggtctattcgtctgccatatacgatgcgttgacgggagccaagctggcctcggtgggtttcgcttccgaaaagcagaagaacaggaggctacagctacacaacccggatgagagtgtgccttttgacaatactagcaagctaggtttcgaatggacattcatcttcgaaggcaacaagtacaggtggacgagagagctatacggaaaagattatatctgctcactagaccggaaacccgatccaagggtggagatctgcctagctcgagacgcagattcgaaagcgcctggacgactgcagattctacactacaacatcgaacgattcccgaacgagatcaaggatttgaggggactggaaacgctactcattgctaccctcatgtgcttcgtcgacgcggccgaagatcggtccaattccggtccgacccgcacttcgcccttgcctgctaagccggttgccaatgctgcagcaggtcaaagcggcaccagcgcaagtggatcttctgatacccgagcgaaagttgcgccggtgacagtgccagtaatcactgcagaggactttgaggatgattgtgacccgaatgagatactggtaggaacggagactgatgtgggcgagcacattgcacgagctatagcgcttttggaggacccgaccatgctgttcattgtcattcgaacgcgaactgcggccgcgagctcaagagcgttagaagtctccttaggggttacaaggttccggcaccgtgagggcatgagcgagctgcatcaatacgtggtagaggaagatccggtccggaagccgaaacccattatgcctgctcagggcctcaagttgatcaacctggatgatcgaccagcggcacaatcacccaccaaaccggaatggtctgccccacctaacatcgctgtttacctatcatcgatcgagttgccagatctcacgcccaagcccaagcctgtccaggggcacacacggccgccaactcaagcacctcatgctcggcctccgccgccttctcaactaccacaaaagccgcagccgcggccacgcccgcctccatccgatggttcaggtagtagtcagactacactcgcttcaacgcgaccgccccaggacgacgggaaggattcgagaaagtctagctttggaagactctttggcaggtagtacgatacacttagcagggcatatgcaggtgtatcgacgg

SEQ ID NO: 43 - DNA, 623 bp, metagenomes purified from environmentally challenged niches
ggcgacgacaacaagaaaacaatacctcacctgaacatattcaataatggcgtcccaattgatgcccctggagctgatcgatcgttgcatcggatcaagaatgcgtgtgatcatgaaaggcgacaaagagttcagcggcacacttctcggattcgacgacttcgtcaatatggtgctcgaggatgtcaccgagtacgactacaccggcgcaacgaccaagcttcccaagatccttctgaacggcaacaacatctgcatgctcatcccaggtggcatgcccgagggcgagtcatgaatcacggacatatgatatcccttcttacgtctcttgaaatggcaaagcgagtctgatttaagaaccacacgtgtcatgagaaggcagactataccgctgtccagtccaagctgcttgaacaataattatcccgacggagccacgaaaacgtgacaagcggaagctcgcattcgcaaagcgccggcgcaataaaacgccttgttcagctcgccgactttgtgcatgcatgcagctcgccacaccccgcagatatcaggctgccttcttgttatcaggtatgcgtgtttatactctagcttatttcagctatgcaaaacctatatcatcc

SEQ ID NO: 44 - DNA, 489 bp, metagenomes purified from environmentally challenged niches
gcaaaggagttgtcgcctgacgtcaagcctgagccgacatggtcttgtggcgaggttgtcaatgtcgtcgatgagcacggcaatgtcatcaaaccgtcagacctctgggtcaagatgggtatgcagcagcaggacaatgtggacaacctattgatcgacgacctgtgtgatcagatgagggccaaggccaaatgcacagagaacggcgctcaattgaatgtcgacgacctgaaccacatgatgtcgtatgacaagtcatataagcagaaaagggtagacgacctcaaagacaagtacggctggggagcagtctttggcccgaaatgagccgcctccgcgggggcaaggtggacggacgatggtagacatgaatatgagagcaaacagacatagggtctgagtccagtagtgtgcttgtaccaccactgtaaatatttgtacgatagccctacaccacttacaattgatcatgtaactgtgtgaaccgtg

SEQ ID NO: 45 - DNA, 480 bp, metagenomes purified from environmentally challenged niches
gggagcctgacccgccgtgcttggttcatccaatccacctgcgccaccactggtgatggtctctacgagggtctggagtggctcgccgacactctccggaaaacgaaccgcgattaaacgcgtataatacgaaattgtgatggggaggattgtgtacgtagcagagcaagagaaataccacgggaaatctgcaaatgatggaatgatgattatggcgggagtttcttccaatgttcttctgcgaggccaaatatcccggcgatgaaaaagaattccctcaccggcatggcatggccatcctcaggagcaaggtgtttgtgtttggctcgccagggctctatttctcttcgctatgctattagcctcatttgttcttttctctctggcgccacgtcaaaattgctggtttatctccttttgattgcatgttcagtatcggtatgatctcagtataccagcacttgggttgagcattcttct

SEQ ID NO: 46 - DNA, 1139 bp, metagenomes purified from environmentally challenged niches
acctcactttgtgcgaattatcctcctacagcatcagctctcttcagaaagaggctaaatctatagaccgtccggaacaggttgtcaacacgcgcgataagagaagaagggaatctactggtagacaacagatcgatcgctcttcagcaaacgcaagatggagaaccttcttcgtcagatgcaagggggaggtggtaggatgggtgcacggccaggccctggaggcgaaactatcctcgccgacaacggtgaaacagtccatatttcatctcttgctctattgaagatgctcaagcatggacgagcgggtgtgcctatggaagtcatgggtctcatgcttggcgaatttgttgatgactacactatctcctgtgtcgacgtttttgcaatgcctcaatccggtacgacagtgacggtcgaatcagtggatcacgtctttcaaaccaagatgttggatatgttaaaacagacgggccgacccgagatggtcgtcggttggtaccactcgcaccccggttttggttgttggctgtccagtgtcgatgtcaacactcagcagtctttcgaacagctacatccgcgagcagtagccgttgtcatcgaccctatccagtctgttcgtggtaaagtcgtcatcgacgctttccgatccatcaaccctcaatcacttgtcgctggacaagagtcgaggcaaacaacgagtaacattggtcatctgaacaaaccgtccattcaggctctcatacacggtctgaataggcattactacagtctggccatcgattacaggaaaacagaaggggagcagggtatgttgttgaacctgcacaagcggggatggacagagggtttgaagatgcgtgatcactcagagatgaaggagggtaatgagaaggcaatcaaggaaatgctctctcttgcctcggcctacacgaaatctgttcaggaagagacgacaatgacggccgaacagcttaaaacccgtcacgtaggaaagcttgatccaaaacgtcatttgggcgaggcggctgagaaagcgatgggtgatcaagtgacgcagagtctggccatgggtgtcctggctgagctgtagacgtagaagagggaagaaaggaaacgacatgcattgtacatatcgc

SEQ ID NO: 47 - DNA, 674 bp, metagenomes purified from environmentally challenged niches
ggacacaccggtgacgtcttgagcgtctcgttctcggccgacaaccgacaaatcgtttctgcttcccgagaccgaactaccaagctctggaacactctcggagagtgcaagttcaacattgttgacgatggtcactcggagtgggtctcttgcgttcgattctctcctaaccccgtcattcccgtcatcgtctctgctggttgggacaaggtcgtcaaggtctgggaattgtccaagtgcaagctcaagaccaaccaccacggtcacactggttacatcaacaccctcgccgtttcgcccgacggatcgctcgccgcatccggtggaaagtatggcatcaccatgctttgggatttgaacgatggcaaacacctctactctctagaggctggagacattgtcaactcgctcgtcttctctcctaaccgatactggctctgtgccgccactgcttcgtcaatcaagatcttagacttggagtccaagtcaatcgttgacgacctcaagccagacttctccgccgagtaccctgacaaggctcaaaagccacaatgtacttccctcgcctggtctgccgatggtcagaccctctttgccggtttctccgacaacctcgtccgagtctgggttgtcactgcttagagtcgtgaggattgtatgcatggataacgtgg

SEQ ID NO: 48 - DNA, 674 bp, metagenomes purified from environmentally challenged niches
ccacgttatccatgcatacaatcctcacgactctaagcagtgacaacccagactcggacgaggttgtcggagaaaccggcaaagagggtctgaccatcggcagaccaggcgagggaagtacattgtggcttttgagccttgtcagggtactcggcggagaagtctggcttgaggtcgtcaacgattgacttggactccaagtctaagatcttgattgacgaagcagtggcggcacagagccagtatcggttaggagagaagacgagcgagttgacaatgtctccagcctctagagagtagaggtgtttgccatcgttcaaatcccaaagcatggtgatgccatactttccaccggatgcggcgagcgatccgtcgggcgaaacggcgagggtgttgatgtaaccagtgtgaccgtggtggttggtcttgagcttgcacttggacaattcccagaccttgacgaccttgtcccaaccagcagagacgatgacgggaatgacggggttaggagagaatcgaacgcaagagacccactccgagtgaccatcgtcaacaatgttgaacttgcactctccgagagtgttccagagcttggtagttcggtctcgggaagcagaaacgatttgtcggttgtcggccgagaacgagacgctcaagacgtcaccggtgtgtcc

SEQ ID NO: 49 - DNA, 480 bp, metagenomes purified from environmentally challenged niches; identical to SEQ ID NO: 45

SEQ ID NO: 50 - DNA, 1170 bp, metagenomes purified from environmentally challenged niches
aaagttgatcgaccacattgggtctgagaaaaacccaatgcttttttgtacagcagtgaggaatattggtcaatggccgaaaggctgaaccagtaacttggaagaatgaaattgtatttgtataaatacaatagtggttaaaccacataaaattctaaatagattatatataatgacaaaatctatttataagtcttgaccaaactacgtgccagcagtcgcggtaatacgtagaaggctagtgttagttatctttattgggtttaaagggtaagtagacggtaaattaaactctaaaagagtacttatttactagagttatatgagagaaggaagaattcctggagtagagataaaattttttgataccaggaggactgtcaacggcgaaggcgtccttctatgtaataactgacgttgagagacgaaggcttgggtagcaaacaggattagataccctaatagtccaagcagacaatgatgaatgtcatacattagatagattttaatgtataaacgaaagtgtaagcattccacctcaagagtactatggcaacatataaactgaaatcattagaccgtttctgaaaccagtagtgaagtatgttatttaattcgatgatccgcgaaaaaccttaccacagcttgtatagcagttatgaaaaattgttacaagcgctgcatggctgtctttagttaatgtcgtgagatttggttaactcctctaattaacgaaaaccctcactttatttatatatataaagtggttcgctattacattggttgataatagggattaagacaagtcattatggcctaaatgctgtgggctatagacgtgccacatacgcctttacaaagggatgcgatattgtgaaatggagctaacccccaaaaaaggaaatactatggatagtagtctgtaactcgactgcttgaataaggaattactagtaatcgtgaatcaccatcgtcacggtgaattatttctcagttaggtactaaccactcgtcaggcgctgaaagaagaagatgcagtaagtttgatgttttctgtgtatgattatacataaagttgttgtataactacgcagaaaagttttcgtatgcaaaactttgattggtgttaagtcgaaataaggttcgtgtaatggaaattgcacggggagc

SEQ ID NO: 51 - DNA, 1231 bp, metagenomes purified from environmentally challenged niches
ggacgatatgacttcaagcagcctcagcgaattcgagacgcttctgtcacggccacgccagaatggaacctgcttgaagagatcgagtttggccgattgggcaagctcaacctttccgtcgaagagcccgaagacctcgaatcgcacggtaccctccaaggttacgacaagacgtttgaccgcatcaacactcgtaccgaaagacctctcgagatcattgatcgagcatggtacaatcaaaccacttctgacgatcccgttattgctcagctcgctcaaacgcagtctgcccaaatcttcgcgacagatgccattcttgcggttctgatgtgcaccactcgttccgtaaactcgtgggatatcattctcgagcgacgaggtaaccagcttttcctcgacaaacgagattctggtccattcgactacgtcactgttcacgaaaacgccgccgacccacctgccgactctgacgatcccaacaacgtaaactcggcttcttccctttcgctcgaggccacctacattacccgaaatttctcgtctcaagtcattgatgccaagtccaagccatattcgcctagccccaatccgttctattcggaggacgagccatcacccgtcgcttcctgcttgtacaggtaccgaaagttcgacctgtctgttggcgaggaagataccctggacctcattgtacgaaccgaagtcgacgcctatcaaggcaagaaggactctctcgtcactgtcaaggcattgaacgagtttgatcctcgagcttcaggtggtggcaaagccctagactggcgaaagtacctcgacactcaaaagggtgccattgtcgcctcggaaatgaagaacaactcggctaaactcgctcgatgggctatccagtctgtcttggccggtgccgaagtcatgaagatgggatacatctcgcgagcttcgcccagggatacaactcatcacgtcattgtcggtgtgcaaaattacaagccaaaagactttgccgctcaaatgaatgtgtccctcaacaacggttggggtatcgtccgaacgattgccgatcttgtcctcaagcagccagagggcaagtatgtcctcgtcaaggacccaaatgcaggcatcattcgtctctacagtgtgccagagaatgctttcgaggcagaggaggaggaggagcaatagtcgaaaagtctagacaggccgtgtcggacatgcatcatatacttcaagg

SEQ ID NO: 52 - DNA, 788 bp, metagenomes purified from environmentally challenged niches
gagcgctcaaggtccttggccccagaagccgatcaaggtgtcgcgactcagtgtcacgaagtcagatcgtcaggtagctacgacacgttcgagatcggccatcaccaacctgacagcgatacctcgggagtagctgacttgcgcacttccagtcgtatggacacctgcgacgcgcatcttctacggcgggtcaaaagctgccctcttttcagctaccgcgaagacgaggtgtccgaaactgtacaattgcctacaggcgaatggacgacgatcagagatatcactccgagtgcaccaaagatcggctttgaagtgcgcgactcgctctccgcgttcccgacagccaagcctgtcgaagcgaagcacgagtccgcctccagcatatccaatgatttaccctctcagccatcctcaaggccgctgattgagtgtccgacactggtcgccgattcacgcacaacgacggggtccaactctgtgcgcagtttcgacgcccagaccgaacgcctgagcggcttgagcgacgtgcaccacagatacatgcaggacaagccgtcacagcgttctgattcctggaccgacgtcaaatcctccgctccgtcctcccagtcgatggcagtccccaacaaagcggcttacctggctccgatcccagctggcccaaatgacagtaagacttcgagttccggtcgcgccccgtcagacgccgcgaccgaacacgagtgttcgctacaataagtcagacttgctgttggaacgtttcctacctcatgcatacctggcatgct

SEQ ID NO: 53 - DNA, 706 bp, metagenomes purified from environmentally challenged niches
accctccaaactccaagctcttttcaaccctttcctaccttacacaacaacttcaacaacaactatggcacccaagtccactgacaagcccgcatccaccgctggcaaggccccctctgctggaggcaaggctcctgcctccaagactgtcggtgctaagaagaccgcagcaaagaagtctgctaagtctactggcgagggcggcgagaagaagaagcgtgtcaagtccagaaaggagacctactctacctacatctacaaggtcctcaagcaggtccaccctgacactggtatctccaacaaggccatgcttatcctcaactctttcgtgaacgacattttcgagcgtattgccggtgaagcctccaagctcgctacttacaacaagaagtctaccatctcctcccgcgagatccagactgctgtccgcctgatcctccccggtgaactgtccaagcacgctatttctgagggcaccaagggtgtcaccaagtactccagctccaagtaaacttgtcttttgcttggctgagagtctttcccctttccttcttcattgtccctaccctcctgttcttcccctctccctcacattcatcatgttgtctattaggcgagctgcctgcagacttgctcgctgtcaaggctgaagcagtcgcgtagttagtgtaatggagccacaaatgtaattctagagcacatgcag

SEQ ID NO: 54 - DNA, 1203 bp, metagenomes purified from environmentally challenged niches
gatgtcaagcgattcaccaaggatctgctgttcaactcggagggcaacctaaccttcaagccccacttgtggaacgacatccgtcacaccctcctccccacctttatccgacagatcggatacgttcccatcccacgagccgagttctcctcgcctgacattgaccttgtcatcgagaatctggtcctgtccggacccaacctcttccccaacgtcgtctcgctcgagagccacaactcgttcaagttctcgccttaccagcagctcaacaagggtatggacacgcatcaccacaagttcaggctgggtatgagccagatccaggccgatatccgagatgtccgattctcgttccgacgaaagactggatggcccaagctcaaggaccacggtctcgccgatgtcatccttgccggtaagggtatgtcgatcgacgtcgagctcgagtctgtcgagggacgacgagactctgttgtgcgagtcaaccacgtccacaccaccatcgacaccctcaccttctccatccgagactccaagcacgacttgctctacaagttcgtcaagtcggtggccacgggtacgatcaagaaggcaatccaggccgccgtcgacaatgccatccgtacggctgtcggtcacctcgacgaccagctcgtccaggtccgaaacaccgtcgatgacgccaagaagtctgacgagaccacccgaacgcaagccctcaaggacttgtactcgaagaaggcggacacggcacagaagaagcaggccgagtccaaggagcagcctggtactttccgaatcgtcgccaaccgagactctgttctcaaccccgacatgggcggtggcaagggcgccatgaccaacaagatgtggaagaccgaggaccttgcacactctggcaaggaatggcactctcccgctttcgacttgctcgactccaagcacccagcacgtaccggtcagacccaccccgaggccaaggagggtgctggacacggaaacagcttgagctcaaaggctcagcccggcgccaacgcggccgaccagctcaaggctactcacggtcagtctgaggctgaggccatcgctggtcagaagcgacagcaataggtggaagagagggagccgcgtattgagaagtaggaaggactagctgtatacccccttatacttttgtgtctatagtaatgaatgcgtgaaacc

SEQ ID NO: 55 - DNA, 962 bp, metagenomes purified from environmentally challenged niches
ggacctttcatccatcagcgtatcgcatatcagcttcctgacaaagtaagaggtaataacaagacaccacactctttcagcacgtacctcataccggaccgccatgtacacatccgccgtgacactgctctctttggtcttgctcctggcgacttccgttattgcacaagaacaagctggtcggcctggcactcagcgaggcggcgtcttctttgggtgttatgccgatcgacctacaggcaatgccaaccagcccatcactcgagtcgccaactccgacacattctttgaatgcatggagaattgtgctgcgataacgtctccttcgttgctgggatactatcaaccctcctccggtcaatgcttctgcggcaaccttttatttaaccctcaagctcaattgaacggtaacggttgtcaaggtagtgattggtcctttggccggacttcgaccaccttcaggaggttcggtgacgcttgtcgacctttcggtggtgtcggattttctgcgaatcaatacactacagtcactggtcccgtagcttgtcatgttcaatgcgcatcaaacagattcgcctatgtctggtccgatactggaagcaactcatggcaatgtgcttgcagcaacaatgtccgtgttcaggaggacttccagtacacttgtcaaggtggcggtgtatttgtgtttgaacattcagtacaagctcaggcttcttcgcttaacaggaagcggacggtggaggaacaatgggctgttccgaaagacgccctctgtccattcggaatgtcagcgtgcaaggtatcaggtgtcgataatgcttacgaggtatgcttcttttcagaccgctaggcccctggttccctggccacgaggtttgaaacacgccattgacctgtagtgcctcgatacctcagccgagctagaatcgtgcggtggttgtctgcatggtcaattgttctga

SEQ ID NO: 56 - DNA, 909 bp, metagenomes purified from environmentally challenged niches
gggggaggaacggtcgttagcaatgctttgctggagaatgccaagctctgcaagacccagggcaaggagagctctcttcgagtcatcgtgtgtggccgaaataggttggagaatgggtctgcacctcattgggccgaggcgtttgctacgcatggcaaattggtggaagtgaggatgccgcaaaacggcattcgcatggagggcatcaaagctatcgccgacggactggccaagtgtccgacattggaagtgcttgatttgcaggacaacacggctaccaagacaggaacacggagtattgtccgacacctctcaacttggcctaaacttcgaatactcaatctctcggactgtcttttgggttcggtcggcggtatcgctcttgcaaccgcattgtccactggctcgaacaagcacctcgaacagctcaaactgcaatatggcgagtttgacaagaggacggttgagatactgtcgacggcaattagccagcatttgccaaaattgacgacactcgaactgaatggaaaccgtttcgatgccgaagacgaatgcgttgagaccctgaagaaggcacttgagctacatgggaacgaggatgctttggacgaacttgacgatatggaggaggtggacgaggacgaagaggatgatgatgacgaggacgaggaggacgaagacgaggacaaggacactagcgccgacgatgggatcgatgcaggagctgctggagaagacgctctaccaccagtcacgaagaaggacgaggacgtacttgcggatctcctgtccaaggtccacgttcagcctagctgagtccaagcgctttccggtcggcaagtagatagactagacagcataataccttgaccctcatgatgccacccgcatgtacacatttgttctccg

SEQ ID NO: 57 - DNA, 909 bp, metagenomes purified from environmentally challenged niches
cggagaacaaatgtgtacatgcgggtggcatcatgagggtcaaggtattatgctgtctagtctatctacttgccgaccggaaagcgcttggactcagctaggctgaacgtggaccttggacaggagatccgcaagtacgtcctcgtccttcttcgtgactggtggtagagcgtcttctccagcagctcctgcatcgatcccatcgtcggcgctagtgtccttgtcctcgtcttcgtcctcctcgtcctcgtcatcatcatcctcttcgtcctcgtccacctcctccatatcgtcaagttcgtccaaagcatcctcgttcccatgtagctcaagtgccttcttcagggtctcaacgcattcgtcttcggcatcgaaacggtttccattcagttcgagtgtcgtcaattttggcaaatgctggctaattgccgtcgacagtatctcaaccgtcctcttgtcaaactcgccatattgcagtttgagctgttcgaggtgcttgttcgagccagtggacaatgcggttgcaagagcgataccgccgaccgaacccaaaagacagtccgagagattgagtattcgaagtttaggccaagttgagaggtgtcggacaatactccgtgttcctgtcttggtagccgtgttgtcctgcaaatcaagcacttccaatgtcggacacttggccagtccgtcggcgatagctttgatgccctccatgcgaatgccgttttgcggcatcctcacttccaccaatttgccatgcgtagcaaacgcctcggcccaatgaggtgcagacccattctccaacctatttcggccacacacgatgactcgaagagagctctccttgccctgggtcttgcagagcttggcattctccagcaaagcattgctaacgaccgttcctccccc

SEQ ID NO: 58 - DNA, 596 bp, metagenomes purified from environmentally challenged niches
ggatggtgaagcttagtaacagtcttgtccgtcgtcttaaatggcaacacgttcgcagtctcggcgtggtggcgctgactgcccaattgcgaggaccacaacctcagagcgccgaggacgaagattctgaagcagctggcaagaagctcaaactggctggcgaccaagctacatctgcggtcattcccaagtccgcagacaagcccgatactttccctctactcgacacactacctgctactatggctgctggcaccaggtctatgactaggcccttgcatgtcggtgatctgaggttggctgatctgcgtaaaatcatgcaggcagctggccacacggctgagttccgaggtgagggaacactactcattgacaagtccgtcgctgtcagaaaatcaggcacagggcagattgaaatcgaggcatctgctcaagcagctgcaaaccaagctactcctggccgaggtgcgagtagcttcctcgctgtcaaaagaaagatatacgagggtctcgctgttgtcacaggaagttaaatgaccgtgtaccctatattcaatttttgtataatttacgcaataccaacgatattctctcgt

SEQ ID NO: 59 - DNA, 418 bp, metagenomes purified from environmentally challenged niches
gaaaatgaaaattgatgtggagaagctgaataaagatatcagccttttcccgcaggtgcatccgattacggaagatatgaaaatcacgcacaaaggtgtttcgcgccttgtaatgctggacaggtattcatttaaagacactgaaaaaattacgctatctgaaggcgattttgtagtgctgacgatcaaggaagatccaaaatttcctgcaagagggctaggctacattaaagaaattgattgggaaaataaaaaggcaaaggttcaggtcgaagaagagtttcgtcatactcttgaaaagcctgaagaacgggagacgggaatcatcgttcgctctttagatgtcatcgaaaaaccgcttgaaattttttatgaacaaattgccaaaagaaatgcaacaggtcttgctgctgttgaa

SEQ ID NO: 60 - DNA, 988 bp, metagenomes purified from environmentally challenged niches
ggggatgcaacggtgactcaactgcgcgaaatcatggacgacccagctggctatttcttgccaaatctcaaacatggcgccgataacatgttctacgtcggtccacgcggacttgcacaagagctcgaggagctttttaccttcccaagcacaatcctcagaaagcgccaggataccagtcagcatgacgaaaggcaggcaaagaaggcgcgcacgcaagaggacgaagcggctggtgacgcgttggaggagcccgagactgggcgacgcgacagtgtgcttccgactgaacgggccgcttttggtctcgagggtgatgactcgggctttttccttggcgaccagacgatgggagacgacatgctgcctatggacgacatgggagccatggacaccggagtggaccagcgacgcatgcgaacaccatcagtcgcaccgtcggtcaccgaatcgatcgcacgtcagattcagaatgaccgaagcgctggcacacacccactggctatattcgagaaggaggcaagggacgacacgcagtcgcaatcgcaggctacgcccaacaaatcggtggcctccgagtctatcagcaagacttcttctggccaatcaaagaatactggcatggccatgggtttgttgcgaagggagattgaggcgatcgaggaggaagacaagatggtcgggtttgatcacttggcagacaaggcgtccaagcgagcagcgtctgcattcttcttcgagctgttggtgcttggtaccaaacatgcggtcaagcttgaacaagctcaggctttcggcgacatccacatacgcggcaaagacaagctgtttgcagaggttgttgcatagacaaacttgaagagccacgatcttacgcgcaacggagggagatctaatgaccatcttgatgtcgactttaatgttatttggtacttgtacatgagctgctaagagggtcttgaatgagatgatgcatcgcttcatgagg

SEQ ID NO: 61 - DNA, 614 bp, metagenomes purified from environmentally challenged niches
gcagaccgtctcttttaaatctcctccttgacacccgtctcctttgcacatttactacactccacatatctccataacaaccttatatctttacacaatgggtgaccacgccactaccaacgacccctccaacgccaccttcgaggagaagggcaagggcaaggacgtccaggatcaaatcgcggaggactccagcgacgaggagagtgaccaggagcctgagatggttgacgaggaagaggatgacaacaacctcgagcccatctcccaagacaacatcatctcaggtggtcgccgtacacgcggcaagatcatcgattatgccgccgaagccgagaagaacaaggatgagatggaggactctgaggatgacgaggattaccaaggcgctaatgacgacgaggatgaccagatgcgcgactaagcgcatggtcttgatgacggatctcaattaacataggactttggaggattggcgctatggtttctgaaggaggttctctcgtgcgcctttgtggttagcatctcacctatgaaatgtcatggcctgagcctggcaatggacatgactatgaataaatgaaatgaagcctgcttctgtctttgtgtaacag

SEQ ID NO: 62 - DNA, 418 bp, metagenomes purified from environmentally challenged niches
gaacttaagtattttaaagcagttgcactatacaacctgagccggtacttggatgcacggaaagcaatcaatgacctcattcagagctacccggacttccggcaagctgaggccctcaagtcagccattgatgacaaggtggtgcgcgatgggctgattggcgtgagtgtggcaggagcagtggtggctggcgtcgtgggcttggctgtggctcttgcacgtggcaacagaggatgatgctacaggaggcagcaggttgttggacagttcagtgcaccgtgccaatgcttcaacggtctggcacaggaggcagcaggttgtgaccctgcacaagcttgggccatgattctacagacacaccttatggcaatcaaatgtgtgtttgcatgtgcgttgaagagtgtaaatgtgctcttcc

SEQ ID NO: 63 - DNA, 94 bp, metagenomes purified from environmentally challenged niches
tatcccgagtagcatgggacacgtggaatcccgtgtgaatcagcgaggaccacctcgtaaggctaaatactcctgggtgaccgatagcgaaaaa

SEQ ID NO: 64 - DNA, 371 bp, metagenomes purified from environmentally challenged niches
cacgatttaaatacccgggggacgttttggattcgacagggatagatcgagcttaagctgcgagccggagggatcgtctccgtcatcaacgtcgcctaaagataactggcaaacaaaacaactacgctttagctgcttaatgctaaaggctcctttcttccatcgcccatgtggaggaaaaggggttcaacttaagtgggctacgcccgattccgccgtctgaggaagagggaagagacgaatcagactagctgtccggatgcctgccgacaggctaaggaacagtgaaatgttaaatatgtcggatacgctcgtagatgcttaagtggcgatatctctggacgtgggttcgattcccaccgtctccacca

SEQ ID NO: 65 - DNA, 681 bp, metagenomes purified from environmentally challenged niches
gccatcagcaccgcaaagctacctcatcaaccattgaaagcacgcaaataactccccaaagttaatgcccgtacgaccctacctggaagaaatggccgacatgcccgtgcccctgttcgcgtacgacgcaccgcccaccctggccgaccaccctcacgcccgcgagcaccaacacacgaccttcatgcaataccttgcgcgcaagcagccggacccaaagaactaccccaactaccctgacgtggacatccgcgacgccatcaatcactacctgatcgagctcgaatgcccggggatcaaagacgcagccgacatccactgccagtggacgagctcgcggcacctgaccgtcaccggcgacatcgcccgtcctgaggaaagccagatcgaagcgcagatcgagagcaggcccgtctacctggttctgggagagagacgcattggctctttccgtcgcaactttaccttccctgtggaggtcgagcaggaaaatatgactgccaagttggaggccggattgttgaagattgtcttgcccaagcacaagcaccatactccgaagggaacaggaaaggtcgacattgatgtcattgagtgaacgtcttttgggtctgcgattatatgcgaggagttcttagattgccggagtgggtacctgtatgggaattatgtatctgcaac

SEQ ID NO: 66 - DNA, 681 bp, metagenomes purified from environmentally challenged niches
gttgcagatacataattcccatacaggtacccactccggcaatctaagaactcctcgcatataatcgcagacccaaaagacgttcactcaatgacatcaatgtcgacctttcctgttcccttcggagtatggtgcttgtgcttgggcaagacaatcttcaacaatccggcctccaacttggcagtcatattttcctgctcgacctccacagggaaggtaaagttgcgacggaaagagccaatgcgtctctctcccagaaccaggtagacgggcctgctctcgatctgcgcttcgatctggctttcctcaggacgggcgatgtcgccggtgacggtcaggtgccgcgagctcgtccactggcagtggatgtcggctgcgtctttgatccccgggcattcgagctcgatcaggtagtgattgatggcgtcgcggatgtccacgtcagggtagttggggtagttctttgggtccggctgcttgcgcgcaaggtattgcatgaaggtcgtgtgttggtgctcgcgggcgtgagggtggtcggccagggtgggcggtgcgtcgtacgcgaacaggggcacgggcatgtcggccatttcttccaggtagggtcgtacgggcattaactttggggagttatttgcgtgctttcaatggttgatgaggtagctttgcggtgctgatggc

SEQ ID NO: 67 - DNA, 50 bp, metagenomes purified from environmentally challenged niches
gggatgatatgcatcatatagatcttgagaaatcaaggtaagtatacaaa

SEQ ID NO: 68 - DNA, 558 bp, metagenomes purified from environmentally challenged niches
gggaaaaaaactttagaatacagtttaatcaatcttcacagctacaaggctatatcatttgatatagcatatcaaagtggctttgatttctgtaaatttatatctaataataatagtgtttatatcagctaaatacatatttctatcctatctatatatcaccgacagaccatatttgaaactgctgttgacactattattcatatgttcggatttaattttaatacgacaaaattgttaaaaacaattctcgttgtttgttatttgcaggcaacagtgttagctgatccttatacaagagtatcttgggaagcgtatatgaatcatgtcaatggatccgacgactatcgtactcaaggggatgataccagagctacacgctttccagagactaaacctccaaaacaaggaaaagatttcctgtggtcgagtaaaccagtccccagttcagatctatttctggagttctttatgtatgagggagaaccagatgaattcagcaggacgactgaatcgtatcaatcacttccgagcaacgcgttaactgctaggcaaaaa

SEQ ID NO: 69 - DNA, 1164 bp, metagenomes purified from environmentally challenged niches
ggacacatcacacaacaacaatgtctccaacaccaacatcaccacacaacaagctctcgctccccgcaagagcttcttcccacgactcgacagacggcatccgtaagcgagtatgcaaggcttgcgacaggtgtcgattgaagaagagcaaatgcgacggatcaagtccatgctctcgatgcaaagcagacaacgccatctgcgtgttcggagagcgcaaacgatcacatgataaacactatcccaaaggctatgtcgagatgctcgaacaacagcagggtcagctcgtctcaggcctcaaagaaatgtaccacagactccagaaagcctccgcctgggatggccctgtgttggacgaaagcaccggacagcctctcactcacgacatcctgtcagcattagacctcctcgaaccaaagcatgacgacagcaacgagccagaagtcttcgaagagaactgcgaaaagctgcaatcaaaattgctcgcagacggcgcgggctttgcccaccgacgaggatcgatcagttcggattctgaacacagccatcacgatcgacccaaaacatcctcacgccacgacacgcccgtgcaacccaaaccgtcgatcttcaaggagaacctgagcttcgccagcgcggcctcatcaccactcacgcaaagccccatccctcgatcgaaacccttgaacgtcatgccataccaaacgctgcaaccgtcgtcaagaccatccccactccagatgccctcagcatacaacgacccgcaactatacgcacccgaatgggcacaagcactggcagacatgagcggcgatcccaactaccgccaaagattctccatgcagcagcaacaacaaaacgacttcgacaacctgctctgggatccctcagcgcaagcgcccatggaatcgcccttcagccaaccagccttcttcaaccaggcgcaactgatcggcagcggcaacgtctttgggctgtctgacatcaacgatctgggccccaaccccgcggatggcgggatggactttgacttcagcaagttcgtgcagcagaccgaagtcatgacatgaacatgattcttgccttctgtcaatacgcgcgagaattttgcttcagagttccagtccgtgtaattcttgtgtatttattacgatacgaacacgc

SEQ ID NO: 70 - DNA, 923 bp, metagenomes purified from environmentally challenged niches
agagctcttcgtactccacaccaccatcttccatccgaccacactttcatcccaaatccatcaacaacccatctcaactccatctcaccacctcaccatcatcacaatgtcttccttccgcgtcgccgcccccaagatggcctccatggccgctcagtcctccgtgaaggtcgcccgcccggccttccaggctgctcagctccagaagttcacccgcgcctactccgcggtccccaagaacaccgtcttcaacaccatgaagcgcacccagatgatggcccgccaggcctcccccatcgccaagcgtgcctactcctctgagatggccaacgccctcgtccaggtctcccagaacatcggtatgggttccgccgccatcggtcttgccggtgctggtgtcggtatcggtctcgtcttcgccgccctcatccaggccgtcgcccgcaacccctccctccgtggccagcttttctcttacgccattcttggtttcgctttcgtcgaggccatcggtctcttcgacctcatggttgccatgatggccaagttcttgtaaaaatgtgcattccattacctaccgagatggagatggatgcgaaggcgattggggacggagacagtgcgttgctgcagcagcattagtaccggtgttggtcgtgtaccagtagtctgatggagacggatagatggatagaaagctggtgaatgggggctacgaagaaaacgtacctctcgatccatttgtacccatactcatgaagtatatccgtcttctttccttctatcattcgcgcgcacttccttgctggtggctttttggggttgcgctctcaccgaaaagcaacgtcactcttgtatataacttattcgaccacggccatatcttggtttggctggggaaataacaatgtctcatttgtacc

SEQ ID NO: 71 - DNA, 923 bp, metagenomes purified from environmentally challenged niches
ggtacaaatgagacattgttatttccccagccaaaccaagatatggccgtggtcgaataagttatatacaagagtgacgttgcttttcggtgagagcgcaaccccaaaaagccaccagcaaggaagtgcgcgcgaatgatagaaggaaagaagacggatatacttcatgagtatgggtacaaatggatcgagaggtacgttttcttcgtagcccccattcaccagctttctatccatctatccgtctccatcagactactggtacacgaccaacaccggtactaatgctgctgcagcaacgcactgtctccgtccccaatcgccttcgcatccatctccatctcggtaggtaatggaatgcacatttttacaagaacttggccatcatggcaaccatgaggtcgaagagaccgatggcctcgacgaaagcgaaaccaagaatggcgtaagagaaaagctggccacggagggaggggttgcgggcgacggcctggatgagggcggcgaagacgagaccgataccgacaccagcaccggcaagaccgatggcggcggaacccataccgatgttctgggagacctggacgagggcgttggccatctcagaggagtaggcacgcttggcgatgggggaggcctggcgggccatcatctgggtgcgcttcatggtgttgaagacggtgttcttggggaccgcggagtaggcgcgggtgaacttctggagctgagcagcctggaaggccgggcgggcgaccttcacggaggactgagcggccatggaggccatcttgggggcggcgacgcggaaggaagacattgtgatgatggtgaggtggtgagatggagttgagatgggttgttgatggatttgggatgaaagtgtggtcggatggaagatggtggtgtggagtacgaagagctct

SEQ ID NO: 72 - DNA, 1368 bp, metagenomes purified from environmentally challenged niches
ggaggattctcggtcaagttcaggaccgcagaaggaaattgggactttgtggccaacaacacccccgtcttcttcctccgagacccggccaagttcccccacttcatccacacccagaagcgagatcccgccacccacttgtctggtgacgatgactcgaccatgttctgggactacctgtcgcagaaccccgagtcgatccaccaagtcatgatcctcatgggtgatcgaggtatccccaagggctggcgattcatgcatggctactacggccacaccctcaagattgtcaatgacaagggcgaatgggtctacgcccagttccacctcatctctgatcagggcacccagaacttcacgggtgacgaggctgctcagcaatccaacgattacggacagaaggatctgtacgaagccatcgagaagggagacttcccctcgtggacgatgaaggttcagatcatgaccgagaagcaagccgaggaggcatgggagcaaaagaggatcaacgtctttgatttgacccacgtctggcctcatggtgattacccacttcgaacagtcggtaaattcacccttaacgagaatgccaagaactacttcgccgaggtggaacaagtcgcattcaacccgtctcacatgattcccggtgtcgagccgtccaacgacccagtgttgcagtcgcgactgttctcttaccccgatgctcaccgacaccgaatcggagccaactatcagcaactgcccgttaaccagaatgtgtgccccttcgccttgggcaacttccagcgagacggccagatggcattctacaatcaaggtagtcgacccaactacctttcttcgattgagccaatctcattcaaggagagggcgtatgatctcaacaaggtccacggcaaattcgtcggagaagccgtcgccttcttgtctgaaatcaggccagaggacttcaatgccccaagggcactgtggcagaaagtctttagcgaggaaagcaagcagcgattcgtcgacaccgtctctggtcacatgtcgacagtccgagacaaagccatcaccgctcgaatgatgactatcttccgagaagtttcgcctgatcttggtgatcgacttgagaaggccactggtgtcaagggcgaatccaccattgccgggatgaagttcaacggaacgcacaatgggtttgacaaggccaacaagatcccggctaatgggatgaagaagggtggagaagtcatctttgacaatggtgcacctgctactgctgccaggtaaatgagcggtcaggcgtacttgatatatgttgttacgatatgtcggtctcgtagtcatgtagccaggataaatgaagcggatgtggcagtg

SEQ ID NO: 73 - DNA, 1368 bp, metagenomes purified from environmentally challenged niches
cactgccacatccgcttcatttatcctggctacatgactacgagaccgacatatcgtaacaacatatatcaagtacgcctgaccgctcatttacctggcagcagtagcaggtgcaccattgtcaaagatgacttctccacccttcttcatcccattagccgggatcttgttggccttgtcaaacccattgtgcgttccgttgaacttcatcccggcaatggtggattcgcccttgacaccagtggccttctcaagtcgatcaccaagatcaggcgaaacttctcggaagatagtcatcattcgagcggtgatggctttgtctcggactgtcgacatgtgaccagagacggtgtcgacgaatcgctgcttgctttcctcgctaaagactttctgccacagtgcccttggggcattgaagtcctctggcctgatttcagacaagaaggcgacggcttctccgacgaatttgccgtggaccttgttgagatcatacgccctctccttgaatgagattggctcaatcgaagaaaggtagttgggtcgactaccttgattgtagaatgccatctggccgtctcgctggaagttgcccaaggcgaaggggcacacattctggttaacgggcagttgctgatagttggctccgattcggtgtcggtgagcatcggggtaagagaacagtcgcgactgcaacactgggtcgttggacggctcgacaccgggaatcatgtgagacgggttgaatgcgacttgttccacctcggcgaagtagttcttggcattctcgttaagggtgaatttaccgactgttcgaagtgggtaatcaccatgaggccagacgtgggtcaaatcaaagacgttgatcctcttttgctcccatgcctcctcggcttgcttctcggtcatgatctgaaccttcatcgtccacgaggggaagtctcccttctcgatggcttcgtacagatccttctgtccgtaatcgttggattgctgagcagcctcgtcacccgtgaagttctgggtgccctgatcagagatgaggtggaactgggcgtagacccattcgcccttgtcattgacaatcttgagggtgtggccgtagtagccatgcatgaatcgccagcccttggggatacctcgatcacccatgaggatcatgacttggtggatcgactcggggttctgcgacaggtagtcccagaacatggtcgagtcatcgtcaccagacaagtgggtggcgggatctcgcttctgggtgtggatgaagtgggggaacttggccgggtctcggaggaagaagacgggggtgttgttggccacaaagtcccaatttccttctgcggtcctgaacttgaccgagaatcctcc

SEQ ID NO: 74 - DNA, 1377 bp, metagenomes purified from environmentally challenged niches
ggacaccattgacgcagaggtgctcgacagtttgggtgtcacccaagagaacttccagtttgcccttggcgtcagcaacccctctgcccttcgcgaggtcgcagtggtcgaggttcccaacgtcagatgggaggacattggtggtctcgaggaggtcaagagggagctcatcgagagcgtgcaataccccgtcgaccaccccgagaagttcctcaagtttggcatgtccccatcaaagggtgtgcttttctacggtccccctggtactggtaagactcttctggccaaggctgtcgccaacgagtgcgcggccaactttatttccgtcaagggtcccgagcttctctccatgtggttcggtgagtctgagagcaacattcgtgacatcttcgacaaggctcgtgctgccgcgccttgcgttgtcttcctcgacgagctggactccatcgccaagtctcgtggcggttctcagggcgatgctggcggtgcttccgaccgtgtggtcaaccagcttctcactgagatggacggtatgaccagcaagaagaacgttttcgtcatcggtgccaccaacaggcctgagcagctcgacaacgctctctgccgtcctggtcgtctcgacactctcgtctacgttcccctgcctgaccaggagggccgtgagagcattctcaaggcccagctccgcaagactcctatcgccgacgacatcgacctttcctacatggcctccaagactcacggtttctctggtgccgatcttggcttcatcacccagcgtgccgtcaagctggccatcaagcagtctattgacctggccatccagaaccaaaaggctagagaggccgagggtgacaccgccatggacgaggacatcgaggaggacgaccccgtgcccgagctgaccaaggctcactttgaggaggctatgagcatggctcgtcgctccgtcaccgacaccgagatcaggcgctacgaggctttcgcccagagcatgaagagctccggtggcggcagcgctttcttccgcttccctgagagcggtgccgatggcaacgcagccgagcagcagcaaaatggtgctggcgaggaggacctctacgactaaattggtttcacgaacctcacgacctaatcctttgctgttatcggagtaatattccagatggagagagcaatcatgcattcaggcgcgtctatggactgaaggggaagatggatagagtgttccagtagcccttttctctttttttctgggaactcttgctgtttggctggtcgcctcttatcgagtgtggttgtgctagagtaggcagttcagagtttccctgttatgttatgcctttccgggcagtatgagaataatttccttgcaaa

SEQ ID NO: 75 - DNA, 1377 bp, metagenomes purified from environmentally challenged niches
tttgcaaggaaattattctcatactgcccggaaaggcataacataacagggaaactctgaactgcctactctagcacaaccacactcgataagaggcgaccagccaaacagcaagagttcccagaaaaaaagagaaaagggctactggaacactctatccatcttccccttcagtccatagacgcgcctgaatgcatgattgctctctccatctggaatattactccgataacagcaaaggattaggtcgtgaggttcgtgaaaccaatttagtcgtagaggtcctcctcgccagcaccattttgctgctgctcggctgcgttgccatcggcaccgctctcagggaagcggaagaaagcgctgccgccaccggagctcttcatgctctgggcgaaagcctcgtagcgcctgatctcggtgtcggtgacggagcgacgagccatgctcatagcctcctcaaagtgagccttggtcagctcgggcacggggtcgtcctcctcgatgtcctcgtccatggcggtgtcaccctcggcctctctagccttttggttctggatggccaggtcaatagactgcttgatggccagcttgacggcacgctgggtgatgaagccaagatcggcaccagagaaaccgtgagtcttggaggccatgtaggaaaggtcgatgtcgtcggcgataggagtcttgcggagctgggccttgagaatgctctcacggccctcctggtcaggcaggggaacgtagacgagagtgtcgagacgaccaggacggcagagagcgttgtcgagctgctcaggcctgttggtggcaccgatgacgaaaacgttcttcttgctggtcataccgtccatctcagtgagaagctggttgaccacacggtcggaagcaccgccagcatcgccctgagaaccgccacgagacttggcgatggagtccagctcgtcgaggaagacaacgcaaggcgcggcagcacgagccttgtcgaagatgtcacgaatgttgctctcagactcaccgaaccacatggagagaagctcgggacccttgacggaaataaagttggccgcgcactcgttggcgacagccttggccagaagagtcttaccagtaccagggggaccgtagaaaagcacaccctttgatggggacatgccaaacttgaggaacttctcggggtggtcgacggggtattgcacgctctcgatgagctccctcttgacctcctcgagaccaccaatgtcctcccatctgacgttgggaacctcgaccactgcgacctcgcgaagggcagaggggttgctgacgccaagggcaaactggaagttctcttgggtgacacccaaactgtcgagcacctctgcgtcaatggtgtcc

SEQ ID NO: 76 - DNA, 699 bp, metagenomes purified from environmentally challenged niches
gaaggtgacgacgagcagactttgcgccccacgacgatactaacgtaacgacccagcacacattaatccacaatgggtcactccgccggtctcaggaagggcactcgctatgccttctctcgcgacttcaagaagaggggcatgatccccctctccacctaccttaagcagtacaaggtcggcgacatcgtccacgtcgtctgcaacggtgccgtccagaagggcatgccccacaaggacttccacggcaagactggtgtcgtctacaacgtgaccaagtccgccgtcggcgtcatcctgtacaagcaggttggcaaccgttacatcgagaagcgcgtcaacctccgcatcgagcacgtccgcctctcccgctcgcgtgaggagttcatcgtccgcgtcaagaccaacgctgagaagaagcgcaaggccaaggaggagggcaccaccgtcttcctcaagcgccaggccgacaagccccgcgaggcccgcaccatcagcgccaaggacaacaagcccgagagcatcgctcctatcgcctacgacacccacatttaagcgtgcttgtttcgaaagggagggcgtacgggctggtatgatggcgaggctaggaggttggtatcggcggatcggattccaccggatgggaaatacctgccggatgagccagctagcttcgcaaggtgcatgaattctagcgcc

SEQ ID NO: 77 - DNA, 1664 bp, metagenomes purified from environmentally challenged niches
ggggacatgggcatcggtggtcttgatacggagttctcggctatcttccgacgagcatttgccagtcgtattttcccgccgggactggtcgagaaattaggtatccagcacgtcaagggtatcttactgtttggcccgccaggaacaggaaaaaccttgatggcacggcagatcggaacgatgctcaacgccagagagcctaaggtggtcaacggtcccgaaatcctcaacaagttcgtcggtcagagtgaggagaatatcagaaagctgtttgccgatgctgagaaagagcaaaaggaaaagggggatgaaagtggcttgcacatcatcatcttcgatgagctggacgctatctgtaaacagcgaggatctacaaacagcggtaccggcgttggagactcggttgtcaatcagctgttatcgaagatggacggtgtagatcaactgaacaatgtcttgatcatcggtatgactaatcgaatggacatgatcgacgaagcgctcctccgacctggacgtctggaagtccacattgagatctcgttgcctgacgaagctggccgattccagatcctcaacattcataccaacaagatgaggacgaatggtgtcatggacagcgatgtggatctgggcgaactagcggccctgacgaagaacttctcgggtgccgagattggtggtctggtcaaatcagcgaccagtttcgctttcaaccgtcacgtcaaggttggctccgtcgccgcgtttgatgatatcgacaatatgaagatctcacgagccgacttcctccacgccctagacgaggttacacctgcgtttggtgtctccgaagaagagctgcaacaggtcgtgcagaacggtatcattcactactcgcaacacgtcaatgacacactaaacgatggaagtctgcttgtggagcaagtgcgaaaatccgaccgcaccccgcttgtctcggccctccttcacggtccatctggcgcgggcaagacggctttggcagccacgatcgccatggcatccgagttccctttcatcaagctcatctcgcctgaaacaatggttgggttttctgagccgcagaagattgctcaactcaacaaggtgttcacagacagctacaagagtccgatgagcatcatcgttgtcgacagtctcgagagattgctggactggaacccgatcggacccaggttctcgaatggtgtgcttcaggctttggttgtcctctttggcaaacgtccgcccaagggtcggcgtcttctcattctggccaccacgtcaaatcgcaacatcctcacggatatggacgtcctttcggctttcgacactgatatccccattaaccccatctcatcgatcgatgcagtggtgcacgttctagatgaggtcaagttattcccgaactcgaaggaaaagcagagagcaacacagatgcttcgcgaggcgagactgggcgaaggtggtcgaccagacttgttggtcggagtgaaaaagctgttgagtatggcagagatggcccggcaggatccggatcccacgatgaagatcgtgacgagcattctcagggaggcgagttaggatgtgtgaagcgtgatcatgatagagtgtagtccaaacaatgtactagtgcaacagaagctatgcagatgaataacgtt

SEQ ID NO: 78 - DNA, 1368 bp, metagenomes purified from environmentally challenged niches; identical to SEQ ID NO: 72

SEQ ID NO: 79 - DNA, 1280 bp, metagenomes purified from environmentally challenged niches
gagcacatacacacaccaccgcaatcatgcctccccgccaaccagcaacacggctctttgccctaccgcctcgcttcctctgcccttcgctgcccaccacgcaaacgcgcaccatccgctccatcgacaaacccgccccaaaacccagccgattcaatgcctcactcaatctccccgtgctgggctcctcgtccaccgccgccttcgcgcgcaaagagcactcgctccccctgcgcaccggcgcgctcgccatcaaaaagggcatgacggcactcttcgacccggtcacagcgaagcgcacgccctgcaccgtcctgcaactcgacagatgccaggtggtcagccacaagcgacgcgacatccacggctactgggcggtgcaagtgggcgcgggcgccaaagaagcgaggaacgtcacgcggccggagaggggccacttcgccgcctacaacgtgcccttgagcaggcacctggccgagttcagagtcaagaacgccgagggcctgccccccgttggctcggctattaccgccgacctgttcatcgagggccagttcatcgatgccaaagccgaccgcagaggcatgggtttcgagggtggtatgaagcgctggaacttcggcggacagcccgcgtcgcacggtaactcgctcgcgcacagattgatgggttcgtccggtggtggacagggcagcggtagcagagtcttgcccggcaagaagatgccgggtcgcatgggtggcgagcaggcgaccgttgcgaacctgagggtcatgcaggtggacaaggagaacggtatcgtggttgtgagtggcgctgtgcctggcccgaagaactgcatggtcaagctgcaggatgcgctcaagaagccttggcctgatgcgacttggccgccgtctattgagggcgcgacggaggttctgagggaggccactgagaaggcgcctgctgcgtaagggggtcggtcgaggtcaagaaatatcgttgcaatttgggagatgatgctgtccgatgcctgtcgaaaaggggttcttgtggggaggtctggagaatcatcgatgcaagcattaacatgagcgtgatctcacgagcaatcccagagaagcggttacagctgcttgctcgaaatgtacactgctcaaagcttgccggagaagttggccaaagtcatcactctcggcacaggaatatactttgtaaccatagggaaaagaggagagggtctcgagccaggatcaaaaataggaaatgtacattataattgcatatcgtcatcatcc

SEQ ID NO: 80 - DNA, 677 bp, metagenomes purified from environmentally challenged niches
ggaatcgacgaacgacacctcaatcgaaaccaccactcgccattgtgaatctttccacctgtcgcaatgggtatctgggacgctttcaccgatattgtcgaggctgtgacgccatggagcgtcgttgaggccgaggctcctgctgaggagccccaggaggagaacgagtccaagaccgagtccaaggacgagcccgaggaggaggaagaggatgaggaagaagaggaggatgaggatgatgaggaggagctcgtcgaccccaaggagactctcgaggaagagtgcaagaactctcctcaatgtgcccccgccaagcaccacttcgacgagtgtgttgagcgcgttcagcagcaggagagcgagggtggtgctaaggaggactgtgtcgaggagttcttccaccttgcccactgtgcgaccgcttgcgccgctcccaagctttggtctcagctcaagtaaactcacaacattgggttatcggttactacgacgacgcaatggctacatacacgtcgaaaagatgcctggagccggaacgaggcaatgctgcccactacggaaggctgttcccttgtacgaatgctcatctgccgggtatcaagtcggccagagattactctgatgtcgactctctctgtaccatacgctcttacgcctgaatagatttcttgcacttt

SEQ ID NO: 81 - DNA, 1019 bp, metagenomes purified from environmentally challenged niches
gggagatactaccgtgcgcccgagatcatgttgacatggcaaaaatacgatgtcgccgtcgacatttggagcacaggatgtatcttcgccgagatgctcgagggaaagcccctgttcccgggcaaggaccacgttaatcagttctcgatcatcacagaattgctcggcacacctcctgacgatgtcatccagaccatcgcatctgagaacaccctccgattcgtccagtcgctgcccaagcgtgagaaggtcccattcactacgaaattcgccaatgccgacccgctttcgcttgacttgttggagaagatgcttgtcttcgatccacgtacccgtatctcggcatcagaagggctgtcgcacgagtaccttgcgccataccatgacccgacggatgagcccgtcgctgccgaggtgtttgactggagtttcaacgatgcggatctaccagtagacacctggaaggtcatgatgtactccgagatcctggacttccacaacttgggtgatatccagcaagaccaggccgccgaaggacccgtcactggcgacctagccccaccttccgctacgacttcggcatagacagcttgcctttaggggtttttttctcgtttttctcttctcgtctcattacgttcctagtcaacatgtgtccattagcatcccaaattattggtggtagaaaggagggaaggaattggtgcaacatgatctctcctagaaaatcgtttctcttcatctctcgtccatgatccacgctttcccaagctttatctcccccttccccttcctcacgcctcaacttctcctgtaccaacaaatcttcgctaccgctttctcgaccgtcgaacgaacatcacaaagaatcaagaaaggtagaagaggtgtgaatagaccaggaaaggcattcttggagcgaggggggaggaggaagtaatctggaacgaaagcccatcacactgttttctttgaacctacatacacggacagaggggaatgcatgtgcatggtaatgt

SEQ ID NO: 82 - DNA, 391 bp, metagenomes purified from environmentally challenged niches
cgctaccggtcgccggcgcgccggggttgacctcggatcaggtagggatacccgctgaacttaagcatatcaataagcggaggaaaagaaaccaaccgggattgccctagtaacggcgagtgaagcggcaagagctcaaatttgaaagctggccccctcggggtccgcattgtaatttgcagaggatgcttcgggaacggcccccatctaagtgccctggaacgggccgtcatagagggtgagaatcccgtctgggatggggtggccgcgcccgtgtgaagctccttcgacgagtcgagttgtttgggaatgcagctctaattgggtggtaaatttcatctaaagctaaatattggccggagaccgatagcgcacaagtagagtgatcgaa

SEQ ID NO: 83 - DNA, 391 bp, metagenomes purified from environmentally challenged niches
cgctaccggtcgccggcgcgccggggttgacctcggatcaggtagggatacccgctgaacttaagcatatcaataagcggaggaaaagaaaccaaccgggattgccctagtaacggcgagcgaagcggcaagagctcaaatttgaaagctggccccctcggggtccgcattgtaatttgcagaggatgcttcgggaacggcccccatctaagtgccctggaacgggccgtcatagagggtgagaatcccgtctgggatggggtggccgcgcccgtgtcaagctccttcgacgagtcgagttgtttgggaatgcagctcaaattgggtggtaaatttcatctaaagctaaatattggccggagaccgatagcgcacaagtagagtgatcgaa

SEQ ID NO: 84 - DNA, 124 bp, metagenomes purified from environmentally challenged niches
gggtctggtggcgatagcgagacggccacacccgttcccatgccaaacacggaagttaagcgtctcagcgccgaaagtagttgggggatctccccctgtgaggataggacgttgccaggcaaaa

SEQ ID NO: 85 - DNA, 717 bp, metagenomes purified from environmentally challenged niches
agatggagcctgaccaagaagagtctgaagaggaagaagaggaagaggatgacgagatggatgaagatgaggatgagggccagcagcaggacgccagtggcatgcagacaccctctgggctcgccacgccctcaggctatgcctctactacatctacaatgcctggtggcatggagacgcctgactttatggacttgcgcaagcagcgacagacgcgcgacgagaccgctgatcaagaggaccagggtgcaccgcgagacctctatacggtcgtgcccgagcgcagagccaccgcttctggcttcctcggttctgaccgcgcctatgacttgtccaatgcgccacagtcttccaacatgcctgtgttgggtcaagaagactcgcgcaagaagaaaggcggcagatctggtgcagacgacgtcgacctggccttggatccagctgagctcgagggcatgtctgagcaagagcttaggcagaagtacgactcgcacaggcgctcctcgtccagtcaaggcgccggcggacagcaggacaaagaagatttctcagatttcgtcgcgcaagaggtcgcaaagaagaggcagagggctcagcagcgcggcggcagtggacgcgaccgcgaaagctctcggagcaaggaaaagttcaagttttagagtgtatgtttgtattgtatgaagatcagacaaaaatgctatgggtggcgttgctgct

SEQ ID NO: 86 - DNA, 872 bp, metagenomes purified from environmentally challenged niches
cgtgtagcataaagctagaagtaatattcacagctaactctacagtagaacaaagttcttgtttcgttctccagatccaagtgatagcaactgcttcacaaggatggaagaaccaaattgttgaaagattcggcacctaataggcggcacccatgttgaaatcgtcagtcatgttgaaactccgtaaacccgcttttggtgccctctaatccgcaaaaccttgaaaccctatgttgaacttttggtatcatcttcgtaatcgtcataaaacagaactccccgtgccagaggcggcaggttgagaataccgccccttgaattaacacattataggaagtggaacaaaggaaaaatgagaaatgttaatgcgcacagaattactgagtgtacttctggcggtagaacttagcagcctcgaccagagaggtcagctggccgatagtctgctcagtggtacgggtcttcagaccgcagtcagggttgatccagagctgctcaggcttgaggtactggagcatctgctcgatacgctccttgatctcatccacggagggaacacgaggagagtggatatcgtagacaccaggtccaatgtgggcggggaaactctgatcaacgaagacctggaggagcttggcatcggacttgctgttctcgatggacaaaacatcggtatcaagggcagcaatagcgtggaagaagtcctggaattcactgtagcagaagtgggagtggacctgggtgctgtcggtgacaccagcagtagacagcttgaaagcattgacagcccacttaacataagcatcacgggcagcgccagtacgcagaggaagaccctcacgcagggcaggctcgtcgacttggatgacccc

SEQ ID NO: 87 - DNA, 872 bp, metagenomes purified from environmentally challenged niches
ggggtcatccaagtcgacgagcctgccctgcgtgagggtcttcctctgcgtactggcgctgcccgtgatgcttatgttaagtgggctgtcaatgctttcaagctgtctactgctggtgtcaccgacagcacccaggtccactcccacttctgctacagtgaattccaggacttcttccacgctattgctgcccttgataccgatgttttgtccatcgagaacagcaagtccgatgccaagctcctccaggtcttcgttgatcagagtttccccgcccacattggacctggtgtctacgatatccactctcctcgtgttccctccgtggatgagatcaaggagcgtatcgagcagatgctccagtacctcaagcctgagcagctctggatcaaccctgactgcggtctgaagacccgtaccactgagcagactatcggccagctgacctctctggtcgaggctgctaagttctaccgccagaagtacactcagtaattctgtgcgcattaacatttctcatttttcctttgttccacttcctataatgtgttaattcaaggggcggtattctcaacctgccgcctctggcacggggagttctgttttatgacgattacgaagatgataccaaaagttcaacatagggtttcaaggttttgcggattagagggcaccaaaagcgggtttacggagtttcaacatgactgacgatttcaacatgggtgccgcctattaggtgccgaatctttcaacaatttggttcttccatccttgtgaagcagttgctatcacttggatctggagaacgaaacaagaactttgttctactgtagagttagctgtgaatattacttctagctttatgctacacg

SEQ ID NO: 88 - DNA, 362 bp, metagenomes purified from environmentally challenged niches
gttgacctcggatcaggtagggatacccgctgaacttaagcatatcaataagcggaggaaaagaaaccaacagggattgctctagtaacggcgagtgaagcagcaatagctcaaatttgaaatctggcgtcttcggcgtccgagttgtaatttgtagaggatgcttctgggcagccaccgacctaagttccttggaacaggacgtcatagagggtgagaatcccgtatgcggtcggaaaggcaccctacacgtagctccttcgacgagtcgagttgtttgggaatgcagctctaaatgggaggtaaatttcttctaaagctaaatattggccagagaccgatagcgcacaagtagagtaacc

SEQ ID NO: 89 - DNA, 663 bp, metagenomes purified from environmentally challenged niches
gaccctcactctctttctccctctcttacatagcgagctggtctccatccttgttgtttgatttgatcttctttgcatttccctatcccagtgatgaagttatccaattccgctcattactcgcttttcctcctatcctccatcctcggcttctccagcgcgtcggccaactctcacctcagtgatgattctccttgtgtggcccgctcgccaacaagtgggctctattatgatctgaatgctatctcattagcaccgccggaatggaagaacgggaagaaagttgatcaggaagcgcgagatgaaagctggcatgccaaggggcatgactaccccgcgaacttcacaatcaatgtctgcgcgccggttcttgagaatgtaaccaatgttgtcggggtagatgcctctcgatgggcgaatgtcagtgctttctatgagcaagctgggaagatatactcaatgggagagcaagcctccgagcctttcttccgcggccgcaagctagtactcaactacacggacggttcgccatgtcccggtgattcgaatactgctagcggcaatagctctattcgaaccaagtccactctgatgtccttcctctgcgatcgcgcggccgaattccccgggctcgagaagcttggatccaccggatctagataa

SEQ ID NO: 90 - DNA, 1243 bp, metagenomes purified from environmentally challenged niches
atgtccatccgcaatgaatggcttcaatgagaaaggcctcgacggggatgcctttggagagaagtccaatctctccgggctaaagacatttgacgctttccccaaaacaaaaacatcctacacaaccccaacccgacgaggcggccaatggaccgttctcatcctagcagtatgcacactattcagcctccacgaactccgcacctggtggcgcggcacagaagcccaccacttcagcgtggaaaaaggcgtatcccacgatctccaattaaacctcgatatggtcgttcacatgccctgtgacactctccgcataaacattcaagacgcctccggagaccgcgttttagctggcgaactcctaacccgcgaagacacaaactgggacctttggatgaagaagcgcaatttcgaatcccacggcgaacacgaataccaaacgctcaatcatgaagcggctgatcgattaagtgcgcaggatgaagacgcgcacgtacaccatgtcctgggtgaagtgcgccgtaacccgcgccgcaagttttctaagggtccacgtctacgctggggcgataacaaggattcttgtcgaatttatggaagtcttgaagggaataaagtgcaaggggatttccatattacggcacggggacatggatatatggaattggcgccgcatttggatcacgaagtcttcaatttctcccacatgattacagaactgtccttcggaccacactatccatcccttctaaaccctcttgacaagaccatcgccgaaagcgaaacccactaccagaaattccaatacttcctttccgtcgtcccgaccctctactcaaagggccacaatgcacttgacctcgtgacaacaaataaagataactccgtccgctacggccgtaacacaatcttcacaaaccaatacgcagccacaagccagagtaccgccctccctgaaatccccaccctaatcccgggaatctttttcaagtataatatcgagccgatcttgctacttgtcagcgaagagcggacgggattcttggctcttgtcattcgagtcattaataccgtttctggggtcttggttacgggtggttggatctaccagatttctgggtggattgttgagatccttgggaaaaggaaacggcagtctgagggtgttttgactgggaagcattattcggattgatttgtttctagtagtttcgtctcaatataagtttgattttccttttcc

SEQ ID NO: 91 - DNA, 1007 bp, metagenomes purified from environmentally challenged niches
gaacggtgatagtagtagtaggctcgtcatctatctacaacccctctctcctcactcccctctctcgacgccatgttcacgcgtactctccgaccggccgtggcggtcgccaggactcaggctgtccagcagcaacaggccggtatggccacattgaaggaaatcgaccagcgtttgaaatccgtcaagaacattgggaagatcaccaagtcgatgaaggtcgttgcctcgaccaagttgacgcgagctgagaaggccatgcgtgaagccaagaagtacggtgccgccaacaacgttctgttcgagcagaccaaggctggtgaggaggagcccaaggagcgcaagatcctctacctcgccatgacatccgacggtggtctgtgcggtggtatccactccaacattacgcgatacatgaagaaggctgtggccaaggaacccggaatgctggctgttgtcggtgacaagcccaaggctcagctctctcgagcgatgcccaaggctttgaccatgtctttcaacggcgtcggcaaggatgtccccactttcgtcgaggccagcgctatcgccgatgagattatgaaatctgccggtgactttgacgagatccgaatcgtctctaacaagtacctttccgctatcgcctacgaacctcacaccaacgccgtcatctccgctgaggcactccgacaagccgccggtttccagcaatacgagatggaggaggatgtctccaaggacttggccgagttcgctcttgccaacgccatctacactgccctggtcgagggacacgccgccgagatctctgcaaggaggcaagctatggagaacgcttccaacaacgccaacgacatgatcaactctctccagctgcagtacaaccgtggtcgacaggctgtcattaccaccgagctgatcgatatcattaccggtgcctcggctctgtaagcgggtgtagactagatggacaaaacaacaaaaatggcatgcagcgaatgacattg

SEQ ID NO: 92 - DNA, 1007 bp, metagenomes purified from environmentally challenged niches
caatgtcattcgctgcatgccatttttgttgttttgtccatctagtctacacccgcttacagagccgaggcaccggtaatgatatcgatcagctcggtggtaatgacagcctgtcgaccacggttgtactgcagctggagagagttgatcatgtcgttggcgttgttggaagcgttctccatagcttgcctccttgcagagatctcggcggcgtgtccctcgaccagggcagtgtagatggcgttggcaagagcgaactcggccaagtccttggagacatcctcctccatctcgtattgctggaaaccggcggcttgtcggagtgcctcagcggagatgacggcgttggtgtgaggttcgtaggcgatagcggaaaggtacttgttagagacgattcggatctcgtcaaagtcaccggcagatttcataatctcatcggcgatagcgctggcctcgacgaaagtggggacatccttgccgacgccgttgaaagacatggtcaaagccttgggcatcgctcgagagagctgagccttgggcttgtcaccgacaacagccagcattccgggttccttggccacagccttcttcatgtatcgcgtaatgttggagtggataccaccgcacagaccaccgtcggatgtcatggcgaggtagaggatcttgcgctccttgggctcctcctcaccagccttggtctgctcgaacagaacgttgttggcggcaccgtacttcttggcttcacgcatggccttctcagctcgcgtcaacttggtcgaggcaacgaccttcatcgacttggtgatcttcccaatgttcttgacggatttcaaacgctggtcgatttccttcaatgtggccataccggcctgttgctgctggacagcctgagtcctggcgaccgccacggccggtcggagagtacgcgtgaacatggcgtcgagagaggggagtgaggagagaggggttgtagatagatgacgagcctactactactatcaccgttc

SEQ ID NO: 93 - DNA, 1139 bp, metagenomes purified from environmentally challenged niches; identical to SEQ ID NO: 46

SEQ ID NO: 94 - DNA, 526 bp, metagenomes purified from environmentally challenged niches
aacccaccccgccattctcaattcttcgtccgtgttcttctcgagaagctacacttcgcaaaaatgggtgccattccggaatatgatcccgaggagcccctcgagaccaagcccttcaagttcgtgactgctggttacgacgctcgtttcccccagcagaaccagaccaagcactgctggcaaaactacgtcgactactacaagtgtgtcgaggccaagggtgaagacttccgcccctgcaagcagttctaccacgctttccgctccctctgccccaaggcctggactgaccgctgggacacccagcgcgagggtggtaacttccctgctatccttaacaaatagataaccaatggctgctttgtgttggtgaattgggttatagcagattctgtattgacaaactttccaatgtactctacctggtcatgcggggatacatttcttttctgtttggatgtaattttcccactctgatgaagaaagtgtgtctataaactcgctgttttgaaactaaacgtcttcc

SEQ ID NO: 95 - DNA, 839 bp, metagenomes purified from environmentally challenged niches
gggccattgctcgaggagctcgatgtcgaggcgtacgccaagaagtaccgttacctgagattcatgtgccaggagacgctggaccatctcgcctttctcaaggacaaagtgaaggatgtcgaagggttctgggcatccaccttgttgaagcaccgcgatctcaggggctacatcacttcacgatccgacaaggacgcattgaagtacttgactcacattgagctcgttcaggatcccaaggatccccgtccgttcgctctcaaattctacttcaaggagaacccatacttctccgacttggtcttggagaagaagtacgatatgtccgagggttccgaacccgcacctgccgatggtagcattacggagggaatgcgcaatttcaaagaagacgagctggtcaccaaggctaccacgatcaactggaagtcggacgacaagaatctagtcgccaagcagcccagatccaaaattcccgacaatgacgacgatgaagatttcgacggggacgtcggatcgttcttcaactactttacagatgacacagatattttccagattggggccctcctgcagtcggagctactgcctgatgccatcgactactttgttggccgaggcgagcaggtggactctgaaggagaggagctagacgagctggaagaggatgatgaagacgacgatgaggatgatgagggcagtatcgacctcgaagacgaggaggagcagccgagtaaaaagaagcccaagagggcctaagaaacatttgatccgtcaacatgtacggacgaggtaatcgtgttcgaatgttaatgatcatgcatatgctagtaaattcg

SEQ ID NO: 96 - DNA, 804 bp, metagenomes purified from environmentally challenged niches
ggatctttcctcacccctcaacacactcacacaccattcggacgcgctatgcacaatgccttgacggtttcgaggctcaacgacaagttccaagagccgctcgttgttcttgtggagcttttgcgtgctcgtgttctgcacgaccgcaacttctcgaacagacaattctcaggtggtccttcattcgggacagacaatcagaagagaagcatgcttttgatcttccgtactctgtccattattccgctccaattcaaggccgagcactggtcaggaccattgtcaagagagctgcttgtcttcaactcattccacaagacactgtcaagatccctgagaacgctggtcgaatcaatcactatgaacgccttcctcaagaacaatgcgagaagagcacgtgacgactatcttgacattgcactttcactaccattccaaaacgataccaacactggattcggtatcttctttaagatttacttggatgcattgactacatttgcagaaggcaacatcactgaagagaacaaagacagcgagtctgtgaaagaggccaagcagtcagcaatggagatcctaggtgacgccataccgaacgtgaaggacccagaggccgagcttttgcggggtttcagattctgggatgctgtgctcgtgtgcgtccgtacactcaaagcagacagggcaatcgatctcaagctagctgagtctttcgaggcggcaaacagctaccttaatatgatgagaccaaattgatacggcgttttgtagcaatcttgagctttatgcaatctacttctgtcg

SEQ ID NO: 97 - DNA, 848 bp, metagenomes purified from environmentally challenged niches
ggatctttcctcacccctcaacacactcacacaccattcggacgcgctatgcacaatgccttgacggtttcgaggctcaacgacaagttccaagagccgctcgttgttcttgtggagcttttgcgtgctcgtgttctgcacgaccgcaacttctcgaacagacaattctcaggtggtccttcattcgggacagacaatcagaagagaagcatgcttttgatcttccgtactctgtccattattccgctccaattcaaggccgagcactggtcaggaccattgtcaagagagctgcttgtcttcaactcattccacaagacactgtcaagatccctgagaacgctggtcgaatcaatcactatgaacgccttcctcaagaacaatgcgagaagagcacgtgacgactatcttgacattgcactttcactaccattccaaaacgataccaacactggattcggtatcttctttaaggttggtggccttgcaggagtctgacatagcgctgacgcagacagatttacttggatgcattgactacatttgcagaaggcaacatcactgaagagaacaaagacagcgagtctgtgaaagaggccaagcagtcagcaatggagatcctaggtgacgccataccgaacgtgaaggacccagaggccgagcttttgcggggtttcagattctgggatgctgtgctcgtgtgcgtccgtacactcaaagcagacagggcaatcgatctcaagctagctgagtctttcgaggcggcaaacagctaccttaatatgatgagaccaaattgatacggcgttttgtagcaatcttgagctttatgcaatctacttctgtcg

SEQ ID NO: 98 - DNA, 628 bp, metagenomes purified from environmentally challenged niches
ggggcatctacctcgacggcaacaacgacctggtcactatgaagggtaactacatctaccacaccagcggccgctctcctaaggttcagggtaacaccttgctgcacgctgtcaacaactactggcacgacaactccggccacgccttcgagatcggtgagggtggttacgttctggccgagggtaacgtcttccaggatgttactacccccgttgaggaccccgttgacggccagctcctcacttcccctgaccccagcaccaacgctcagtgctcgtcataccttggccgggcctgcgaaatcaacggcttcggtaactctggtaccttcaaccaggctgacactagcctgctgtctaaatttaagggtcagaacattgcttctgctgatgcttactctaaggttgcctcgagcgttgccagcaacgccggtcagggacacctgtaaaatggaaagaggaggttcagagcttaatttgctcatgtcggacgacatagccctagcggcttgctggtgaatttggcataatagcgtttctcttctcatacctactttattactccgtttggatccttattaggtaaatattagcccattgtatggttcaattcgattgactttgaggc

SEQ ID NO: 99 - DNA, 804 bp, metagenomes purified from environmentally challenged niches
agttggaaatctgatcaattactctccatcttctcgttctactatctaatcctctcttccttccaaaacatatcatcatgtctgctcaacctctccgcattgtcatggcctgtgacgaggctggtgttccttacaaggatgccatcaaggccgttctcgagaagagccccctcgtcgcctccgtctctgacgtcggtgtcaacgatgcctccgataagaccgcctacccccaccccgccgtcgagggtgctcaacagatcaaggccggtaaggctgaccgtggcctcttcatctgcggtactggtctaggtgtcgctatcgccgccaacaaggttcccggtattcgtgccgttactgcccacgaccctttctccgtcgagcgttccattctgagcaacgatgctcaggtcctctgcatgggtcaacgtgtcattggcgtcgaacttgcgaagaagcttgccctcgattggctcaactaccgtttcgatcctaagagtgcctctgccgcgaaggtccaggctatctccgactacgagaccaagttcgctggctcttcttaaatgcattatcttgcatgaatgacggtcttcgtacatactttgccacatatgggttctaattgcactgcgtctgcagtctcgatatgaaaccattggattgcgatggatgtcccttttccatttgcaactttttatatactttcttttctaccaagcgcttcatgataccacgattcgattaccgagttctgctgtttgctttggtcggtagatctagatacacaatgcagtatattcgagtttc

SEQ ID NO: 100 - DNA, 782 bp, metagenomes purified from environmentally challenged niches
acttctccttttctgttagctttgactctactatcctgctcctcctctaaatccgtggaatccaattttttcacaataacttcgctaccataatgtccgtcactaccacttcctccgccgccgcagcctcctgcactccctcttggcagattcctgtcgacgatgttgcctgtgccggtcagatcagcggtaatatcaccaaggttttcgatacctgctgtaagggaaacagccctgtcaagtacaacgacgactgcaacatctactgtcttgcccaaggacaaaccaagcaagagttgaccgactgtttgaccgagaagagcggaaacaaccagatcttctgtggtcatggcaagcagaatgccactgctacagctgaagccaccaccaccaaggagactggcacatcgaccggcacttcaacctcttccactggcacttctaccgagaccaacgctgccgtgctcaaccaacccatctccaagaccggtcttggactcgtcgccatgctcttctgctctgccctcgttggtgttgtcgcctaagttatgactccaaaacgaacacattactgcggtatggatacggcaattatgacaaccagaggaccgcagggacggagaatggtaattgatgaacccggaaaagatacgtggtgcatggacataaatgtttgatttactcttactgtctgcttcaactttccgagaggaatattgtttcttctgtaccaatagcgatagcattaacagcatcttaattctaattttgcatatcacttc

SEQ ID NO: 101 - DNA, 693 bp, metagenomes purified from environmentally challenged niches
gccggggtcgatcgaggtgtcatcaccaaggacgagaaggacagcagtatcaatagactactcgtcactggttacggtctggccgaggtcatgggtacagatggtgtgaacggcatcaagacgcgaaccaatcacgtcatggagacgtgcgaggttctgggcatcgaagccgctcgacagaccatctacaacgagattcagcataccatgacatcgcacggaatgtcaatcgatcctcgacacgttatgctgctcggagacgtcatgacttacaagggcgaggtgctcggtatcactcgattcggtgtgcaaaagatgaaggactcggttctcatgttggccagtttcgagaagaccactgatcatctgttcgatgcctcgctgttttcgaaaaaggatgaaatccaaggcgtctccgagtgtatcattatgggcacacccgcgccaggttgtggcacctcacttgcatcgatcgtcacacctgcccctctcctcccacgcaaaaagcctttgctgtttgaaacagcgttcaaagctggtcaggatcgattgagctatcacgaaaacaatggcggcatggaggtggacatgtgaacccggtccctcatacatcttcttctgattgtctgtaccatacatacatcgcattgcttcttttcacatacgacacgacatgcatctgacatctacgac

SEQ ID NO: 102 - DNA, 776 bp, metagenomes purified from environmentally challenged niches
gcaggatcaggaggagcatattccttctctctgaccaccttctcgccttctggaaagcttgtccagatcgaacatgcattggcagcagtagcgggtggaacaacatcactgggtatcaaagctaccaacggtgttgtccttgcgactgagaagaagtcaccgtcactcctgctcgatacgtctgttctcgaaaaggtagctcctatatgtcccaacattggtttcgtctactcgggtatgggacccgatttccgagtcctggtcgccaaagctaggaagatcgcccaagcgtactataaagtgtatggcgagtacccacctacaaaggttctagtgcaggaggtggcgggcgtgatgcaaaaggctacgcaatctggtggtgtgcgaccatatggtatctccctcttgatcgctggttgggattcgcaccgaggtcagagcctgtaccaagtggatccgtcaggtagctactgggcgtggaaggcaagcgcgatcggcaagaacatggtcaacggaaagacattccttgagaagcgatacaatgacgacctgtcactcgaagatgccattcacacggcccttctcacgctgaaagaaggtttcgagggacagatgactgagaacacgatcgagatcggtgtagtgacggtaccgacggccgagcagatgcaggagaagccaggagagaggctacctcccacgttcaggaagttgacggagcaggaagtgagggactatctcgccttgtagacgatgcagacagaacatgaccatcc

SEQ ID NO: 103 - DNA, 1191 bp, metagenomes purified from environmentally challenged niches
aagtctacgactcctccagccaatttactttgatccaaaatgttgaccagcgccttttctacatctgcttccaagatgctcggcaagagagcagtctcgtcttccagcgccttgaacggaaaggttgccgtcctcggtgctgctggcggtattggccagcccctctccttgctggtcaagcagaaccctgctgtctccagcctctccctttacgatgttcgcggctcccctggtgttgctgctgacattagccacatcaacacccctgctgtcaccgagggcttcctccccgacaacgatggcctcaagcaagccctcgagggtgctgaggtggtcctcattcctgctggtgttcctcgcaagcccggcatgacccgtgacgaccttttcaacaccaacgcttccatcgtcaagatgcttgctgaggcttctgccaagtactgccccaaggctatgatgctcatcattgccaaccccgtcaactccaccgtgccgatcgtcgctgagaccttcaagcgtgctggtgtctacgaccctgcccgtctcttcggtgtcaccaccctcgacgttgtccgctcttccactttcgtctctggcatcaccggtgccaagccctccgacaccgtggtccaggtcatcggtggtcactctggcgccaccatcgtgcccctgctctcccagatccctcagggcgacaagattgtcaaggctggcggccagcagtacgctgacctcgtcaagcgcatccagtttggcggtgacgaagtcgtcaaggccaaggacggcactggctccgctaccctctccatggcttacgccgctgccgtcttcaacgacgctctcctcaaggctatggacggccaaaagggtctcgttcaacccgcttacgtcgagagcccccacttcgccaaggagggtgctaagtacttcgcctccaacgtcgagctcggccccaacggtgttgagaagatcctcgacatcggcaacatgtcctctgaggagcaggagctccttaaggagtgccttccccagctcgccaagaacattgctgctggtgagaagttcgtcgctgacaactagaggatatcccacgacgttgctccctataataatgagagcaagcgagaacaagagaaataaagacatagcaaattgaatagggcttccaactgcaccaaaaagcagtgatgc

SEQ ID NO: 104 - DNA, 1191 bp, metagenomes purified from environmentally challenged niches
gcatcactgctttttggtgcagttggaagccctattcaatttgctatgtctttatttctcttgttctcgcttgctctcattattatagggagcaacgtcgtgggatatcctctagttgtcagcgacgaacttctcaccagcagcaatgttcttggcgagctggggaaggcactccttaaggagctcctgctcctcagaggacatgttgccgatgtcgaggatcttctcaacaccgttggggccgagctcgacgttggaggcgaagtacttagcaccctccttggcgaagtgggggctctcgacgtaagcgggttgaacgagacccttttggccgtccatagccttgaggagagcgtcgttgaagacggcagcggcgtaagccatggagagggtagcggagccagtgccgtccttggccttgacgacttcgtcaccgccaaactggatgcgcttgacgaggtcagcgtactgctggccgccagccttgacaatcttgtcgccctgagggatctgggagagcaggggcacgatggtggcgccagagtgaccaccgatgacctggaccacggtgtcggagggcttggcaccggtgatgccagagacgaaagtggaagagcggacaacgtcgagggtggtgacaccgaagagacgggcagggtcgtagacaccagcacgcttgaaggtctcagcgacgatcggcacggtggagttgacggggttggcaatgatgagcatcatagccttggggcagtacttggcagaagcctcagcaagcatcttgacgatggaagcgttggtgttgaaaaggtcgtcacgggtcatgccgggcttgcgaggaacaccagcaggaatgaggaccacctcagcaccctcgagggcttgcttgaggccatcgttgtcggggaggaagccctcggtgacagcaggggtgttgatgtggctaatgtcagcagcaacaccaggggagccgcgaacatcgtaaagggagaggctggagacagcagggttctgcttgaccagcaaggagaggggctggccaataccgccagcagcaccgaggacggcaacctttccgttcaaggcgctggaagacgagactgctctcttgccgagcatcttggaagcagatgtagaaaaggcgctggtcaacattttggatcaaagtaaattggctggaggagtcgtagactt

SEQ ID NO: 105 - DNA, 1505 bp, metagenomes purified from environmentally challenged niches
ggggcaagcgtgctgcttccggcactgcatttcgacgagcgggagcaacgacctggacgtacgtcttcgactgcaagtctgctgcagcgtcacgatcgcaatgaacctttatcgctcaactcgcactcgccgacatctgtggaccacactcccactactgcgcatttcactggtgctgaagagttgctcgcctccgacgtcggaccgaccgcgacagctgggctacccggtgatgcggagcttgagagcaagctcaagctgcttgaagaggtcaaacgtgcacgggaatcggtacatagctcgctcgagaggatcagagccggcacgcctaccccgtctatcagccagggaatgcccagcccgacaccctctggtgcccctggttacgctagaactccgtcgtctgtcggcctgtcggacgacgtgcgctcgagacgaggctcaacgaccagctccaaggttcttgacgctatcgacaagcctcgagtcgctacccaatccgaatgggacgagtacgttcgcaaccggcatgtcatctcacctccacccactcagtttgccgtattgcccacatctgctgcgatggtcgatcgtggtaccagtcgacacagccagtatgcccttgtttccgacggcgttgccaaagcgcttgacaggcgggagcgaactatttcaatgatggagccgcaagttgccgaggactggggaccaagagagacgctcgacagcactccggctcatgtctcgatgggccgtcgagccatgtcattccatgagatacctctggcatcgcctgtcgctgcctctcgacctcaggaccgctcctcctactctgccggaccacgtcaggtcatagggtcagctgctggccacacgcagcgaccgggtatcagtcaatcgagatcagcccacggccggactatgacatacgacgagctgacggagagacatcgtcagcgcttgtcggcattgcaagcgccagtcagcgccaaaatcagggagccgatggacatcgcgtccgccaaagccagctgggacaagcaaaagcgggtcgagcgggacgaaatgaagaggcgagaagccgagaagctcgctcaggctcacgcaagagagcgacgagggcccgctgtcgacaagaaggaagttctcaagtcgaccgacgaatggaggcgaagcgtccacggcggtctcgacggtttcgccgttccgcacctaccggcccacgctcgaggttccacgcagcctggtggatccggcgccaagcgatcttcactctctcaaaggcccagcaactacttcgccaactaggcataatcgaatcgcggacagtcatctgtacatagaaccgtacctgtattaccaaccctgcacttccgctcacacctgttgcctatacctcgtctaccaacgctcattccaatatcatagctacattcatttgcaaggacactatcacaccgcagtcatgactccgtatggatattcaatgcatacctcttccagag

SEQ ID NO: 106 - DNA, 1391 bp, metagenomes purified from environmentally challenged niches
aacctcggccgagaggacaagattatcaagaatgggatctcctgcgcctcaccaccgccatcaatcctcacttgaaggagtcattgacttttctactggtagagggcatccattgaatccctatcaacgcgacaaggccgagagcgtttttactggcattatcaaccgcttcgaggactcgtcgaccgtagagaaaccatacaaccgtgccaagctggttcgcctgacgtatgagtatgctcgctcggaagattctcgatgcaatttcttgcaagcattcttcggatcagtaaacgttacgatggatgactctattgatttcgacgatgaagcggtagaagaggggattcgctcgagcctgaattccttcgcagatttcttggtggagaacttcttccttccactcaaggcttccgccagcaggacgcccccagccccccagcccaagttccgagcagacgtcctgctgtggggtctgtggaaagagtggcctcgctcagacgcgactgcctcatccgcgatcgacatcgttgcgtaatctctcgcaacttcgacatgaaagaagctgagcgacgtcttgacgatagcggatatgaccatgcctcggacgatgaaggacatttactgaaagatcaggagcatgggtcattcgcggaactagaagttgcgcatatacttcctcactcattgatgactacgacagcgaactccgagctgaacaagtccaaagaaacggcattgacaatacttaatatgttcgacagtggcattgtccatctaatcgacggtccagacattgatcgccctcgaaatgctcttaccttaagcattgacctccatcgacagtttggcaacttcaaggttttttttgagcctatgcctgagccccatacctaccggattgattcaaccctccgccagccatttagaaacccgattttccctgtaacccgtgcactctacctcacccctgagcgaactattgatcccccgtccggtcgacttcttgccgttcatcgcgcaatttgccacattttacatctcagtgctgctgggaattacatcgacagcatacttcgcgacatggatgacgggactgtacaagccaacggctcgactcgcctggctagcatagttcgtctgaaactggggggttggtgggatggcactgttgttggatagtcaaccacttcgaccctctccatacaccacaacggcaactcgagctgatgcatcaccgatctacctacgccattcgcgtggaggattgtcgcatatcaccactaggttcgtgcgactggatatgaaacgcggcccgtactttggggtcgtgtatccggtttcacatccagcttgtcgcatcaaggattccaatcctaacgacatgagcc

SEQ ID NO: 107 - DNA, 665 bp, metagenomes purified from environmentally challenged niches
ggacgaccgaaataccgtcaaaatggtcaacatcccgaagacgcgcaggacctactgcaagggcaaggaatgcaagaagcacacccagcacaaggtcacccagtacaaggctggcaaggcctccctcttcgcgcagggtaagcgtcgttacgaccgtaagcagtccggttacggtggtcagaccaagcccgtcttccacaagaaggccaagaccaccaagaaggtcgtcctcagattagaatgcacttcgtgcaagaccaaggcgcagctcgctctcaagcgctgcaagcacttcgagcttggtggtgacaagaagaccaagggtgccgctcttgtcttctagatgggtgcataacggttatggcgctagggatgatgatggagcggtctgtgcatgtagcctccttgagtacatgatcctcgagggctcggaatcaaagcttcgtttctcctacgatcgtcccactcgcaaagacatgtctcgtcatatcatggcttgcgcacaacattcttcgagggtccatcagagatgcccgaccctgccgctacgctgcgtgggatgtgactccagcacaaccgccttccagtatcatctcttcgcgtgcagaagtgaggacgattttacgacagtccatataacaaatcggaaatgccaacaagatcaa

SEQ ID NO: 108 - DNA, 1327 bp, metagenomes purified from environmentally challenged niches
ggcccctcttgaactttggactttttagcatctattttctctacttctctctccctcctcctatctaccttctctatcatctccttcagctccctacaacatgaagctcacctttaaggacctgaagcaggagaagttcgtaatcgaggtcgagccctccgagactgttcgcgaagtcaagcaaaaaattgctcaagaaaaaggcgaatatgaggcggaacgaatgaaagttatctactcgggcaagatccttcaggatgacaagaccgtcgaatcatacaacatccaggagaaggatttcctagtctgtctgccttcaaagggtcctaagcccgctgcctcgtcgtctgcctcccaggcacccgccactccggcccctagagctcctgttgctactcctgctgctcctgcccccgctgctcctgcacctgctagttctacgcctgctgtccctgcgactccctcgcctgctggcgcccagaccggtccctctttcggtgacccatctgcattgaccatgggttctgcggctgagggtgccgtcactcagatggaagcaatgggatttgccagaagcgatattgaccgggccatgcgggctgcattcttcaatcctgaccgcgctgtcgattacctcttgaacggtattcccgccgatgttcaacaggaacaacagcagcggcaacaagagcaacaagcggaccgtgctgcagaacaagctcctgtgcccagcgctgaggatgctgctgctgccgccgctctgggtggcgatgagggttttaacatgttcgaggctgccgctcaggctggtgatggtcgtggtggtggtgctcggtctggaggtagcgaggcccttgcgaacctggactttctccgcagtaacccccatttccagcaactgagacagttggtccagcagcagccgcacatgctcgaacccatcctgcaacaggttgctgccggaaacccacagatttcccagatcattggccaaaactctgaacagtttctccaactgctaagtgaggagggtgatgaggaagatgcggccctgcctcctggtacacaagctatctccgttacagaggaggagcgggacgccattgagcggttgtgccgtctgggtttcccccgggattccgtcatccaggcctacttcgcctgcgacaagaacgaagaactcgcagcaaacttcctcttcgaccagccggacgatgatgaggagtaaatctgatccacgatgctgtggttcacttctttactccatgtcttatccccttccccttttgcttctttacgttctgatgaataccaagcatgcctgttg

SEQ ID NO: 109 - DNA, 1326 bp, metagenomes purified from environmentally challenged niches
ggcccctcttgaactttggactttttagcatctattttctctacttctctctccctcctcctatctaccttctctatcatctccttcagctccctacaacatgaagctcacctttaaggacctgaagcaggagaagttcgtaatcgaggtcgagccctccgagactgttcgcgaagtcaagcaaaaattgctcaagaaaaaggcgaatatgaggcggaacgaatgaaagttatctactcgggcaagatccttcaggatgacaagaccgtcgaatcatacaacatccaggagaaggatttcctagtctgtctgccttcaaagggtcctaagcccgctgcctcgtcgtctgcctcccaggcacccgccactccggcccctagagctcctgttgctactcctgctgctcctgcccccgctgctcctgcacctgctagttctacgcctgctgtccctgcgactccctcgcctgctggcgcccagaccggtccctctttcggtgacccatctgcattgaccatgggttctgcggctgagggtgccgtcactcagatggaagcaatgggatttgccagaagcgatattgaccgggccatgcgggctgcattcttcaatcctgaccgcgctgtcgattacctcttgaacggtattcccgccgatgttcaacaggaacaacagcagcggcaacaagagcaacaagcggaccgtgctgcagaacaagctcctgtgcccagcgctgaggatgctgctgctgccgccgctctgggtggcgatgagggttttaacatgttcgaggctgccgctcaggctggtgatggtcgtggtggtggtgctcggtctggaggtagcgaggcccttgcgaacctggactttctccgcagtaacccccatttccagcaactgagacagttggtccagcagcagccgcacatgctcgaacccatcctgcaacaggttgctgccggaaacccacagatttcccagatcattggccaaaactctgaacagtttctccaactgctaagtgaggagggtgatgaggaagatgcggccctgcctcctggtacacaagctatctccgttacagaggaggagcgggacgccattgagcggttgtgccgtctgggtttcccccgggattccgtcatccaggcctacttcgcctgcgacaagaacgaagaactcgcagcaaacttcctcttcgaccagccggacgatgatgaggagtaaatctgatccacgatgctgtggttcacttctttactccatgtcttatccccttccccttttgcttctttacgttctgatgaataccaagcatgcctgttg

SEQ ID NO: 110 - DNA, 1162 bp, metagenomes purified from environmentally challenged niches
gcgccgggggacatggagactgccgacgccaagaacagggctatgcgagccgctggcttcatcgttcccgacaccttcgaagacctgcccgaggtcctcaagaccacctacactggtctggttcaaaagggtgtcatcgttcccaaggccgagatcgacccacccaacatccccatggactaccagtgggcttccaagttgggtcttatccgaaagcccgccgccttcatctcgaccatctcggacgagcgaggtcaggagttgatgtacgccggtatgcgaatctccgacgttttcaaggaggagatcggtatcggtggtgtcatctccctcctgtggttcaagcgacgattgccacctttcgcctgcaaattcatcgagatggttctgcaattgactgccgaccacggacccgccgtttcgggtgccatgaacaccatcatcaccgctcgagcaggcaaggacctgatctcgtccctggccgctggtctcttgaccatcggtgaccgattcggtggcgctctcgatggtgccgccgccgagttctctcgaggtctcaactctggtgctaccccacgagaatttgtcgactcgatgcgaaaggccaaccgattgattcccggtatcggacacaagatcaagtcaaagaccaaccccgatctccgagtcgttctcgttgtcgattacgtcaagaagcacttcccgtctcacaagacgctcgactttgccttggccgtcgaggacgtcacgacgcaaaagtccaacacgctcatcttgaacgttgatggtgctattgccgcttccttctgtgatttgcttagcggttgcggtgctttcactgaggatgaggctgccgattacctcaagaacggtactcttaacggtcttttcgttcttggtcgatcgatcggtttcatcggtcactacctcgaccaaaggctcctcaagcagcctctctaccgacaccccgccgacgacattttcatcaacatgcaagagcgagttgtcttccagcctgggtccaactaagaggcgaccgcgactacgggtctcggccaatttctcccttgggtttcctccttcaattaaaactactgtacataccacccacatcatttatctcttctttcatgactatagacgcatgcacgggatcgctcgg

SEQ ID NO: 111 - DNA, 965 bp, metagenomes purified from environmentally challenged niches
ggggcatacaaggagggcaagttcaccagcgaaagcatccaaaagtcaaagctcagattccaggacatcctcgttgagctgcccctcagggttcacaactcccaccttctcaccagcttcctgcaccaggtcccgcaggcgccgccggcaaagaaccccctcgacttcccttcatcccttgcagagctttcgcgcgactccgatgtcagctccaaccccttcgcacccaaccttgacaccctggacctcagcatcgaccccttccagtactggcagcgcgccctcggccgcgagcagcagaagatcaccgcatggcaacagaagcgcaaggctgagaatgctgcacgcgccgcgagcaagcagccgccccttgacgagaatgagtggcagaagctgttcaagctgcccacggagcccagcaggctcgaggctctgcttgtcggcaggcaggtcgagcagtacgcccgccaggtcgacggattctccgccaccgtttccgccaagatgtttggcgtcaggggcaacctcctccctaacgagatcgagtagaggacgaatattacggagacgggaccggcgtttatgcatagcgaggcgttctcggctgggtggggtagagtacatgcggcatggctacaaaaaaaaggatgatgtggttccgccatcgacgagttcagggcaacgctgcatagaatcccaaaagaagaaaggattttaacgtttttgaatttggaacttcttcgcattggacgattgctttcttgacgactccgtcagttgcgcgctttttccatggcccataccctctttatctctaatgagggtgcgccaccgcagacccaccagctactcgaagaaaagtcgctattttttatttggagttattagcgagtacaaacggaggcatgtctagaggctgaggagtgtggtagtaagattatagatgtctttatgctcgatatgag

SEQ ID NO: 112 - DNA, 965 bp, metagenomes purified from environmentally challenged niches
ctcatatcgagcataaagacatctataatcttactaccacactcctcagcctctagacatgcctccgtttgtactcgctaataactccaaataaaaaatagcgacttttcttcgagtagctggtgggtctgcggtggcgcaccctcattagagataaagagggtatgggccatggaaaaagcgcgcaactgacggagtcgtcaagaaagcaatcgtccaatgcgaagaagttccaaattcaaaaacgttaaaatcctttcttcttttgggattctatgcagcgttgccctgaactcgtcgatggcggaaccacatcatccttttttttgtagccatgccgcatgtactctaccccacccagccgagaacgcctcgctatgcataaacgccggtcccgtctccgtaatattcgtcctctactcgatctcgttagggaggaggttgcccctgacgccaaacatcttggcggaaacggtggcggagaatccgtcgacctggcgggcgtactgctcgacctgcctgccgacaagcagagcctcgagcctgctgggctccgtgggcagcttgaacagcttctgccactcattctcgtcaaggggcggctgcttgctcgcggcgcgtgcagcattctcagccttgcgcttctgttgccatgcggtgatcttctgctgctcgcggccgagggcgcgctgccagtactggaaggggtcgatgctgaggtccagggtgtcaaggttgggtgcgaaggggttggagctgacatcggagtcgcgcgaaagctctgcaagggatgaagggaagtcgagggggttctttgccggcggcgcctgcgggacctggtgcaggaagctggtgagaaggtgggagttgtgaaccctgaggggcagctcaacgaggatgtcctggaatctgagctttgacttttggatgctttcgctggtgaacttgccctccttgtatgcccc

SEQ ID NO: 113 - DNA, 1160 bp, metagenomes purified from environmentally challenged niches
gacttcggcgaaggcgatgagcaactctttcataaggcaccttccttcgactcttcgtgcgtttcgttcatctactgcattctctcttacacgttcattctcttccaccatggcatccaacgggacatccacaaatggcgttcagcatgacgctcgcaaggtcttcttcttcgacatcgacaactgtctttacccgaaatcgtatcaaatacacgacaagatggccgtgctgatcgacaactactttcaaaaccatctgtcgctgtcccaagaagatgcgaccactcttcatcagcggtactataaggactacggcctcgccatcgaggggcttgttcgccaccacaaagtcgacccacttgagtacaacgagaaggtcgacgatgcgttgcctctggatgatatcatcaaacccgatccgaaacttcgaaaattgctgcaagacatagacaccgacaaggtgaagctgtggctattcaccaacgcctacgtgaaccacgccaaaagggtgactcgcctgcttggtgtagacgatttgttcgaaggcatgactttttgcgactacgccgcggaacgcctcctctgcaagcccacgacggagatgtacaacaaggctatgcaagaggcgaacgccaccgatatcgatcagtgctactttgttgatgattcagcgctgaatgcggctgctgctatgaaatacggttggaaaactgcgcatctggtcgagcctaccgcgaagcctccgccccagcccgtctcacaacaccagatcagcaaccttgaagagctgcgcaaggtcttccctgaagtatttaagacttcatgatggcatggaaattttaacgaagacacgagtgtattttacgaaaactactcaggattcccttgccttgtaagatgcgaccatcgctactgggttgggattggagatggtgcccagcaacgcttttgcgacactatcaggtctaaggactctattgtaaaacccgggtcgatttgcatatggttaattcgaatcttccatgaacacagcatttcgtgaaccaaagagcacacacgtcgaagtgttgggatgtctttgagcagccagcttggatttcttgagaggtcggaagcaattctataggatagacagcataaatgcaataaagccactattg

SEQ ID NO: 114 - DNA, 982 bp, metagenomes purified from environmentally challenged niches
atacaagacttaccatcaacacaatggctcgcatctttatcactggcagcaccgacggcctcggtcttctttctgcgaagcttctctcggaacaaggccacagcgtcttcctccatgcccgcaatgccgaacgagcatcccaggccaaagcagcagtgcccaaagcccaaggtgtcatcatcggcgatctttcaaacgtctcagacgtgaagcagctcgccgccgatgccaacaaggctggaccttttgacgccgttgttcacaatgctggcctcggactcaccaccaatggccagaagactgctgagggcgtagcccagatttttgccgttaacagcatggcaccttacattctgaccgctctcatggacaagccgaagaggctcttgtacgtcagctccggactgcacttcggtggcgaccccagcctcgaggacgtcacttgggccacaagggagttccgaccatcggatgcatacaacgatacaaagatgcaaaacgtcatgctctcgaaagcagtcgccaaacgctggcctgatgtgcagagcggctctcttgacccaggctgggtgaagactaagctcggcgggtcggccgcgcctggcaccaccgacgctccagcagagatgattgctgagtacgctgccggcaaatcttgcgcaggcgatcaaacaggtgcctacttgactccgcgtggcgtggaagagccgcatgatgcgactaagctggccgagaagcaggatcgtctgatgcagatttacaaggaggtatcgggtgtttcgttcccccagtaaacacagcttcatggctttgcctcgcggagacctcacattttcaattagatctccctgccgattgcagcagaccagtactcactaggctgtgcagggggcatgttgatcaagaacgagccataacgacatgccatgtcaacggacaatgagtgggcgaagtaacacatgaaattcattatctaagcgcc

SEQ ID NO: 115 - DNA, 982 bp, metagenomes purified from environmentally challenged niches
ggcgcttagataatgaatttcatgtgttacttcgcccactcattgtccgttgacatggcatgtcgttatggctcgttcttgatcaacatgccccctgcacagcctagtgagtactggtctgctgcaatcggcagggagatctaattgaaaatgtgaggtctccgcgaggcaaagccatgaagctgtgtttactgggggaacgaaacacccgatacctccttgtaaatctgcatcagacgatcctgcttctcggccagcttagtcgcatcatgcggctcttccacgccacgcggagtcaagtaggcacctgtttgatcgcctgcgcaagatttgccggcagcgtactcagcaatcatctctgctggagcgtcggtggtgccaggcgcggccgacccgccgagcttagtcttcacccagcctgggtcaagagagccgctctgcacatcaggccagcgtttggcgactgctttcgagagcatgacgttttgcatctttgtatcgttgtatgcatccgatggtcggaactcccttgtggcccaagtgacgtcctcgaggctggggtcgccaccgaagtgcagtccggagctgacgtacaagagcctcttcggcttgtccatgagagcggtcagaatgtaaggtgccatgctgttaacggcaaaaatctgggctacgccctcagcagtcttctggccattggtggtgagtccgaggccagcattgtgaacaacggcgtcaaaaggtccagccttgttggcatcggcggcgagctgcttcacgtctgagacgtttgaaagatcgccgatgatgacaccttgggctttgggcactgctgctttggcctgggatgctcgttcggcattgcgggcatggaggaagacgctgtggccttgttccgagagaagcttcgcagaaagaagaccgaggccgtcggtgctgccagtgataaagatgcgagccattgtgttgatggtaagtcttgtat

SEQ ID NO: 116 - DNA, 821 bp, metagenomes purified from environmentally challenged niches
agcgactccgacaacaacgaccaccgggacgactcatatccttcacaatggccattggacaatcctcgcagcagcaggccgacggccagaatgtcgtcacccagggcaactctgacaaggccgccaaccccatgcgcgagctgcgcatccagaagctcgtcctcaacatctccgtcggcgagtctggtgacagacttactcgtgccgccaaggtgctcgagcagctgagcggtcagacccccgtctacagcaaggcccgctacaccgtccgtaccttcggtatccgccgtaacgagaagatctccgtccacgttaccgtccgtggcgccaaggccgaggagatcctcgagcgtggcctcaaggtcaaggagtacgagctccgcaagcgcaacttctctgccaccggtaatttcggtttcggtatctccgagcacatcgacctgggtatcaagtacgaccctgcgatcggtatctacggcatggacttctacgtcgtcatgtcccgtcccggtgagcgtgtcgcccgccgccgtcgcgcgaagacccgcgttggtgcttctcacaaggtcaacgctcccgaggtcatcaagtggtacaagaaccgcttcgagggcatcgtcaggtaaaaagcttgaaaggtggtctgggatgatgaaaaattcaacttgtggttttggcaacggcgcaaaagagcgaggctatttttccgtagcttgaggatatatccggcctatcggagctttacttttacgcttgagcaagatcgcaaaaatggaggcctcgtataccaagcgagcgtgccgcataaccattgatcgctc

SEQ ID NO: 117 - DNA, 674 bp, metagenomes purified from environmentally challenged niches
ggacacaccggtgacgtcttgagcgtctcgttctcggccgacaaccgacaaatcgtttctgcttcccgagaccgaactatcaagctctggaacactctcggagagtgcaagttcaacattgttgacgatggtcactcggagtgggtctcttgcgttcgattctctcctaaccccgtcattcccgtcatcgtctctgctggttgggacaaggtcgtcaaggtctgggaattgtccaagtgcaagctcaagaccaaccaccacggtcacactggttacatcaacaccctcgccgtttcgcccgacggatcgctcgccgcatccggtggaaaggatggcatcaccatgctttgggatttgaacgatggcaaacacctctactctctagaggctggagacattgtcaactcgctcgtcttctctcctaaccgatactggctctgtgccgccactgcttcgtcaatcaagatcttcgacttggagtccaagtcaatcgttgacgacctcaagccagacttctccgccgagtactctgacaaggctcaaaagccacaatgtacttccctcgcctggtctgccgatggtcagaccctctttgccggtttctccgacaacctcgtccgagtctgggttgtcactgcttagagtcgtgaggattgtatgcatggataacgtgg

SEQ ID NO: 118 - DNA, 1183 bp, metagenomes purified from environmentally challenged niches
gaagtaccgttttctgtgcagttttttttaaacccagaacttgcaattgagatcacgcgtcgcaatggcaccctctacccagaagcaatggaccgttaaaaacggggagcaggactttgacggcctcgtttacggcgacgcgccagttccgactgcgggggactcggaagtcgttgtcaagctccatggtgcctcgctcaactaccgtgacctgattatccccaagggaaagtaccccttcccgctctcgttcccggtcgtccccggctctgacggtgccggtgaagtcgtcgaggtcggatccaaggtcaagcaattcaagaagggcgacaaggttgttaccctcttcaaccagctccatcagtacggtcccgttgacgctgctgcggcatcgtcgggcctcggtggtgcggttgacggaaccctgcgccagtacggtgtcttcaatgagaacggcgtcgtcagggccccgaccaacctgaacttccttgagtcgagcacactaacctgtgcgggactaacaagctggaatgcgctgtatgggctgaagccgcttcttcctggccagaccgtcctggtgcagggcactggcggtgtgagtatctttgctttgcagttcgcaaaagcagcgggcgcaactgtgatcgcaacaacctcatccgaagagaaaggcaagcgccttaaggacctcggtgccgatcacgtcattaactacaagacccaaaccaactggggcgagatcgcgcgcggtttgacgcgcgacaacatcggggttgaccacatcattgaggttggaggcgccggcaccctggagcagagcttcaagtgcatcaagttcgagggagtcattagtattattggcttcttgggcggaatgaaccccagcaccatacccaatgttctgcagaccctgagcaacatctgcactgtgcgcggtgtgtatgttggcagcaaggcgctgatgaacgacatgatcaacgccatcgaggcgaacaatatccaccctgttgtggatggaactgtgttcacccttgagaagacacgagaggcctatgagtacatgtgggcgcagaagcacttcggaaagctgaccatccagatcgcttaatcacttgatgaatataatgagggatatatgcgactaggaattatgcgctaatgaatataataaccatgcaattag

SEQ ID NO: 119 - DNA, 1563 bp, metagenomes purified from environmentally challenged niches
ggggccatgctcgagcagcagtaccagatgcgaaaggagcagcaagtgcaatttacacctatggcatcgccgtccagcactccttaccacatgcatcaagatttcactgttccgggcgactttttctcccccctcacatcgcctgcgctccacgctcagaatcagccacaatcgcgacagcaattcacggctcatcaacagggctactacacgaatcccagcaccgctgcgagctcggcggctccgagtccaatcgacgcgaacggagatgtggaaatgggtggcgacggtgttgcgctgccagagtcagcgagccaaccgaagaagccttcccgaaggaagcctgcgacaccgaggactttcgccatgaacaaggtcaagcaaagtcccatacaaaaaccgcaaaaaaggaagtctgtggcgttggcacacaaggatgcagatgctgtggtgcaggacgcccaacggtctggccatatcgcgcccaaatccgcaggtctccaaatgccgcctccgtttgagagctcggaaaacgacagtgtttcgccggaagcgctgaacgacctgcctatgggccccccgcctagacctggatcggtttcgcagtcgcccgccatcgctcctcagaatcagagcgtttctggaccggccgcgactcccaaatctctcctttctatgaagggcgctcaagatatgaatgcacctgccagtactggtatttctggccaaatgggacaggcatccttagaagatctcgaacttcccgaagctgccgaaaatccaggatcgactgcgacacactcgcaagtcttgaactcgcaagagccgacacctcgcctcatgccctcccgtaaaacgccaaaactcggccctcttagcacgccttcatcgggcaagcctacttctgcttccaacagtcccgctcatgcgttgtctcccatgacagcgagtacccctgctggtctgctgaaggacaagaaggacaacaaaggcggacgtgcaaccagcaagaagcgtggtagtgtcagtaccaccaattcagcaatggtctctccggcactccgaccgaaggtcagcccgagtatcaagcctctgctacccgaaggcaccagcctcaactccccgacccatgccctcctcctcgcctccaaatccaattaccagaacctcctggaaggcaaccacctccccggcatctcctacccggactccctctcaaccggcctcaccagcaaacgcacctcgcacaaagtcgccgagcaaggccgccgcaaccgcatcaacgacgccctcaaagaaatgcaagccctcatccccgcctcgtccggcgcccgcgccgaagagctcatgaccgccgacgccggcgacgacgacagccaggaaaccaaggagaaggaccgcgacgccgctgtcaagagcaatagctccaaagccgcgaccgtcgagagtgcgaatcggtatattcgcgtgttgaaggagagcgacgcggcgcagaaggatgcgatcgcgcggccgaattccccgggctcgagaagcttggatccaccggatctagataactga

SEQ ID NO: 120 - DNA, 939 bp, metagenomes purified from environmentally challenged niches
gacgacacaatgagaaacatcctcctagtattggcgtctgcagcgcttgctgttgtggcacaaaagccagatctcgacgtgaaaggcacgtttggagacgcgaaccccttctccaaggtcgtcaacggccaaagcaacaagctctacctcacgctggacaaccacagccctgagtctctggtggtcaagtctatcagcgggtcatggtctgagaagacgtccgcttcatccggtcaagagaagtttcttaagaactctaccacccaagagaagctcactgtccccatccctcccaagtccgagggcgcattccagcctcctacagtcttgacctaccagttctggagcgaattcaagcctagagagttgctcttgaccgttttgggttgactatgttgatgctaccggtcactcgtacagagaaacagcctacgaaggccaagtgactgtcgttgaggccccgggatctttctttgaccccgccttgctctttgcctacgccatggtgctggctctcgtcggcggcgccggctaccttgcctacaacatctactttccacctgcccgcaagcccagaagaagcgccaacaccgcacctacagatgctcctgctgctccggctgaccctgacgaatggattcctgtccaccacaagagggccaaaaagacgtctggcggcggggccaccagtggtgaagagagcgaagccactgaaggctatgcaagcgagaagtctgccagtggagccaagaagagaggcaaaggtggcagaaaataaatactgacatgtgcctcgagctgcagacgacgctcgtcaaaagtgtagcaagttgaagaagcccagcacgaagtccccagcttgactgctgccgtttggcttaatggcacagaaagcgagtgtacgtcgtacacggcttatagtctcgaatgcaacaaagg

SEQ ID NO: 121 - DNA, 896 bp, metagenomes purified from environmentally challenged niches
gccaaccacgacattgatccctttcacgacttgctttcgccatgtcagataacaacgatggaaatcacgggggaggcgtaggcgcgtcttactactatggcggcatcgcgattgcgctgtgtcttgtgattgtgttgacgcttgtatcaagaatattatatcgacgacgtgtaaggaacagactcctgcgagccaacagacaagagcgcattactttgcgagaccggggagaagcgccaggcctgccaacctatcgggagtctcgcaatcagccctcattaccgcgatacacggccgaggcagactacgcacctccacccggcccgcctccttccaacagcccggacaacgaaggccaccacttccacttccatttcccctctttacatgtgcctcaggcactgcacttgcggcctaggcaggcagacgatcctgctgaccagatccccaccgtgccccctccgtcctacgagccgcccaagtatgagccgcccagtggagcgcctccagagcagcaacaagagcctgtggctagcgggagtagcgagcatcatcaccagcagtctgctttgggcgaacataccgcggcggcaacagccgctgccacaactccggcagagcacagtggcgagtcgacagagcttaggagtgcgtcgccttctcagccacaatctcaatcccaacctcaagcaccagcacaaccacaagagcaggattacggctacgacgatgccgactttatccatcctgaagagcgacgcaggatcgaggctgcgcagcgcaatgatccgcagacatgattcaaacatgtgttgtaaagtgtactactatgaactcgttgaccagtataatcgaagcgtatataacggcacaaatgcaaagctgccatcatcccg

SEQ ID NO: 122 - DNA, 697 bp, metagenomes purified from environmentally challenged niches
cattacggccgggaagctttcagaagctaatcgagttcttcctatccctttcaactttacacaccatgtctagaattggcgatccaacgaacaaccctgctacccagcaactgtactctgataggcccttgcatctccctggccccggcctcaagccatccaggcagctcactatcagctcggctgttgcgttccgcgaggattcgggccaaacacgcttcaacctcatcagctctgaccaccgcgaggtgttgcacattagtattcgtgcaagggacaacgttctcgtgctcaacaccaaggcccccgatggcgattggggcaaagaagagcgacatgatctcaaaccccttttcgataccccactgctgccttacatcaccgtaatggcaacgaagaacagctatatcctttctgttcctggtaaacgggagatcatcttcaataagaggaaagggttcatggagcctgctgtgaggattgagtatgactatgatgagatgtctgcgttctccgacccctgctacattacagtcccatcttcatcttaaagctttcctagttggcttggagttggcggatatggtcacattggttttttcacacggcaaacggtaaagaattacggcttctctctcctgtcatgttcagcggacgatgtatgatgtagtgttctgttcaattgatctggttgttg

SEQ ID NO: 123 - DNA, 329 bp, metagenomes purified from environmentally challenged niches
ggaacgaccacgagcagtttttaaaatgccacaagaaatcaaggacatcaagaacttactcgaaatcgctcgtcgtaaggacgctcgttccgcccgcatcaagaagaccaagaccgttggtgctaagggcgagccagctcaacttaccaagttcaagattcgttgctctcgctacctctacactctcgtcgtctctgacggtgagaaggcagagaagcttaagcaatcactcccaccaaccctcaacgtcgaggagattggtaaggtttcaaagaagtagattagtgatgtaatttgctgccttgattgattgtccttgttggtatttt

SEQ ID NO: 124 - DNA, 747 bp, metagenomes purified from environmentally challenged niches
gtacacataactcttcattcctcatcatgtctcacactttctacgatggcaccatcgtggtgcttcaaggcattcttgaaactttttctcatatccttcacaaagccgaagaaagcccaaactctagcgcttttcccgcagctcgtctgcacgaggacatgtatccattgaccgaccaaattcgcctagcaactcaattttctgagtatattctggctaaagtgaccggccgcgagccaaggaagttcgaaggcaatccattgaccttcgctgaattctatgagcgtatcgataccatgctgaagtcactcaaagaagcagataaggatgtcgtcaatgcaaatgccgacaaggaggagcttactcaagttggacctaccgcaaaaattgaattgagtaatgctatatacgcccatcgcatagccttgcccaacatttacttccatctcaacattgcttacggcattttgcggaaggagggcgtgcctcttggcaagcttgactattttgcgggctttttcccaccgagcatggctcaaggcaagtaaagaagtgatgttggttatgtttccggatggagagggtgctgatctatgagaatgagttccgagtagaccatgatggtctagatgtggacttgagctttcatttgccaaattcttgtggaaagatagcaatgacggaacaagcgatttgtatgtacatttaatgaagtctatctatagaattaatctccgatctatcgcg

SEQ ID NO: 125 - DNA, 693 bp, metagenomes purified from environmentally challenged niches
aagctcttcaaagctaattatcgagttctcctatctcttgcacttatacacaccatgtctagaattggcgattttgcgaacaacaaccaggctacccagcagctgttctctgatagacccatgcagctccctggccccggccttaagccgtccaggcagctcacggtcagctcagctatggcgttccgctgggactctggccaaacccgcttcaacctcatcagctctgaccgtcgtgaagtgctgcacatcagcatccgcgcaaaagacgacgtccttgtgcttaacactaaggctcctgatggcaattggggcaaggaagagcgacacgagctcaaaccccttttcgacaccccgatgctgccttatatcaccgtaacggcgactaagactagctatatcctgtccgttcctggtaatcaggagatcatcttcaataagaggaaagggttcatggagcctgctgtcaagattgagtatgactatgacgagaaccctgcgttctctgatccgtgctacgtcacagttccgcatttatcttaaggtcttattggcttggagttggcggatagtcacaccggtttttttcacacggcaaaaggcaaagtattacggcttttctctcctgtcctgtttagcggatgtacgatgtatgttgtagtagtgttctggaatttgtgttcaagttgttgg

SEQ ID NO: 126 - DNA, 1030 bp, metagenomes purified from environmentally challenged niches
gagcgacttcatcaaaaatgtcagagcaacttcactacaagggttcattggccggccacggcaactgggttactgccatcgctacctctgcagagaacccagacatgatcctcactgcttcccgtgacaagtctgtcatcgtctggcaactcacccgtgacgacgctcagtacggttacccaaagagaatcctcaagggccacaaccacttcgtctctgacgtctccatctcatacgacggtcaattcgctttgtcctcctcatgggacaagaccctccgtctctgggacctcaacactggtcttaccaccagacgtttcgttggccacgaagcagacgttctctccgtctccttctccgccgacaacagacaaatcgtctctggctcccgcgaccgcaccatcaagctctggaacacccttggtgaatgcaagttcgacatcaaggatgaaggccactccgaatgggtttcatgcgttcgtttctctccaaacccaatgaacccagtcatcgtctcagctggttgggacaaggttgtcaaggtttgggaactctcaaactgcaagctcaagaccaaccactacggtcacactggctacatcaacaccgtctctgtctccccagacggatcccttgctgcctccggcggtaaggacggcatcaccatgctttgggacctcaacgagggcaagcacctctactccctcgaggctggtgacattgtcaacgcactcgtcttctcaccaaaccgttactggttgtgcgctgctactgcctcatgcatcaagatcttcgacctcgagtccaagtccatcgtcgacgagctcaagccagactttgtcgacgtcggcaagaactcccgcgagccagaagctgtctccctctcctggtccgctgatggtcaaaccctcttcgctggtttcaccgacaacgccgtccgtgtctggaccgtcgcataaaactaagctgtatctaatagacagggtattgggttttgtaacactattgcgaggaactcatgattttaccg

SEQ ID NO: 127 - DNA, 668 bp, metagenomes purified from environmentally challenged niches
ggggaaggtggtggtatccacggaaccaccttcaactccatcatgaagtgtgatgttgacgtccgtaaggatctctatggcaacattgtcatgtctggtggtactactatgtaccctggtattgccgaccgtatgcagaaggaaatcaccgctcttgctccttcgtcgatgaaggtcaagatcattgctcctcctgagcgtaaatactctgtgtggattggtggttccatcctggcttctctgtccaccttccagcagatgtggatctcgaagcaggagtacgacgagagcggcccttcgatcgtccaccgcaagtgcttctaagcttaagcgcatggttgatttgcttgtttgtacttcttttctggcgtatcaaaaggcaggacagtgtggcatgcggaccttttctgacctgatgacgagagggatcgcctaagaaaaaggaactttattttagttgtggaatagagacggtttatttgacgctagttctcgtccagagcatcctcgagacgatagtctgggttcgtcttaagcgatggatggtggtgattctcttcgtattgttcctgtacctgtactacatattgcctacaccatgtcctgttcatttcttctctgtttgcgttgcgttagaccttataaatttaaatgtcgtattgctcccc

SEQ ID NO: 128 - DNA, 668 bp, metagenomes purified from environmentally challenged niches
ggggagcaatacgacatttaaatttataaggtctaacgcaacgcaaacagagaagaaatgaacaggacatggtgtaggcaatatgtagtacaggtacaggaacaatacgaagagaatcaccaccatccatcgcttaagacgaacccagactatcgtctcgaggatgctctggacgagaactagcgtcaaataaaccgtctctattccacaactaaaataaagttcctttttcttaggcgatccctctcgtcatcaggtcagaaaaggtccgcatgccacactgtcctgccttttgatacgccagaaaagaagtacaaacaagcaaatcaaccatgcgcttaagcttagaagcacttgcggtggacgatcgaagggccgctctcgtcgtactcctgcttcgagatccacatctgctggaaggtggacagagaagccaggatggaaccaccaatccacacagagtatttacgctcaggaggagcaatgatcttgaccttcatcgacgaaggagcaagagcggtgatttccttctgcatacggtcggcaataccagggtacatagtagtaccaccagacatgacaatgttgccatagagatccttacggacgtcaacatcacacttcatgatggagttgaaggtggttccgtggataccaccaccttcccc

SEQ ID NO: 129 - DNA, 1018 bp, metagenomes purified from environmentally challenged niches
gactttctcatttcagaattattttctatactctgacaagagcaagcaataccaaacatcttccacatcgaagctttaaccattttgcccttaacatttgaacaagacgaaatggccttcttcccacactacaccactaatctgtcgcctctgctctacttgttggacgacgactatgctgtctaccgctcaacttgtccaaagtccaactaccaccacaagcaacaccacagccgccgtcagccttcgccagttcgttactttagtccgaattttgatatgcgagaggggaatgactcctactaccttgacggagagctccctggtgtcaaccagaatgatgtcgatattgaattctctgaccctcagacactggtgatcaagggtcgagtggagcggaattacaacaatctcgacggcatgaacgaggaaaaccagcaagatgaagaacaattctctgaaactctctctagcaagtcgtaccaacccactgtcgaggacgaggacgaggcgaaccattcaccacccgtggcgacaccaacctactctgagaagtctgttactgagaaaactcagaagcctgcgtacaaataccgaaattctgaacgtgctattggcgaattccaccgagccttcaatctccctacaagagtcgatcaagatgcggtcagggctacattgaggaatggaatcctctcgctggagctcccgaaggagccggcaccgaagatgaagaagattcggattgaatagaggatttcgaataaaatttttgatttgatgagtagttggtgtttattgttatgtctaattatatggggctatgtcatgattgggaaatgggacaccgcatttgtttcctttttccccatttcttcagacgccatctatattgcatgtatgttgcatgaactatggtttttgctaggagcggttgcttctgctttgcattttcatgaactattttctttttattaaattaataactagcatatcaattaatgatctgtcatatggc

SEQ ID NO: 130 - DNA, 686 bp, metagenomes purified from environmentally challenged niches
aagctttcagaagctaatcgagttcttcctatccctttcaactttacacaccatgtctagaattggcgatccaacgaacaaccctgctacccagcaactgtactctgataggcccttgcatctccctggccccggcctcaagccatccaggcagctcactatcagctcggctgttgcgttccgcgaggattcgggccaaacacgcttcaacctcatcagctctgaccaccgcgaggtgttgcacattagtattcgtgcaagggacaacgttctcgtgctcaacaccaaggcccccgatggcgattggggcaaagaagagcgacatgatctcaaaccccttttcgataccccactgctgccttacatcaccgtaatggcaacgaagaacagctatatcctttctgttcctggtaaacgggagatcatcttcaataagaggaaagggttcatggagcctgctgtgaggattgagtatgactatgatgagatgtctgcgttctccgacccctgctacattacagtcccatcttcatcttaaagctttcctagttggcttggagttggcggatatggtcacattggttttttcacacggcaaacggtaaagaattacggcttctctctcctgtcatgttcagcggacgatgtatgatgtagtgttctgttcaattgatctggttgttgac

SEQ ID NO: 131 - DNA, 698 bp, metagenomes purified from environmentally challenged niches
gggcatataaccacaggtcattcgcatccgtcgcagaacttcttacatctgagctttcctgtccgttagatataggcaaaatgaaggcctactggtacgataaccaaccgggcgaccagcgcttgcctcacgactccggccgccccgtcaccgagtcctacctcgagtccatcggcgtcttctaccgccactgcccaacaattgaccttgtcgactccctggccgccgagcgcggctacaagaaccgcgacgaggtctgcgtctcgccgcagactatgggcgatgtctacgaggagaaggtgaagacgttctttagtgaacatttgcacgaggacgaggagattcggtacattcgagatggggaggggtactttgatgtgcgtgggcaggaggatgagtgggtacggattcggttgagtaaggatgatctgatcattcttccggctgggatctaccatcggtttacgacagatgataagaactacgtcaaggctatgcgtctcttccaggaggagcccaagtggacgcccttgaaccgtggccctgaggttgatgtcaaccctcaccggaagacatacctggaaaccgtccccagccctgctgtggctgcgaactaagtgagcatcgaatgctcttgttgaacaatctatttgcacatctttagcctttatacacctcaatgcatcaatggatttagg

SEQ ID NO: 132 - DNA, 884 bp, metagenomes purified from environmentally challenged niches
gtggctgccggctacacccccgaggccctcgagatcctctccaagaagaagggcggcaagtacctcgtcctcgagatggacgagacctacaacccccccgccgaggagacacgtactctctacggtgtccagctcacccaggcccgcaacgatgctgtcatctccccccagaagaccttcaataccatcattacccccaagaacaccgagtccctccccgagtccgccctccgcgacctcaccgtcgccaccctcgccctgaaatacacacagtccaactccgtctgctacgcgctcaacggacaggtcgtcggcctcggtgccggccagcaaagtcgtatccactgcactcgtcttgccggcgacaagaccgacaactggtggatgcgcttccacgagcgcgtgctcaacatcaagtggaagcagggcaccaagcgtgctgacaagagcaacgccatcgacctgctctgctcgggccagacgccccgcaatgacgctgagaaggtcgagtacgagcgtgtgttcgcggaggttcctgctccgttcacccaggaggagcgtgatgcttggctctcgcagttgaccaacgttgctatttcttcggatgctttcgtatgtctctcccctctgttagagcattctaagttctaagatcatgctaattggtgaaatagttccccttcatcgacaacgtcttccgagccgcccgctccggcgtcaagtacatcgctgcacccagcggttcgcagaacgacggccctgtcttcgagactgccgagaagcttggtatctcgttcgttgagcagggtactcgtctgttccaccactaacttgcttttccggtggcgtggtattatggtataaaaagaaaaagggtttggggg

SEQ ID NO: 133 - DNA, 822 bp, metagenomes purified from environmentally challenged niches
gtggctgccggctacacccccgaggccctcgagatcctctccaagaagaagggcggcaagtacctcgtcctcgagatggacgagacctacaacccccccgccgaggagacacgtactctctacggtgtccagctcacccaggcccgcaacgatgctgtcatctccccccagaagaccttcaataccatcattacccccaagaacaccgagtccctccccgagtccgccctccgcgacctcaccgtcgccaccctcgccctgaaatacacacagtccaactccgtctgctacgcgctcaacggacaggtcgtcggcctcggtgccggccagcaaagtcgtatccactgcactcgtcttgccggcgacaagaccgacaactggtggatgcgcttccacgagcgcgtgctcaacatcaagtggaagcagggcaccaagcgtgctgacaagagcaacgccatcgacctgctctgctcgggccagacgccccgcaatgacgctgagaaggtcgagtacgagcgtgtgttcgcggaggttcctgctccgttcacccaggaggagcgtgatgcttggctctcgcagttgaccaacgttgctatttcttcggatgctttcttccccttcatcgacaacgtcttccgagccgcccgctccggcgtcaagtacatcgctgcacccagcggttcgcagaacgacggccctgtcttcgagactgccgagaagcttggtatctcgttcgttgagcagggtactcgtctgttccaccactaacttgcttttccggtggcgtggtattatggtataaaaagaaaaagggtttggggg

SEQ ID NO: 134 - DNA, 996 bp, metagenomes purified from environmentally challenged niches
tgaagcagtggtatcaacgcaagcagtggtatcaacgcagaatgtgcgatcgctctagaatcggtcccaagggttgggaagcagtggtatcaacgcaagcagtggtatcaacgcaagcagtggtatcaacgcaagcagtggtatcaacgcaagcagtggtatcaacgcaagcagtggtatcaacgcagagtgcgcagcccggtgctatctctgctcctgtggcagctggtaaggacgttgagctgcagtggaccgaatggccggaaagtcatcatggccctgtcattacttacctggccaactgcaacggtgactgctctgaggtcgacaaatcctctctggagtttttcaagatcgatcagaagggtctcatcgatgacagcaatgtccctggcacatgggctaccgacaaactaatctccaacaacaacagctacaccgtcaccatccccagcgacattgctgccggtaactacgtcctccgccatgaaatcattgctctgcactccgctggcaacgaggatggtgcccagaactacccccagtgtctcaacctcaaggttactggtggtggcaacgcttctccctcaggtactcttggtaccaagctctacaacgaggacgactcgggtatccttgtcagtatctaccagcagcttgactcctacgacatccccggccctgctctgtactctggcgcttcctcgtcctccaactctggttcttcttccagcgttgcttcggccactgcttctgccacttctgccgctgcttcctctccctcgtcctctcaggcttccggtacccccgcttcccaggtcaaggctcagaccgctagctctactcctagcgcttcgtccggtgccacttccggcagtctgtccgactacttcagctctctgagcgctgaggagttcctcaacgttatcagcgagactctgtcttggttggtcactgacaagattcacgctcgtgacttgtcgaccgcataaatgg

SEQ ID NO: 135 - DNA, 823 bp, metagenomes purified from environmentally challenged niches
gtggtatcaacgcagagtgcgcagcccggtgctatctctgctcctgtggcagctggtaaggacgttgagctgcagtggaccgaatggccggaaagtcatcatggccctgtcattacttacctggccaactgcaacggtgactgctctgaggtcgacaaatcctctctggagtttttcaagatcgatcagaagggtctcatcgatgacagcaatgtccctggcacatgggctaccgacaaactaatctccaacaacaacagctacaccgtcaccatccccagcgacattgctgccggtaactacgtcctccgccatgaaatcattgctctgcactccgctggcaacgaggatggtgcccagaactacccccagtgtctcaacctcaaggttactggtggtggcaacgcttctccctcaggtactcttggtaccaagctctacaacgaggacgactcgggtatccttgtcagtatctaccagcagcttgactcctacgacatccccggccctgctctgtactctggcgcttcctcgtcctccaactctggttcttcttccagcgttgcttcggccactgcttctgccacttctgccgctgcttcctctccctcgtcctctcaggcttccggtacccccgcttcccaggtcaaggctcagaccgctagctctactcctagcgcttcgtccggtgccacttccggcagtctgtccgactacttcagctctctgagcgctgaggagttcctcaacgttatcagcgagactctgtcttggttggtcactgacaagattcacgctcgtgacttgtcgaccgcataaatgg

SEQ ID NO: 136 - DNA, 1000 bp, metagenomes purified from environmentally challenged niches
gacggtgaagttggaatagaataaaatgttgagcatgtttaccagagtggccagaggacaggccaaggtgtttacccgcaacgcatccacagcatcatccaaaccaacgaatcaatcatccaacaaggctgccactatcgcagcttcaatttcaggtgttaccgccgcgttatacgcccaccaatacggcctcattgacagcgtcttcgctagtggcttagaagagggtttgcacgctcctcatttcccttggtcacacaatggctggttggacagctttgaccacaactccattagacgcggttaccaagtttaccgtgaggtgtgcagctcgtgtcactctttggacagaatagcgtggagaaaccttgtcgctgtgtcacacacttcagatgaagccagagcgatggctgaagagcaagagtacactgatggtccaaatgaccaaggagagtctttccaaagacctggtaaattggctgattacatgccagctccttatccaaatgaggaagcttcgagggccgccaatggtggtgctcttcctcctgatctttctctcatcgttaaagcaagacacggaggagctgattacattatggctctgctcactggttaccaggatcctcctgctggtattcaagttcaagagggcatgaacttcaacccatatttcccaggtggtggtattgccatgggtagagttttgttcgatggtctggtagaatacgacgatggcactcctgctactactacacaaatggctaaggatgtcgctactttcctcagctgggctagtgagccagaacacgacgacagaaagaagatgggcttccaagctgtcattatcctctcagctatgaccgccatctcactctacgtcaagagactcaagtggtcgcctatcaagacgaggaaactgacttacaacccaccaaagtgatctgaatgtagagaaaagtttgacccgtataaaaaatttcatcctctcctttttccg

SEQ ID NO: 137 - DNA, 544 bp, metagenomes purified from environmentally challenged niches
ggaggtagtccagccaaaaagagtttgataggcgcgatggaggcacaaaatctcaagactttcccaaagcaacctatcttccaaaactcaaagacccgtggtaacaagaaggtcaccaaggaccgtcgttggtacaaggacgtcggtctcggtttcaagactcctcaagaagccatcaccggtacttacatcgacaagaagtgcccatggaccggtgaggtttccatcagaggccgtatcttgtccggcaaggtggtctctaccaagatgacccgtacgatcgtcatcagaagagagtaccttcactacgtgccaaagtacaacagatacgagaagcgtcacaagaacctcccagtgcacgcatcacctgcattccgtatcgagaatggtgaccaagtcgtcgttggccaatgccgtccactttcaaagactgtgagattcaacgtcctccgtgtcatcaagaacaaggctgctgctaaggctttcgcaaagttctaaacttgttattaatgtagttggtccattcacagaattttgaaagtcc

SEQ ID NO: 138 - DNA, 938 bp, metagenomes purified from environmentally challenged niches
acgttcaattgacttttccattcttttgttcgttctgaagagttttcttttttctttcattgtcgcctcctttctttcgccttcccgttgtttccgatcatcgggtgttgccagagtatatatagagttggggctcccttttatctatctcaccgcaaccgtcctcctgatcctctctcctgatcctcctccttcattccttgactcctcttcacgctcctcctgaccagccaagtcttacatccctctctacaactactactcttcaaataatcctctcctctcggtgggcttgaatcccttatcttccgcctctccccacgaaccggaccggatcgtcttatcgcctccgcaccagctggcgcttactacctcatccacctctttcccgtctcgccaccgaaaccagtctacaatgcctcctcgcaagcccagatgctcctttaaggagtgcaaggaacaagcccagcgcattgtcggagactgcagcttctgcagcggtcacttctgctccaagcatcgcatgctcgaagcccactcctgctccggtctggaagactgcaagaaggagtcccacgcccgcaatgctgataagttgaacagcgagcgcacacaggttatcaagggtgtatgacgggatcacatctacactactacaacaatctcggcgcatttcgattgcatttacttgccatttttatccgacgttgagttagcgcggtgttatttacaatttcttcttttctttattttgcctacgatgtctccccctatcggtatggtggtgtctcgtttcgggagcgacatggtttacaatgattttggtttggggtggtctctcggtatttgtctattatccacttattttccggggtattatgcgcatggcgttactatatggagtttgatattctatctcgaatcgatacttttacaac

SEQ ID NO: 139 - DNA, 687 bp, metagenomes purified from environmentally challenged niches
aagctctcccaagctaatcgagtttttactgtcacttgcatttatacataccatgtctaggaacttcggcgatttttcgactaaccaggctactcagcagctgtactccgatagacccttgcatctccctggaaatggccttaagccggctagacagctcacgatcagttcagctgtcgcattccgctgggactctgaccaaacccgcttcaacctgatcagctctgaccgtcgcgaagtgttgcacatcagcattcgcgcaaaagacaacgttctcgtcctcaacaccaaggcgcccgatggtgactggggcagggaagagcgacacgagctcaagaaacttttcgatacccctatgctgccttacatcaccgtgacggcgacgaagatgacctataacatcactgtccctagtggtcaagaaatcatcttcaacaagaggaaaggattcatggaacctgctgtgaagattgagtatgactatgatgagcactctgcgttctccgacccatgctacattacggttccatcttcttaaaggctcgtcggcttagagttggcggatagtcacactggtttttcatacggcaaacggcaatgtattacggcttttctctcctgtcctgttcagcggtagatgtacgatgtatgttgtagtgtttcaaatttgagttcaagttgttggcc

SEQ ID NO: 140 - DNA, 601 bp, metagenomes purified from environmentally challenged niches
gtctgcttgcttcaacgagcgctgaatttcttgttggccggtgttgattccccggattccctgttatcgcctgctgtgttcgccttggtagcaggtgtttgaattggtcctgcaatttcgctgattgctggcctcgaactcccgatcgaacgaactctcctctcctccgtcaacgcaccttcacatatcgcaaagcacaatggtttccaagattctcttctggagtggcttcggcatcgccgtccgtctctggcaactcggtatcgaaatgcgtcccattcttgccaagcagggtctctgggcctaccccgtcttcgcaggtgtcggtggaagcttcggttactggctccagggtgtcgaggaccgtcagctgaagattcttgcgcagcgccgcgaagccatcctcgacaagcgccggagacgggacgagcgtgagggtctgagcaacattgagaaggagggtactttggctgcgaccccatgatttgttgcgttggctgttgtttattttcactgccttcggagaaagaccggcaattgcattgctgggcatgtatcataccaaaacagaggaaggttaatggtcaattgtttaatgacc

SEQ ID NO: 141 - DNA, 601 bp, metagenomes purified from environmentally challenged niches
ggtcattaaacaattgaccattaaccttcctctgttttggtatgatacatgcccagcaatgcaattgccggtctttctccgaaggcagtgaaaataaacaacagccaacgcaacaaatcatggggtcgcagccaaagtaccctccttctcaatgttgctcagaccctcacgctcgtcccgtctccggcgcttgtcgaggatggcttcgcggcgctgcgcaagaatcttcagctgacggtcctcgacaccctggagccagtaaccgaagcttccaccgacacctgcgaagacggggtaggcccagagaccctgcttggcaagaatgggacgcatttcgataccgagttgccagagacggacggcgatgccgaagccactccagaagagaatcttggaaaccattgtgctttgcgatatgtgaaggtgcgttgacggaggagaggagagttcgttcgatcgggagttcgaggccagcaatcagcgaaattgcaggaccaattcaaacacctgctaccaaggcgaacacagcaggcgataacagggaatccggggaatcaacaccggccaacaagaaattcagcgctcgttgaagcaagcagac

SEQ ID NO: 142 - DNA, 380 bp, metagenomes purified from environmentally challenged niches
gggggcgacatggcttcgacgccggtgacaatccctgaggtgcatgccgagagcgtaacgtatctcgtaaatccaacgttacgataaaatagtcgcaaacgacgacaactacgctcagggcgcgctggcagcgtaacaactgctagcttctagtccggcccggaggtgatgtgcccattcatcaccgaagggatacgagctcagactgatgggatcgcggctggctttgtcctcgcgtcagccgctaaaacttagaggaatcgcgtcgctggatcctgcccgtcggagccagaggcgctaaatcaaaagacggacctaagcatgtagagccgatgggtgagtgccggcggacgggggttcaattccccccgcctccacca

SEQ ID NO: 143 - DNA, 977 bp, metagenomes purified from environmentally challenged niches
gggaccagaacagcttcagctacaatgccattcatcaaggaagccaagagcaacagctacttctctcgctaccaagtcaagtaccgcagacgtcgtgaaggcaagactgacttctacgcacgtaagcgcttggtaacgcaagctaagaacaagtacaacgcaccaaagtaccgtctcgtagttagattcacgaacaaggacatcatctgtcaaatcgtgtcatcaaagcttcaaggtgacgttgttctcactcacgctcgcgcccgcgaacttccacgttacggcatcaagcacggtctcacgtcatggtcatccgcttacgcggttggtctcctcgtcgcaagaagagcgctcaccaagctcggtcttgctgacaagtacgagggtgacgttgaagctactggtgaatacaacctcaccgagccacttggcgatgatgaaccacgtcctttcaaggtcttccttgacgttggtcttaagcgtacctctactggttctagagtcttcggtgctcttaagggcgcctcagacggtggtctctacatccctcactctgagaaccgtttcccaggttacgatatcgagagcaaggaactcgacgctgaaatcttgaacaagtacatcttgggtggtcacattgctgagtacatggaggctcttgaggaggaagatgaggagagattcaaggctcaattctctacctatcttgaagacggtattggatctgaggacattgaagaaatcttctcgggcgcacacgaggctatccgtgctgacccaaccttcaagccaagtgaggctgccaagggcaccgactggaagtccgagtcaaagaagcaccgcgctgtcagactcaccaagcaacaacgcgaggacgctatccaacagcgtatcaagtactaccagcaagctggcgacctcgagtaaacggtaattgtagcggtctacatagacaatcaatgtctgttgttccttag

SEQ ID NO: 144 - DNA, 73 bp, metagenomes purified from environmentally challenged niches
gattacccgctgaacttaagcatatcaataagcggaggaaaagaaactaacaaggattcccctagtaacggcg

SEQ ID NO: 145 - DNA, 823 bp, metagenomes purified from environmentally challenged niches
gggtctcttccatttgaatttttcaacccacagcatggccttcatgaatctcccatggcccactgaatgcctacatgccgctctcaagaacggatccttacctttctggggatttgtaatctatcgaacgacctacaccgctcagtcagatgccgcctggccgcagattatcgagcttattgcctcctatatgaaagccttactctaccacgagtataacgacaagaaaaaagatggagatgagcctacagtctacgacgaaatctgggcaaggcatcagttgacgattatggatgatagacaattcaacggagcgtctgtgtttgatatccaacttcacttcgaaaagtgggttgaggcgcagggaaagcgagatgaatctactatgtatcgcatgtgtatggtcattgatgatgaatcaatccagacgttattggaggcgccacccggggaaaataggaaactcggacgacgtatagggggccctgtacgctttgtcaaagtcgtggaggctttccccgagctagacagccttgacgaattccagggatggatgaaatgtgagatcaacgcgttatggccgctgtggaagatgatgtctgacggagatgaaatgaggatgtcatatgatgagatgaaggggaatggaaagcaggtctatggcgcaatttaatcggtttttcttcatgttatcctgatggaaaaaatggcagaacatatgtctgtacatgcagaaaataaggtgattggaaaatacttgaatgctatgaagttagatagtagctgttctagcggccagataaagccgcgcatgtgaatttcg

SEQ ID NO: 146 - DNA, 181 bp, metagenomes purified from environmentally challenged niches
gtactaaccactcgtcaggcgctgaaagaagaagatgcagtaagtttgatgttttctgtgtatgattatacataaagttgttgtataactacgcagaaaagttttcgtatgcaaaactttgattggtgttaagtcgaaataaggttcgtgtaatggaaattgcacggggagtataaaatgt

SEQ ID NO: 147 - DNA, 734 bp, metagenomes purified from environmentally challenged niches
atgacagagaaactttacaccgagcaagtgaatgcgttcggaaacgaattacctcctctatcatacaaagacctggacaaactccccttacaccaaaacgtcatcaaagaaactcttcgaatccacaactcaattcatacactcatgcgtaaagtgaaaaatcccctcccagtcccaggaacaagattcgttataccaaccagtcacaccctcctcgcgtccccgggcgtaacaacccgcgacgattcacacttccgaaacgcaatgacctgggatccacaccgttgggaaacacgaagtgaggtcgaagatgatggtgagacaatcgattatggatatggggttgtttcaaaggggacgaagagtccttatttgccctttggagcgggtcgacatcgatgtattggggagaaattcgcatacttgaatcttactgttattgttgctactcttgtgaggaattttcggttttctgaacctgatgatagagagggtgttcctgaaacggattattcgtcactcttttctagacctatgcggccggcgactgctcggtgggaacgacgtggggagtactagaggtgggattattggggatttgattgctttttggaattgggatggaagagttcttgggatatattcttgttcttcgaggctttcccaggtgatttttcacagggcttggtattatcgtatttaatcaatcaattcactacacttttcgagcttgc

SEQ ID NO: 148 - DNA, 801 bp, metagenomes purified from environmentally challenged niches
gacatcattgcatccaatatcagatcacattccatagcctcatttactgcccaagaaggcttatggcccattggagagaggagtacctaactgcactggcagtgcgagatcagagggagaaggccaatctcagtatttacgatgcctatacccgactcgcagatagcacggccaaacttccagctacaatagatacaagtggcagcccctcaggtgataaagggccatctggtacctacgagtccgaaaagacggcattttctcaatcaaggacagccaagaagcagcagacagaagtggagccttcagttacggagcttctaaatactacacgtgcagaactagccgaagcacagcgctctcgggcagaattgcgagatcgtctagagcgagctactaacgaagcggagaaattgcggaaacagattggcaaagatggtcgacgaatacatggactggaaaatgaagttgctcaacagcaaaagcgccgcaaagatgttgaagaagagttgagaggaaaggctaagctactcaatgaattccaagacgaaattgcagctctgactctccaggtgaacatggccgagagaaaagctaagaagcttggagaggagaacgatgatcttgttaatcgttggatgaagagaatgggccaggaagctgatgcaatgaatgatgcctccaagttttcgtgactgccgaatcagaatagaatcaaatggcccagataggccttcgcattgttatgacatgatcgaattccgaggcaaattcgcctatcatggtaatgaacggataaag

SEQ ID NO: 149 - protein, 213 aa, metagenomes purified from environmentally challenged niches
MAFFPHYTTNLSPLLYLLDDDYAVYRSTCPKSNYHHKQHHSRRQPSPVRYFSPNFDMREGNDSYYLDGELPGVNQNDVDIEFSDPQTLVIKGRVERNYNNLDGMNEENQQDEEQFSETLSSKSYQPTVEDEDEANHSPPVATPTYSEKSVTEKTQKPAYKYRNSERAIGEFHRAFNLPTRVDQDAVRATLRNGILSLELPKEPAPKMKKIRIE

SEQ ID NO: 150 - protein, 164 aa, metagenomes purified from environmentally challenged niches
MQLLSTLTPLALLVTVASATGKAVNNAVGNAVVTNHCKDPIYLWSVGSSVSPKHTIPSGSNYTEPFRHDDASGGIALKITRNDNGLYDGSAQLVYSYALDGEQVWYDLSSVFGDAFAGEAVAVKPENEGCGSICWPKGTTPGGSQVKVCDAEGDVGLVVCAKGC

SEQ ID NO: 151 - protein, 149 aa, metagenomes purified from environmentally challenged niches
LLAEAIRRGLLGWRRAEAKWQRCCCWLSTGHSARKCTREHSLVLHERLSRNRARHWQGVVALCLRCQQPLCFRTVSFALTVLLECIINRQRLVHQVLAIHSRDCLVRAVKVVVLDESISFQKKKKKKKKKTGGQVLKLPEGISPHGQKF

SEQ ID NO: 152 - protein, 119 aa, metagenomes purified from environmentally challenged niches
LKGYGFIQYNDFDSSDQAITAMNGQYLMNKPLTVDYAFKKDGKGERHGTEAERLLAAEAKRNNALPMPGAIPGQPFMQYQGMFAGALSGAMPGAQPAATPLPFGFSPAPPQQSTPYGFS

SEQ ID NO: 153 - protein, 188 aa, metagenomes purified from environmentally challenged niches
MFGFNFNTTKLLKTILVVCYLQATVLADPYTRVSWEAYMNHVNGSDDYRTQGDDTRATRFPETKPPKQGKDFLWSSKPVPSSDLFLEFFMYEGEPDEFSRTTESYQSLPSNALTARQNALTCQDIESCSYPPQVNNFQALFDDLGPSTCNLIKDETRDWILQQWPGLAVGAVISFAVAVAGSSCDILY

SEQ ID NO: 154 - protein, 187 aa, metagenomes purified from environmentally challenged niches
MVRYAHNAENPEKTAKARGQHLRTHFKNTREVAAALTGLKLSKAYKYLGDVQEHKDVIPFRRFNGGVGRAAQAKNHGTTQGRWPVKSIGFLLRLLKNAEANADAKSLDTEDLLIKHIVVQQAPKTRRRTYRAHGRINPYQGHPCHIEITLAVPDEQVARNKDVEVNQPKKIQGNKRQVAAQRRLTSA

SEQ ID NO: 155 - protein, 103 aa, metagenomes purified from environmentally challenged niches
MTGRGKGGKGLGKGGAKRHRKILRDNIQGITKPAIRRLARRGGVKRISAMIYEETRGVLKTFLEGVIRDAVTYTEHAKRKTVTSLDVVYALKRQGRTLYGFGG

SEQ ID NO: 156 - protein, 307 aa, metagenomes purified from environmentally challenged niches
MSLDVGDVDAWIDTLSQCKQLSESDVKLLCDKAREILIEESNVQPVRCPVTVCGDIHGQFHDLIELFRIGGNSPSTNYLFMGDYVDRGYYSVETVTLLVALKLRYRERITILRGNHESRQITQVYGFYDECLRKYGNANVWKFFTDLFDYLPLTALIDNQIFCLHGGLSPSIDTLDHIRSIDRIQEVPHEGPMCDLLWSDPDDRCGWGISPRGAGYTFGQDISEAFNHSNGLTLVARAHQLVMEGYNWSQDRNVVTLFSAPNYCYRCGNQAAIMEIDENLKYTFLQFDPAPRAGEPMVSRRVPDYFL

SEQ ID NO: 157 - protein, 103 aa, metagenomes purified from environmentally challenged niches; identical to SEQ ID NO: 155

SEQ ID NO: 158 - protein, 151 aa, metagenomes purified from environmentally challenged niches
GATTTSILHHFQLSTSSNNSFYHYYLNNLHQNDWTRQGRQGSRKGRRQASPQDLARQHPGHHQARHPPSGASWRCQAYLRHDLRGDPRCPQDLPRGCHPRRRHLHRARQAQDRHLPRRRLRPQEARPHPLRFRWLSSSLFSLRLLCFLQTQ

SEQ ID NO: 159 - protein, 146 aa, metagenomes purified from environmentally challenged niches
MFSKLIAIASLALAANAAVIDPSDHTVQYEAAPGKVVTEHYEVLSHAEASRIIEANPHISDYRYRCNYQCNDSSGNYMRNLQQGVPNQACIFSSCYDCDWKFQNCSYCRLSTGHNYRDIGGLESWCYNNGGTTVTHNCGYTDGDQC

SEQ ID NO: 160 - protein, 142 aa, metagenomes purified from environmentally challenged niches
MHFKSLFIAGALFMVGASAVDCATPEIHCETSDGSPWYDDAVQATEYWKEIQDAGKDSCGDAGCAQPHGSGCHSDGGSYGTAEIVLCQDDSSSSTPQCADCRCVYSYLKPLLDQCKGANNKIGGYAHVDMGGNYINYEFVKK

SEQ ID NO: 161 - protein, 100 aa, metagenomes purified from environmentally challenged niches
LLAPSSWSVPVPLIVPLLRFTARLVMAAPGTTMPSKPLNTGKKSRTPAKTAAVMLVAHSPMALDATATVVAMVPPRSFSARMTRPLQLPNVPTAGVSTAT

SEQ ID NO: 162 - protein, 185 aa, metagenomes purified from environmentally challenged niches
RAGGNWTMIDDLTTGSEDSFSNSWISWFLSTKGNEYFCEVDEEYILDRFNLTGLNNDVQNYSQALELITDSLDDEDLDDEQRDAIENSARYLYGLIHARYIITSRGLAKMLFLVYPQQLPSKTTNSVPSTKPATSADAAVGVDRYLPKIFGFPVHEMSKHARWQEAQRDLQISRLQQSASDPSYV

SEQ ID NO: 163 - protein, 415 aa, metagenomes purified from environmentally challenged niches
MSLTPEQTEIIKATVPVVKEHGKTITTVFYKNMLEAHPELNAIFNTTNQVNGHQPNALAGALFAYASNIDNLGALGPAVELICNKHASLYIQPEHYGIVGKFLLEAMGQVLGDALTPQILDAWAAAYWQLANLFIGRESAIYKQSEGWTQWREFRVAQKVPESAEITSFYLKPVDEKPLPRFRPGQYISVQVHVPQLECPQARQYSLSDKPRDDYYRISVKKETGLNTAKPEAKVNPGYVSNILHENVNEGDVIKVSHPCGDFFLTEQEPSHPVVLIAAGVGLTPLTSMLNTLDSTPADSQRKIHFIHGARTTSVRAFKDQIKSRAERLPNLQATFFTSSPSADEKQGVDYDVQGRIDVSKMDASKDLFLDNAQTEFYICGPTSFMNDIANSLKARGATSERIHMELFGTGGVPV

SEQ ID NO: 164 - protein, 212 aa, metagenomes purified from environmentally challenged niches
MAFMNLPWPTECLHAALKNGSLPFWGFVIYRTTYTAQSDAAWPQIIELIASYMKALLYHEYNDKKKDGDEPTVYDEIWARHQLTIMDDRQFNGASVFDIQLHFEKWVEAQGKRDESTMYRMCMVIDDESIQTLLEAPPGENRKLGRRIGGPVRFVKVVEAFPELDSLDEFQGWMKCEINALWPLWKMMSDGDEMRMSYDEMKGNGKQVYGAI

SEQ ID NO: 165 - protein, 222 aa, metagenomes purified from environmentally challenged niches
MARRPARCYRYCKNKPYPKSRFNRGVPDPKIRIFDLGRKKASVDDFPLCVHMVSNEYEQLSSEALEAARICANKYLVKIAGKEGFHLRVRAHPFHVVRINKMLSCAGADRLQTGMRGAFGKPNGVVARVNIGQILLSIRTRDSNRAAAVEAMRRSTYKFPGRQKIIISKNWGFTPVRREEYVKLRQEGKLKQDGAYVQFLRGHGLVEENMKRFPQAYEGVAQ

SEQ ID NO: 166 - protein, 252 aa, metagenomes purified from environmentally challenged niches
MSFYQSRPDTIKGPDPLTDNWTYDSAIDLFSWNPMMPDPFTFDLPDDLMKFESKDMSAGMVAPSDISGFAIGNHLGEDAASISDPESDDHPWSPSAHAAFPELSPITSTEQVHQETARYSTTPDATSPQEQPSSPPTRSTRRRSSADGPVRNAAKRAAHNVIEKRYRTNMNAKFVALEKAMNGGNGVQTSSRGGGSASLKKSEILSNAIAYMHGLQEENRYLQKELAIVKQNLVPAGIWRGAPSCKRETSYR

SEQ ID NO: 167 - protein, 254 aa, metagenomes purified from environmentally challenged niches
MGRVIRNQRKGRGSIFTAHTRLNKAPAQFRTLDFAERHGYTRGVVKEIIHDAGRGAPLAKVQFRHPYKFKMVTETFIANEGMYTGQFIYAGKNAQLTVGNVLPLASMPEGTVISNVEEKSGDRGALGRTSGNYVTVIGHNPEDGKTRVKLPSGAKKVIKNTARGMVGIVAGGGRTDKPLLKASRAKHKFAVKRNSWPKTRGVAMNPVDHPHGGGNHQHIGKASTISRYAAQGQKAGLIAARRTGLLRGTQKTKD

SEQ ID NO: 168 - protein, 249 aa, metagenomes purified from environmentally challenged niches
GAEAYYSPVSSLIGMSTGLRFSTLPAASNPQSSSLIPSPSAPISTFPYTLTLTLTPLTGSLSTSYSLRASPNLSFSSRFGFNVYSWESEMVAGFELWRQSKKPKLAAGSDGDDLEWARRKVRVWDPSAFPLAPPEPEIPQPNHEDESQESVLKLRVDQSWNVRLLWEGRVKELLVSAGVGLGPSSFSPSSYANPPGTAGAQGSGGGSPASYWRGVGGFGIIFFMRDFFGSMYLNEHCLDVYSLSDFMRQ

SEQ ID NO: 169 - protein, 211 aa, metagenomes purified from environmentally challenged niches
GPGVLSGFQPPDLPLITSIELDLDVVLPPPACRTMFLRTVSRAVPRSTAAIRAAPTASVNALQTRAASDHAIPNPTLANIEKRWEVMPPQEQAELWMQLRDRMKVDWHQMTLQEKKAAYYIAFGAHGPRAQPPKGEGMRVFAKVLQLTAASVAVFYAIHAFAGKQPATMSKEWQEASNEYALKEKINPIHGISKEGYEGKGFVQSPPAEKS

SEQ ID NO: 170 - protein, 153 aa, metagenomes purified from environmentally challenged niches
VARRGGIYLDGNNDLVTMKGNYIYHTSGRSPKVQGNTLLHAVNNYWHDNSGHAFEIGEGGYVLAEGNVFQDVTTPVEDPVDGQLFTSPDPSTNAQCSSYLGRACEINGFGNSGTFNQADTSLLSKFKGQNIASADAYSKVASSVASNAGQGHL

SEQ ID NO: 171 - protein, 120 aa, metagenomes purified from environmentally challenged niches
VRVVTFWPRVTSSRMLLPPLRTPLTASSSLPLTPAPTLSARHTLAGPAKSTASVTLVPSTRLTLACCLNLRVRTLLLLMLTLRLPRALPATPVRDTCKMERGGSELNLLMSDDIALAACW

SEQ ID NO: 172 - protein, 80 aa, metagenomes purified from environmentally challenged niches
MPSKTEAARLQNDFGADYWVRNTQERRHSTAGRGLFAGLQDVKHYNVDHGWARRKSSDNPGLLASFFSRFTGGSYHPPSE

SEQ ID NO: 173 - protein, 137 aa, metagenomes purified from environmentally challenged niches
VARRDSHHQIKSRLILLDITTIQHKVPSYFKQISTIESKCHPKPKQPVYKTTSAQTTGLEIPKNAATQPLAADYSPVSRMSSTITSTMAGPVASLAITPDSLLLSSVDSPGDHTIRPRNRIPFLNVRYWEECDLNWE

SEQ ID NO: 174 - protein, 181 aa, metagenomes purified from environmentally challenged niches
VVSTQSDEPTIPGGAAVTIHSRNEKKARKAIGKLGLKHVPGITRVTLRRPKNILFVVNQPDVYKSPSSNTWIIFGEAKIEDLNSQAQASAAQQLAAAEAAAGGEHAGHDHEHDILGKGKAPETEGKKEEEEDDGEEVDEAGLEAKDIDLVMAQANVSRKKAVKALRENDNDIVNSIMALSI

SEQ ID NO: 175 - protein, 191 aa, metagenomes purified from environmentally challenged niches
MFLQRTVSTLARRTPVRGLAAARPFSSSVSRFNKYEVKEAKLRSLDEIQTEEDLIPPGAKPGTVPSDIEHATGLERLELVGKMQGIDIFDLRPLDASRKGTLENPIVVNGAGDEQYAGCTGYPVDSHQVNWLTVSRERPIERCNECGNVVKLNYVGPEEDPHAHDHGHGHHPAPEEPKTFADYVKPEYWYR

SEQ ID NO: 176 - protein, 261 aa, metagenomes purified from environmentally challenged niches
MNPYIVDPMLKYVAFDIPALARLDPSLCLFLILFFENSRVVLLGYLPVPVLGLDVVGEGLGLLGGRVVAVAVVVSVRVLLRSDIVQLDNVTAFVAALDGALTRDSQPVNLVRVDGVTSATSVLLVTSTVDNNGVFEGSLAGSIQRPQVEDVNSLHFTDEFETLETSGVFDIARDGTGLSTRGDEVFFSLDLVKRTELGLLNLVLVESANGRRKRARGSKAPHGGAPREGRYRTLKEHSPCCNRTGRSNGRGEGGGGVDVGS

SEQ ID NO: 177 - protein, 221 aa, metagenomes purified from environmentally challenged niches
MADITAVGEENPSPTQDELQQAAAGNGAPDNRTPKRRMSDDEEDEEKQGRERRKIEIKFIQDKSRRHITFSKRKAGIMKKAYELSVLTGTQVLLLVVSETGLVYTFTTPKLQPLVTKAEGKNLIQACLNAPDPTTSENGVDAPEVPAETPEDVNHANVNAAAAQQTNIPRPTGMHPGYMTNEQQQQMAYYQNHLQQQQQAGGQYPGMSVGGRMPTQHQPTA

SEQ ID NO: 178 - protein, 176 aa, metagenomes purified from environmentally challenged niches
MSFAADPPPNNHGTLTHLFRAPEDLVYPIPENFSLEETVLVEPLSVAIHGARVAGITPGHTVLVQASGTIGLFCAATATAFGAKQVIISDINQTKLDFARDYLGCPIFLPNISSSHPEEEASRMKEYIESQRRCRYSSVVYGSGILVAKSGPGGVVVPNWTRFNRVQSNGTYHQYV

SEQ ID NO: 179 - protein, 86 aa, metagenomes purified from environmentally challenged niches
MPRGAEYANGPLQSDNAIEAGENKAHGTSGNTGLNRVNKVAEFPEGARGTGTAANPLSGQGSAGHQDGKGGHDPKTLGENKGLGTQ

SEQ ID NO: 180 - protein, 78 aa, metagenomes purified from environmentally challenged niches
MPSKLAKIRPTEPPVTPASTASTRSPNSPKAPEEPVPLLTRSVARVAPAIRMERVAMTRRPLERTRDWVLNDLMIQKT

SEQ ID NO: 181 - protein, 166 aa, metagenomes purified from environmentally challenged niches
MTTITEFPPFYTQQPNASALTQQLGLWQKHILSTCKQRRQFKLSVSDDIWANERIKRAASREFISVIISSLVTEGLASYTDATKEAVWVYWRSLSDWAQAAYAYAESTAQLNTPLTYYELVQGEYSHLSELHEMPVELLKLAVSLLVKQNKAVIIKTSQGEGVKFV

SEQ ID NO: 182 - protein, 130 aa, metagenomes purified from environmentally challenged niches
MSIPKAAAHTDKAPQPFKDLYSQAVIAGGVVYCSGIVAIDPETGSLIEGDVKAHTERILQSLSSTLQAAGTSLDRAVKINVYLANMEDFTSMNSVYEKYFVDGVKPCRTCVAVKSLPFGTDVEMECIAVL

SEQ ID NO: 183 - protein, 113 aa, metagenomes purified from environmentally challenged niches
MLRSQFGVISNAAKTAAFLKPVQTRLYASGALSKGDIQTRIFDVLKSFDKVKADNLTESASFTNDLGLDSLDAVEVVMAIEEEFAIEIPDAEADAIQNVNQAIEYIAKTPEAH

SEQ ID NO: 184 - protein, 200 aa, metagenomes purified from environmentally challenged niches
VVSTQSGAPGTKKVSSTYLSKICKEQHKSIFFYLIDLHSSASLRSVTTLPARMERIRLSEQAATICNQIREMIPETATLPNQPGKDQAELMHEDENGNKIYGGKLLTERAARLKEHMKIDQVSARFISQYFTNGIQDWTERLVYWTKPTKLLNQRKQGYIIPLSKDIVLQPGGPLEANNGFRVTNERILSSGAALFIMPQ

SEQ ID NO: 185 - protein, 524 aa, metagenomes purified from environmentally challenged niches
MLARSLQQIRRSSRLSLQLRAYASSPDRSASFSKLSEQDLPSLASIFSSPDTSLLTTLGDKPTATSDDLEPFNVDWMGKYKGHSSIIVKPKTTQEVSKVLQWCNERNVAVVPQGGNTGLVGGSVPLHDEVVLSLSSMNSIRHFDPLSGYVSVDSGIVLENLDNYLAQQGHIVPLDLGAKGSCQIGGNVATNAGGLRMLRYGSLHGNVLGLEVVLPDGRVINGMKGLKKDNTGIDLKQLFIGSEGVLGVITGVTLATPVRPSATNVAVFALPDYESVQTAFSSARRDLGEILSAFEFFDAASYKLVRSHGHAAERKTFEDGEDAPFFCLVETSGSNKDHDDEKLGAFLEQLMESGIVNDGVLAQDETQIGQLWSLREGIPEAAGKAGRVYKYDLSLPVEKMYSLVPELRQKLAEKGLLAAESEGGNGDGPVKTVFGFGHLGDGNLHINIVADAYRKEVEEVVEPYIYELVAKYNGSISAEHGLGLMKAPYVAYSQDAPSLDLMRTLKKTLDPKGILNPYKCVTAE

SEQ ID NO: 186 - protein, 185 aa, metagenomes purified from environmentally challenged niches
MALYYGIVFGILTFEIILFFLFLLPIPTRWQKPVFRWLATSPTIAHAQYIMKIVFVFIFVLFLDSVNTLRAFYEVVNTEDENGGIPAAGNSDFRAQVGQAAKKFYAQRNLYLTGFTILLLLILNKIKNMAMDYIRLEDQFIELEGSVSKDPAIRKASKEIDTTPIEDHVTRLEPVEQEQENKKDI

SEQ ID NO: 187 - protein, 138 aa, metagenomes purified from environmentally challenged niches
VARREAPNGHELPPRGYDPGENTYQAPPDERSQVDVAIDPKSNRLQLLKPFQKWDGKDITNVPILIKVQGKCTTDHISMAGPWLKYRGHLDNISNNFLIGAKSSEGKVNSIKNAFTGEYKGVQKQLVITRRKVFVGSW

SEQ ID NO: 188 - protein, 144 aa, metagenomes purified from environmentally challenged niches
GCPETARDYKKEGVRWVVVGDENYGEGSSREHAALEPRFLNGAAIITKSFARIHETNLKKQGMLPLTFADPKDYDKVDASDKVDILGLTDFQEGKPLTLRLHKKDGSTVDVPLNHTFNGQQIEWFKHGSALNLMKENTAKNGSL

SEQ ID NO: 189 - protein, 264 aa, metagenomes purified from environmentally challenged niches
VARREAPNGHELPPRGYDPGENTYQAPPDERSQVDVAIDPKSNRLQLLKPFQKWDGKDITNVPILIKVQGKCTTDHISMAGPWLKYRGHLDNISNNFLIGAKSSEGKVNSIKNAFTGEYKGVPETARDYKKEGVRWVVVGDENYGEGSSREHAALEPRFLNGAAIITKSFARIHETNLKKQGMLPLTFADPKDYDKVDASDKVDILGLTDFQEGKPLTLRLHKKDGSTVDVPLNHTFNGQQIEWFKHGSALNLMKENTAKNGSL

SEQ ID NO: 190 - protein, 195 aa, metagenomes purified from environmentally challenged niches
GAPLTQEHGFPVRVIVPGVAGARAVKWLDHITVQREMSSNHYMHFDYKVLPPEAVDAERARTFWHKVPPVIDMPANSAITSPRNEDTVEVDAEGFITVDGYALPGGEDGPVKRVEVSIDKERWVDAELFTHPMESKWTWKIWKAKVQVEPGERRCLYSRTTDEAGNSQPQRSQWNLRGVCYNGYGEVRNLKVVKG

SEQ ID NO: 191 - protein, 50 aa, metagenomes purified from environmentally challenged niches
MPANTMSATLRSLHVPGKPVIFANVWDTVSAKSIAPLDSCKALATASYAI

SEQ ID NO: 192 - protein, 373 aa, metagenomes purified from environmentally challenged niches
ALPMLLINPPRNLIGQSQSGTGKTAAFTLNMLSRVDPNIMTPQAICLAPSRELARQIQEVVDKIGQFTQIKSFLAVPGSWSRNVKIDKHILVGTPGTLVDMLSRGGRIFDPKQIRVFVLDEADEMIALQGLGDQTKRIKRMLPPGVQNVLFSATFPDNVRDFAGDFAPEANQIFLKKEEITVDAIKQLYLECDGEEQKYNALSALYDIMSIGQSIVFCKRKDTADRIAARLTDEGHSVASLHGDKQTRDRDDILDAFRDGKTKVLITTNVVARGIDIQQVNMVVNYDVPDLGPEGDWKPDIETYIHRIGRTGRFGRKGCSVIFAHDQRSMQDVQFIADTLGKKMSRINATRQTDLDQLEAALKAAIKGNQPKE

SEQ ID NO: 193 - protein, 274 aa, metagenomes purified from environmentally challenged niches
MATFSTRINLVPTSRTLASGVPFAPRIALVHPPASHGHGTSGPRSDVPPRWAGVQGGFASNSRVNVLPTGNFQQRFMSTTPARKIEAQPHVRGVPDWSAYQSSGKGENTRSLSYFMVGSLGVLAASGAKSTVSDILSNMAASADVLALAKIEVEMGAIPEGKNLIVKWRGKPVFIRHRTEDEINEARAVDIKSLRDPESDEDRTQRGEWLVMLGVCTHLGCVPIGEAGDYGGWFCPCHGSHYDISGRIRRGPAPLNLEVPEYAFNDDEEKLVIG

SEQ ID NO: 194 - protein, 472 aa, metagenomes purified from environmentally challenged niches
GEHHHSDRDCSSVKRVFALGRLDVTLAVECGSVRTMSLRDLACYTLTLKPSTENTLLTELTALEGPSEEPRFARVREKVEGEVYSSAIYDALTGAKLASVGFASEKQKNRRLQLHNPDESVPFDNTSKLGFEWTFIFEGNKYRWTRELYGKDYICSLDRKPDPRVEICLARDADSKAPGRLQILHYNIERFPNEIKDLRGLETLLIATLMCFVDAAEDRSNSGPTRTSPLPAKPVANAAAGQSGTSASGSSDTRAKVAPVTVPVITAEDFEDDCDPNEILVGTETDVGEHIARAIALLEDPTMLFIVIRTRTAAASSRALEVSLGVTRFRHREGMSELHQYVVEEDPVRKPKPIMPAQGLKLINLDDRPAAQSPTKPEWSAPPNIAVYLSSIELPDLTPKPKPVQGHTRPPTQAPHARPPPPSQLPQKPQPRPRPPPSDGSGSSQTTLASTRPPQDDGKDSRKSSFGRLFGR

SEQ ID NO: 195 - protein, 82 aa, metagenomes purified from environmentally challenged niches
MASQLMPLELIDRCIGSRMRVIMKGDKEFSGTLLGFDDFVNMVLEDVTEYDYTGATTKLPKILLNGNNICMLIPGGMPEGES

SEQ ID NO: 196 - protein, 116 aa, metagenomes purified from environmentally challenged niches
GDDNKKTIPHLNIFNNGVPIDAPGADRSLHRIKNACDHERRQRVQRHTSRIRRLRQYGARGCHRVRLHRRNDQASQDPSERQQHLHAHPRWHARGRVMNHGHMISLLTSLEMAKRV

SEQ ID NO: 197 - protein, 108 aa, metagenomes purified from environmentally challenged niches
AKELSPDVKPEPTWSCGEVVNVVDEHGNVIKPSDLWVKMGMQQQDNVDNLLIDDLCDQMRAKAKCTENGAQLNVDDLNHMMSYDKSYKQKRVDDLKDKYGWGAVFGPK

SEQ ID NO: 198 - protein, 38 aa, metagenomes purified from environmentally challenged niches
GSLTRRAWFIQSTCATTGDGLYEGLEWLADTLRKTNRD

SEQ ID NO: 199 - protein, 311 aa, metagenomes purified from environmentally challenged niches
MENLLRQMQGGGGRMGARPGPGGETILADNGETVHISSLALLKMLKHGRAGVPMEVMGLMLGEFVDDYTISCVDVFAMPQSGTTVTVESVDHVFQTKMLDMLKQTGRPEMVVGWYHSHPGFGCWLSSVDVNTQQSFEQLHPRAVAVVIDPIQSVRGKVVIDAFRSINPQSLVAGQESRQTTSNIGHLNKPSIQALIHGLNRHYYSLAIDYRKTEGEQGMLLNLHKRGWTEGLKMRDHSEMKEGNEKAIKEMLSLASAYTKSVQEETTMTAEQLKTRHVGKLDPKRHLGEAAEKAMGDQVTQSLAMGVLAEL

SEQ ID NO: 200 - protein, 213 aa, metagenomes purified from environmentally challenged niches
GHTGDVLSVSFSADNRQIVSASRDRTTKLWNTLGECKFNIVDDGHSEWVSCVRFSPNPVIPVIVSAGWDKVVKVWELSKCKLKTNHHGHTGYINTLAVSPDGSLAASGGKYGITMLWDLNDGKHLYSLEAGDIVNSLVFSPNRYWLCAATASSIKILDLESKSIVDDLKPDFSAEYPDKAQKPQCTSLAWSADGQTLFAGFSDNLVRVWVVTA

SEQ ID NO: 201 - protein, 76 aa, metagenomes purified from environmentally challenged niches
MVTRSGSLAFDSLLTPSFPSSSLLVGTRSSRSGNCPSASSRPTTTVTLVTSTPSPFRPTDRSPHPVESMASPCFGI

SEQ ID NO: 202 - protein, 99 aa, metagenomes purified from environmentally challenged niches
MLWDLNDGKHLYSLEAGDIVNSLVFSPNRYWLCAATASSIKILDLESKSIVDDLKPDFSAEYPDKAQKPQCTSLAWSADGQTLFAGFSDNLVRVWVVTA

SEQ ID NO: 203 - protein, 124 aa, metagenomes purified from environmentally challenged niches
VFAIVQIPKHGDAILSTGCGERSVGRNGEGVDVTSVTVVVGLELALGQFPDLDDLVPTSRDDDGNDGVRRESNARDPLRVTIVNNVELALSESVPELGSSVSGSRNDLSVVGRERDAQDVTGVS

SEQ ID NO: 204 - protein, 38 aa, metagenomes purified from environmentally challenged niches; identical to SEQ ID NO: 198

SEQ ID NO: 205 - protein, 393 aa, metagenomes purified from environmentally challenged niches
GRYDFKQPQRIRDASVTATPEWNLLEEIEFGRLGKLNLSVEEPEDLESHGTLQGYDKTFDRINTRTERPLEIIDRAWYNQTTSDDPVIAQLAQTQSAQIFATDAILAVLMCTTRSVNSWDIILERRGNQLFLDKRDSGPFDYVTVHENAADPPADSDDPNNVNSASSLSLEATYITRNFSSQVIDAKSKPYSPSPNPFYSEDEPSPVASCLYRYRKFDLSVGEEDTLDLIVRTEVDAYQGKKDSLVTVKALNEFDPRASGGGKALDWRKYLDTQKGAIVASEMKNNSAKLARWAIQSVLAGAEVMKMGYISRASPRDTTHHVIVGVQNYKPKDFAAQMNVSLNNGWGIVRTIADLVLKQPEGKYVLVKDPNAGIIRLYSVPENAFEAEEEEEQ

SEQ ID NO: 206 - protein, 106 aa, metagenomes purified from environmentally challenged niches
MTSSSLSEFETLLSRPRQNGTCLKRSSLADWASSTFPSKSPKTSNRTVPSKVTTRRLTASTLVPKDLSRSLIEHGTIKPLLTIPLLLSSLKRSLPKSSRQMPFLRF

SEQ ID NO: 207 - protein, 245 aa, metagenomes purified from environmentally challenged niches
ERSRSLAPEADQGVATQCHEVRSSGSYDTFEIGHHQPDSDTSGVADLRTSSRMDTCDAHLLRRVKSCPLFSYREDEVSETVQLPTGEWTTIRDITPSAPKIGFEVRDSLSAFPTAKPVEAKHESASSISNDLPSQPSSRPLIECPTLVADSRTTTGSNSVRSFDAQTERLSGLSDVHHRYMQDKPSQRSDSWTDVKSSAPSSQSMAVPNKAAYLAPIPAGPNDSKTSSSGRAPSDAATEHECSLQ

SEQ ID NO: 208 - protein, 148 aa, metagenomes purified from environmentally challenged niches
MAPKSTDKPASTAGKAPSAGGKAPASKTVGAKKTAAKKSAKSTGEGGEKKKRVKSRKETYSTYIYKVLKQVHPDTGISNKAMLILNSFVNDIFERIAGEASKLATYNKKSTISSREIQTAVRLILPGELSKHAISEGTKGVTKYSSSK

SEQ ID NO: 209 - protein, 369 aa, metagenomes purified from environmentally challenged niches
DVKRFTKDLLFNSEGNLTFKPHLWNDIRHTLLPTFIRQIGYVPIPRAEFSSPDIDLVIENLVLSGPNLFPNVVSLESHNSFKFSPYQQLNKGMDTHHHKFRLGMSQIQADIRDVRFSFRRKTGWPKLKDHGLADVILAGKGMSIDVELESVEGRRDSVVRVNHVHTTIDTLTFSIRDSKHDLLYKFVKSVATGTIKKAIQAAVDNAIRTAVGHLDDQLVQVRNTVDDAKKSDETTRTQALKDLYSKKADTAQKKQAESKEQPGTFRIVANRDSVLNPDMGGGKGAMTNKMWKTEDLAHSGKEWHSPAFDLLDSKHPARTGQTHPEAKEGAGHGNSLSSKAQPGANAADQLKATHGQSEAEAIAGQKRQQ

SEQ ID NO: 210 - protein, 173 aa, metagenomes purified from environmentally challenged niches
MSDSRSDERLDGPSSRTTVSPMSSLPVRVCRSTSSSSLSRDDETLLCESTTSTPPSTPSPSPSETPSTTCSTSSSSRWPRVRSRRQSRPPSTMPSVRLSVTSTTSSSRSETPSMTPRSLTRPPERKPSRTCTRRRRTRHRRSRPSPRSSLVLSESSPTETLFSTPTWAVARAP

SEQ ID NO: 211 - protein, 248 aa, metagenomes purified from environmentally challenged niches
MYTSAVTLLSLVLLLATSVIAQEQAGRPGTQRGGVFFGCYADRPTGNANQPITRVANSDTFFECMENCAAITSPSLLGYYQPSSGQCFCGNLLFNPQAQLNGNGCQGSDWSFGRTSTTFRRFGDACRPFGGVGFSANQYTTVTGPVACHVQCASNRFAYVWSDTGSNSWQCACSNNVRVQEDFQYTCQGGGVFVFEHSVQAQASSLNRKRTVEEQWAVPKDALCPFGMSACKVSGVDNAYEVCFFSDR

SEQ ID NO: 212 - protein, 116 aa, metagenomes purified from environmentally challenged niches
MFNAHQTDSPMSGPILEATHGNVLAATMSVFRRTSSTLVKVAVYLCLNIQYKLRLLRLTGSGRWRNNGLFRKTPSVHSECQRARYQVSIMLTRYASFQTARPLVPWPRGLKHAIDL

SEQ ID NO: 213 - protein, 271 aa, metagenomes purified from environmentally challenged niches
GGGTVVSNALLENAKLCKTQGKESSLRVIVCGRNRLENGSAPHWAEAFATHGKLVEVRMPQNGIRMEGIKAIADGLAKCPTLEVLDLQDNTATKTGTRSIVRHLSTWPKLRILNLSDCLLGSVGGIALATALSTGSNKHLEQLKLQYGEFDKRTVEILSTAISQHLPKLTTLELNGNRFDAEDECVETLKKALELHGNEDALDELDDMEEVDEDEEDDDDEDEEDEDEDKDTSADDGIDAGAAGEDALPPVTKKDEDVLADLLSKVHVQPS

SEQ ID NO: 214 - protein, 222 aa, metagenomes purified from environmentally challenged niches
LDRRSASTSSSFFVTGGRASSPAAPASIPSSALVSLSSSSSSSSSSSSSSSSSSTSSISSSSSKASSFPCSSSAFFRVSTHSSSASKRFPFSSSVVNFGKCWLIAVDSISTVLLSNSPYCSLSCSRCLFEPVDNAVARAIPPTEPKRQSERLSIRSLGQVERCRTILRVPVLVAVLSCKSSTSNVGHLASPSAIALMPSMRMPFCGILTSTNLPCVANASAQ

SEQ ID NO: 215 - protein, 176 aa, metagenomes purified from environmentally challenged niches
MVKLSNSLVRRLKWQHVRSLGVVALTAQLRGPQPQSAEDEDSEAAGKKLKLAGDQATSAVIPKSADKPDTFPLLDTLPATMAAGTRSMTRPLHVGDLRLADLRKIMQAAGHTAEFRGEGTLLIDKSVAVRKSGTGQIEIEASAQAAANQATPGRGASSFLAVKRKIYEGLAVVTGS

SEQ ID NO: 216 - protein, 139 aa, metagenomes purified from environmentally challenged niches
KMKIDVEKLNKDISLFPQVHPITEDMKITHKGVSRLVMLDRYSFKDTEKITLSEGDFVVLTIKEDPKFPARGLGYIKEIDWENKKAKVQVEEEFRHTLEKPEERETGIIVRSLDVIEKPLEIFYEQIAKRNATGLAAVE

SEQ ID NO: 217 - protein, 282 aa, metagenomes purified from environmentally challenged niches
GDATVTQLREIMDDPAGYFLPNLKHGADNMFYVGPRGLAQELEELFTFPSTILRKRQDTSQHDERQAKKARTQEDEAAGDALEEPETGRRDSVLPTERAAFGLEGDDSGFFLGDQTMGDDMLPMDDMGAMDTGVDQRRMRTPSVAPSVTESIARQIQNDRSAGTHPLAIFEKEARDDTQSQSQATPNKSVASESISKTSSGQSKNTGMAMGLLRREIEAIEEEDKMVGFDHLADKASKRAASAFFFELLVLGTKHAVKLEQAQAFGDIHIRGKDKLFAEVVA

SEQ ID NO: 218 - protein, 261 aa, metagenomes purified from environmentally challenged niches
MAPITCSTSVHADLHKSSRSFLPSQAQSSESARIPVSMTKGRQRRRARKRTKRLVTRWRSPRLGDATVCFRLNGPLLVSRVMTRAFSLATRRWETTCCLWTTWEPWTPEWTSDACEHHQSHRRSPNRSHVRFRMTEALAHTHWLYSRRRQGTTRSRNRRLRPTNRWPPSLSARLLLANQRILAWPWVCCEGRLRRSRRKTRWSGLITWQTRRPSEQRLHSSSSCWCLVPNMRSSLNKLRLSATSTYAAKTSCLQRLLHRQT

SEQ ID NO: 219 - protein, 108 aa, metagenomes purified from environmentally challenged niches
MGDHATTNDPSNATFEEKGKGKDVQDQIAEDSSDEESDQEPEMVDEEEDDNNLEPISQDNIISGGRRTRGKIIDYAAEAEKNKDEMEDSEDDEDYQGANDDEDDQMRD

SEQ ID NO: 220 - protein, 78 aa, metagenomes purified from environmentally challenged niches
ELKYFKAVALYNLSRYLDARKAINDLIQSYPDFRQAEALKSAIDDKVVRDGLIGVSVAGAVVAGVVGLAVALARGNRG

SEQ ID NO: 221 - protein, 27 aa, metagenomes purified from environmentally challenged niches
MGHVESRVNQRGPPRKAKYSWVTDSEK

SEQ ID NO: 222 - protein, 27 aa, metagenomes purified from environmentally challenged niches
MLKAPFFHRPCGGKGVQLKWATPDSAV

SEQ ID NO: 223 - protein, 177 aa, metagenomes purified from environmentally challenged niches
MPVRPYLEEMADMPVPLFAYDAPPTLADHPHAREHQHTTFMQYLARKQPDPKNYPNYPDVDIRDAINHYLIELECPGIKDAADIHCQWTSSRHLTVTGDIARPEESQIEAQIESRPVYLVLGERRIGSFRRNFTFPVEVEQENMTAKLEAGLLKIVLPKHKHHTPKGTGKVDIDVIE

SEQ ID NO: 224 - protein, 163 aa, metagenomes purified from environmentally challenged niches
MVLVLGQDNLQQSGLQLGSHIFLLDLHREGKVATERANASLSQNQVDGPALDLRFDLAFLRTGDVAGDGQVPRARPLAVDVGCVFDPRAFELDQVVIDGVADVHVRVVGVVLWVRLLARKVLHEGRVLVLAGVRVVGQGGRCVVREQGHGHVGHFFQVGSYGH

SEQ ID NO: 225 - protein, 118 aa, metagenomes purified from environmentally challenged niches
MFGFNFNTTKLLKTILVVCYLQATVLADPYTRVSWEAYMNHVNGSDDYRTQGDDTRATRFPETKPPKQGKDFLWSSKPVPSSDLFLEFFMYEGEPDEFSRTTESYQSLPSNALTARQK

SEQ ID NO: 226 - protein, 349 aa, metagenomes purified from environmentally challenged niches
MSPTPTSPHNKLSLPARASSHDSTDGIRKRVCKACDRCRLKKSKCDGSSPCSRCKADNAICVFGERKRSHDKHYPKGYVEMLEQQQGQLVSGLKEMYHRLQKASAWDGPVLDESTGQPLTHDILSALDLLEPKHDDSNEPEVFEENCEKLQSKLLADGAGFAHRRGSISSDSEHSHHDRPKTSSRHDTPVQPKPSIFKENLSFASAASSPLTQSPIPRSKPLNVMPYQTLQPSSRPSPLQMPSAYNDPQLYAPEWAQALADMSGDPNYRQRFSMQQQQQNDFDNLLWDPSAQAPMESPFSQPAFFNQAQLIGSGNVFGLSDINDLGPNPADGGMDFDFSKFVQQTEVMT

SEQ ID NO: 227 - protein, 149 aa, metagenomes purified from environmentally challenged niches
MSSFRVAAPKMASMAAQSSVKVARPAFQAAQLQKFTRAYSAVPKNTVFNTMKRTQMMARQASPIAKRAYSSEMANALVQVSQNIGMGSAAIGLAGAGVGIGLVFAALIQAVARNPSLRGQLFSYAILGFAFVEAIGLFDLMVAMMAKFL

SEQ ID NO: 228 - protein, 165 aa, metagenomes purified from environmentally challenged niches
MECTFLQELGHHGNHEVEETDGLDESETKNGVREKLATEGGVAGDGLDEGGEDETDTDTSTGKTDGGGTHTDVLGDLDEGVGHLRGVGTLGDGGGLAGHHLGALHGVEDGVLGDRGVGAGELLELSSLEGRAGDLHGGLSGHGGHLGGGDAEGRHCDDGEVVRWS

SEQ ID NO: 229 - protein, 425 aa, metagenomes purified from environmentally challenged niches
GGFSVKFRTAEGNWDFVANNTPVFFLRDPAKFPHFIHTQKRDPATHLSGDDDSTMFWDYLSQNPESIHQVMILMGDRGIPKGWRFMHGYYGHTLKIVNDKGEWVYAQFHLISDQGTQNFTGDEAAQQSNDYGQKDLYEAIEKGDFPSWTMKVQIMTEKQAEEAWEQKRINVFDLTHVWPHGDYPLRTVGKFTLNENAKNYFAEVEQVAFNPSHMIPGVEPSNDPVLQSRLFSYPDAHRHRIGANYQQLPVNQNVCPFALGNFQRDGQMAFYNQGSRPNYLSSIEPISFKERAYDLNKVHGKFVGEAVAFLSEIRPEDFNAPRALWQKVFSEESKQRFVDTVSGHMSTVRDKAITARMMTIFREVSPDLGDRLEKATGVKGESTIAGMKFNGTHNGFDKANKIPANGMKKGGEVIFDNGAPATAAR

SEQ ID NO: 230 - protein, 239 aa, metagenomes purified from environmentally challenged niches
VSVSIGVREQSRLQHWVVGRLDTGNHVRRVECDLFHLGEVVLGILVKGEFTDCSKWVITMRPDVGQIKDVDPLLLPCLLGLLLGHDLNLHRPRGEVSLLDGFVQILLSVIVGLLSSLVTREVLGALIRDEVELGVDPFALVIDNLEGVAVVAMHESPALGDTSITHEDHDLVDRLGVLRQVVPEHGRVIVTRQVGGGISLLGVDEVGELGRVSEEEDGGVVGHKVPISFCGPELDRESS

SEQ ID NO: 231 - protein, 368 aa, metagenomes purified from environmentally challenged niches
DTIDAEVLDSLGVTQENFQFALGVSNPSALREVAVVEVPNVRWEDIGGLEEVKRELIESVQYPVDHPEKFLKFGMSPSKGVLFYGPPGTGKTLLAKAVANECAANFISVKGPELLSMWFGESESNIRDIFDKARAAAPCVVFLDELDSIAKSRGGSQGDAGGASDRVVNQLLTEMDGMTSKKNVFVIGATNRPEQLDNALCRPGRLDTLVYVPLPDQEGRESILKAQLRKTPIADDIDLSYMASKTHGFSGADLGFITQRAVKLAIKQSIDLAIQNQKAREAEGDTAMDEDIEEDDPVPELTKAHFEEAMSMARRSVTDTEIRRYEAFAQSMKSSGGGSAFFRFPESGADGNAAEQQQNGAGEEDLYD

SEQ ID NO: 232 - protein, 317 aa, metagenomes purified from environmentally challenged niches
MHDCSLHLEYYSDNSKGLGREVRETNLVVEVLLASTILLLLGCVAIGTALREAEESAAATGALHALGESLVAPDLGVGDGATSHAHSLLKVSLGQLGHGVVLLDVLVHGGVTLGLSSLLVLDGQVNRLLDGQLDGTLGDEAKIGTRETVSLGGHVGKVDVVGDRSLAELGLENALTALLVRQGNVDESVETTRTAESVVELLRPVGGTDDENVLLAGHTVHLSEKLVDHTVGSTASIALRTATRLGDGVQLVEEDNARRGSTSLVEDVTNVALRLTEPHGEKLGTLDGNKVGRALVGDSLGQKSLTSTRGTVEKHTL

SEQ ID NO: 233 - protein, 166 aa, metagenomes purified from environmentally challenged niches
VSPKRTSSLPLASATPLPFARSQWSRFPTSDGRTLVVSRRSRGSSSRACNTPSTTPRSSSSLACPHQRVCFSTVPLVLVRLFWPRLSPTSARPTLFPSRVPSFSPCGSVSLRATFVTSSTRLVLPRLALSSSTSWTPSPSLVAVLRAMLAVLPTVWSTSFSLRWTV

SEQ ID NO: 234 - protein, 160 aa, metagenomes purified from environmentally challenged niches
MGHSAGLRKGTRYAFSRDFKKRGMIPLSTYLKQYKVGDIVHVVCNGAVQKGMPHKDFHGKTGVVYNVTKSAVGVILYKQVGNRYIEKRVNLRIEHVRLSRSREEFIVRVKTNAEKKRKAKEEGTTVFLKRQADKPREARTISAKDNKPESIAPIAYDTHI

SEQ ID NO: 235 - protein, 526 aa, metagenomes purified from environmentally challenged niches
DMGIGGLDTEFSAIFRRAFASRIFPPGLVEKLGIQHVKGILLFGPPGTGKTLMARQIGTMLNAREPKVVNGPEILNKFVGQSEENIRKLFADAEKEQKEKGDESGLHIIIFDELDAICKQRGSTNSGTGVGDSVVNQLLSKMDGVDQLNNVLIIGMTNRMDMIDEALLRPGRLEVHIEISLPDEAGRFQILNIHTNKMRTNGVMDSDVDLGELAALTKNFSGAEIGGLVKSATSFAFNRHVKVGSVAAFDDIDNMKISRADFLHALDEVTPAFGVSEEELQQVVQNGIIHYSQHVNDTLNDGSLLVEQVRKSDRTPLVSALLHGPSGAGKTALAATIAMASEFPFIKLISPETMVGFSEPQKIAQLNKVFTDSYKSPMSIIVVDSLERLLDWNPIGPRFSNGVLQALVVLFGKRPPKGRRLLILATTSNRNILTDMDVLSAFDTDIPINPISSIDAVVHVLDEVKLFPNSKEKQRATQMLREARLGEGGRPDLLVGVKKLLSMAEMARQDPDPTMKIVTSILREAS

SEQ ID NO: 236 - protein, 425 aa, metagenomes purified from environmentally challenged niches; identical to SEQ ID NO: 229

SEQ ID NO: 237 - protein, 122 aa, metagenomes purified from environmentally challenged niches
MLTDTESEPTISNCPLTRMCAPSPWATSSETARWHSTIKVVDPTTFLRLSQSHSRRGRMISTRSTANSSEKPSPSCLKSGQRTSMPQGHCGRKSLARKASSDSSTPSLVTCRQSETKPSPLE

SEQ ID NO: 238 - protein, 309 aa, metagenomes purified from environmentally challenged niches
MPPRQPATRLFALPPRFLCPSLPTTQTRTIRSIDKPAPKPSRFNASLNLPVLGSSSTAAFARKEHSLPLRTGALAIKKGMTALFDPVTAKRTPCTVLQLDRCQVVSHKRRDIHGYWAVQVGAGAKEARNVTRPERGHFAAYNVPLSRHLAEFRVKNAEGLPPVGSAITADLFIEGQFIDAKADRRGMGFEGGMKRWNFGGQPASHGNSLAHRLMGSSGGGQGSGSRVLPGKKMPGRMGGEQATVANLRVMQVDKENGIVVVSGAVPGPKNCMVKLQDALKKPWPDATWPPSIEGATEVLREATEKAPAA

SEQ ID NO: 239 - protein, 130 aa, metagenomes purified from environmentally challenged niches
MGIWDAFTDIVEAVTPWSVVEAEAPAEEPQEENESKTESKDEPEEEEEDEEEEEDEDDEEELVDPKETLEEECKNSPQCAPAKHHFDECVERVQQQESEGGAKEDCVEEFFHLAHCATACAAPKLWSQLK

SEQ ID NO: 240 - protein, 136 aa, metagenomes purified from environmentally challenged niches
MRKKRRMRMMRRSSSTPRRLSRKSARTLLNVPPPSTTSTSVLSAFSSRRARVVLRRTVSRSSSTLPTVRPLAPLPSFGLSSSKLTTLGYRLLRRRNGYIHVEKMPGAGTRQCCPLRKAVPLYECSSAGYQVGQRLL

SEQ ID NO: 241 - protein, 194 aa, metagenomes purified from environmentally challenged niches
GRYYRAPEIMLTWQKYDVAVDIWSTGCIFAEMLEGKPLFPGKDHVNQFSIITELLGTPPDDVIQTIASENTLRFVQSLPKREKVPFTTKFANADPLSLDLLEKMLVFDPRTRISASEGLSHEYLAPYHDPTDEPVAAEVFDWSFNDADLPVDTWKVMMYSEILDFHNLGDIQQDQAAEGPVTGDLAPPSATTSA

SEQ ID NO: 242 - protein, 134 aa, metagenomes purified from environmentally challenged niches
MSPSTFGAQDVSSPRCSRESPCSRARTTLISSRSSQNCSAHLLTMSSRPSHLRTPSDSSSRCPSVRRSHSLRNSPMPTRFRLTCWRRCLSSIHVPVSRHQKGCRTSTLRHTMTRRMSPSLPRCLTGVSTMRIYQ

SEQ ID NO: 243 - protein, 111 aa, metagenomes purified from environmentally challenged niches
GYPLNLSISISGGKETNRDCPSNGERSGKSSNLKAGPLGVRIVICRGCFGNGPHLSALERAVIEGENPVWDGVAAPVSSSFDESSCLGMQLKLGGKFHLKLNIGRRPIAHK

SEQ ID NO: 244 - protein, 41 aa, metagenomes purified from environmentally challenged niches
GLVAIARRPHPFPCQTRKLSVSAPKVVGGSPPVRIGRCQAK

SEQ ID NO: 245 - protein, 218 aa, metagenomes purified from environmentally challenged niches
MEPDQEESEEEEEEEDDEMDEDEDEGQQQDASGMQTPSGLATPSGYASTTSTMPGGMETPDFMDLRKQRQTRDETADQEDQGAPRDLYTVVPERRATASGFLGSDRAYDLSNAPQSSNMPVLGQEDSRKKKGGRSGADDVDLALDPAELEGMSEQELRQKYDSHRRSSSSQGAGGQQDKEDFSDFVAQEVAKKRQRAQQRGGSGRDRESSRSKEKFKF

SEQ ID NO: 246 - protein, 210 aa, metagenomes purified from environmentally challenged niches
MTRWMKMRMRASSRTPVACRHPLGSPRPQAMPLLHLQCLVAWRRLTLWTCASSDRRATRPLIKRTRVHRETSIRSCPSAEPPLLASSVLTAPMTCPMRHSLPTCLCWVKKTRARRKAADLVQTTSTWPWIQLSSRACLSKSLGRSTTRTGAPRPVKAPADSRTKKISQISSRKRSQRRGRGLSSAAAVDATAKALGARKSSSFRVYVCIV

SEQ ID NO: 247 - protein, 164 aa, metagenomes purified from environmentally challenged niches
GVIQVDEPALREGLPLRTGAARDAYVKWAVNAFKLSTAGVTDSTQVHSHFCYSEFQDFFHAIAALDTDVLSIENSKSDAKLLQVFVDQSFPAHIGPGVYDIHSPRVPSVDEIKERIEQMLQYLKPEQLWINPDCGLKTRTTEQTIGQLTSLVEAAKFYRQKYTQ

SEQ ID NO: 248 - protein, 125 aa, metagenomes purified from environmentally challenged niches
VRVFLCVLALPVMLMLSGLSMLSSCLLLVSPTAPRSTPTSATVNSRTSSTLLLPLIPMFCPSRTASPMPSSSRSSLIRVSPPTLDLVSTISTLLVFPPWMRSRSVSSRCSSTSSLSSSGSTLTAV

SEQ ID NO: 249 - protein, 171 aa, metagenomes purified from environmentally challenged niches
MLMRTELLSVLLAVELSSLDQRGQLADSLLSGTGLQTAVRVDPELLRLEVLEHLLDTLLDLIHGGNTRRVDIVDTRSNVGGETLINEDLEELGIGLAVLDGQNIGIKGSNSVEEVLEFTVAEVGVDLGAVGDTSSRQLESIDSPLNISITGSASTQRKTLTQGRLVDLDDP

SEQ ID NO: 250 - protein, 66 aa, metagenomes purified from environmentally challenged niches
LKSGVFGVRVVICRGCFWAATDLSSLEQDVIEGENPVCGRKGTLHVAPSTSRVVWECSSKWEVNFF

SEQ ID NO: 251 - protein, 189 aa, metagenomes purified from environmentally challenged niches
MKLSNSAHYSLFLLSSILGFSSASANSHLSDDSPCVARSPTSGLYYDLNAISLAPPEWKNGKKVDQEARDESWHAKGHDYPANFTINVCAPVLENVTNVVGVDASRWANVSAFYEQAGKIYSMGEQASEPFFRGRKLVLNYTDGSPCPGDSNTASGNSSIRTKSTLMSFLCDRAAEFPGLEKLGSTGSR

SEQ ID NO: 252 - protein, 393 aa, metagenomes purified from environmentally challenged niches
MNGFNEKGLDGDAFGEKSNLSGLKTFDAFPKTKTSYTTPTRRGGQWTVLILAVCTLFSLHELRTWWRGTEAHHFSVEKGVSHDLQLNLDMVVHMPCDTLRINIQDASGDRVLAGELLTREDTNWDLWMKKRNFESHGEHEYQTLNHEAADRLSAQDEDAHVHHVLGEVRRNPRRKFSKGPRLRWGDNKDSCRIYGSLEGNKVQGDFHITARGHGYMELAPHLDHEVFNFSHMITELSFGPHYPSLLNPLDKTIAESETHYQKFQYFLSVVPTLYSKGHNALDLVTTNKDNSVRYGRNTIFTNQYAATSQSTALPEIPTLIPGIFFKYNIEPILLLVSEERTGFLALVIRVINTVSGVLVTGGWIYQISGWIVEILGKRKRQSEGVLTGKHYSD

SEQ ID NO: 253 - protein, 292 aa, metagenomes purified from environmentally challenged niches
MFTRTLRPAVAVARTQAVQQQQAGMATLKEIDQRLKSVKNIGKITKSMKVVASTKLTRAEKAMREAKKYGAANNVLFEQTKAGEEEPKERKILYLAMTSDGGLCGGIHSNITRYMKKAVAKEPGMLAVVGDKPKAQLSRAMPKALTMSFNGVGKDVPTFVEASAIADEIMKSAGDFDEIRIVSNKYLSAIAYEPHTNAVISAEALRQAAGFQQYEMEEDVSKDLAEFALANAIYTALVEGHAAEISARRQAMENASNNANDMINSLQLQYNRGRQAVITTELIDIITGASAL

SEQ ID NO: 254 - protein, 317 aa, metagenomes purified from environmentally challenged niches
MSFAACHFCCFVHLVYTRLQSRGTGNDIDQLGGNDSLSTTVVLQLERVDHVVGVVGSVLHSLPPCRDLGGVSLDQGSVDGVGKSELGQVLGDILLHLVLLETGGLSECLSGDDGVGVRFVGDSGKVLVRDDSDLVKVTGRFHNLIGDSAGLDESGDILADAVERHGQSLGHRSRELSLGLVTDNSQHSGFLGHSLLHVSRNVGVDTTAQTTVGCHGEVEDLALLGLLLTSLGLLEQNVVGGTVLLGFTHGLLSSRQLGRGNDLHRLGDLPNVLDGFQTLVDFLQCGHTGLLLLDSLSPGDRHGRSESTREHGVERGE

SEQ ID NO: 255 - protein, 311 aa, metagenomes purified from environmentally challenged niches; identical to SEQ ID NO: 199

SEQ ID NO: 256 - protein, 93 aa, metagenomes purified from environmentally challenged niches
MGAIPEYDPEEPLETKPFKFVTAGYDARFPQQNQTKHCWQNYVDYYKCVEAKGEDFRPCKQFYHAFRSLCPKAWTDRWDTQREGGNFPAILNK

SEQ ID NO: 257 - protein, 252 aa, metagenomes purified from environmentally challenged niches
GPLLEELDVEAYAKKYRYLRFMCQETLDHLAFLKDKVKDVEGFWASTLLKHRDLRGYITSRSDKDALKYLTHIELVQDPKDPRPFALKFYFKENPYFSDLVLEKKYDMSEGSEPAPADGSITEGMRNFKEDELVTKATTINWKSDDKNLVAKQPRSKIPDNDDDEDFDGDVGSFFNYFTDDTDIFQIGALLQSELLPDAIDYFVGRGEQVDSEGEELDELEEDDEDDDEDDEGSIDLEDEEEQPSKKKPKRA

SEQ ID NO: 258 - protein, 165 aa, metagenomes purified from environmentally challenged niches
GSFLTPQHTHTPFGRAMHNALTVSRLNDKFQEPLVVLVELLRARVLHDRNFSNRQFSGGPSFGTDNQKRSMLLIFRTLSIIPLQFKAEHWSGPLSRELLVFNSFHKTLSRSLRTLVESITMNAFLKNNARRARDDYLDIALSLPFQNDTNTGFGIFFKVGGLAGV

SEQ ID NO: 259 - protein, 94 aa, metagenomes purified from environmentally challenged niches
QIYLDALTTFAEGNITEENKDSESVKEAKQSAMEILGDAIPNVKDPEAELLRGFRFWDAVLVCVRTLKADRAIDLKLAESFEAANSYLNMMRPN

SEQ ID NO: 260 - protein, 251 aa, metagenomes purified from environmentally challenged niches
GSFLTPQHTHTPFGRAMHNALTVSRLNDKFQEPLVVLVELLRARVLHDRNFSNRQFSGGPSFGTDNQKRSMLLIFRTLSIIPLQFKAEHWSGPLSRELLVFNSFHKTLSRSLRTLVESITMNAFLKNNARRARDDYLDIALSLPFQNDTNTGFGIFFKIYLDALTTFAEGNITEENKDSESVKEAKQSAMEILGDAIPNVKDPEAELLRGFRFWDAVLVCVRTLKADRAIDLKLAESFEAANSYLNMMRPN

SEQ ID NO: 261 - protein, 148 aa, metagenomes purified from environmentally challenged niches
GIYLDGNNDLVTMKGNYIYHTSGRSPKVQGNTLLHAVNNYWHDNSGHAFEIGEGGYVLAEGNVFQDVTTPVEDPVDGQLLTSPDPSTNAQCSSYLGRACEINGFGNSGTFNQADTSLLSKFKGQNIASADAYSKVASSVASNAGQGHL

SEQ ID NO: 262 - protein, 120 aa, metagenomes purified from environmentally challenged niches; identical to SEQ ID NO: 171

SEQ ID NO: 263 - protein, 160 aa, metagenomes purified from environmentally challenged niches
MSAQPLRIVMACDEAGVPYKDAIKAVLEKSPLVASVSDVGVNDASDKTAYPHPAVEGAQQIKAGKADRGLFICGTGLGVAIAANKVPGIRAVTAHDPFSVERSILSNDAQVLCMGQRVIGVELAKKLALDWLNYRFDPKSASAAKVQAISDYETKFAGSS

SEQ ID NO: 264 - protein, 150 aa, metagenomes purified from environmentally challenged niches
MSVTTTSSAAAASCTPSWQIPVDDVACAGQISGNITKVFDTCCKGNSPVKYNDDCNIYCLAQGQTKQELTDCLTEKSGNNQIFCGHGKQNATATAEATTTKETGTSTGTSTSSTGTSTETNAAVLNQPISKTGLGLVAMLFCSALVGVVA

SEQ ID NO: 265 - protein, 197 aa, metagenomes purified from environmentally challenged niches
AGVDRGVITKDEKDSSINRLLVTGYGLAEVMGTDGVNGIKTRTNHVMETCEVLGIEAARQTIYNEIQHTMTSHGMSIDPRHVMLLGDVMTYKGEVLGITRFGVQKMKDSVLMLASFEKTTDHLFDASLFSKKDEIQGVSECIIMGTPAPGCGTSLASIVTPAPLLPRKKPLLFETAFKAGQDRLSYHENNGGMEVDM

SEQ ID NO: 266 - protein, 249 aa, metagenomes purified from environmentally challenged niches
AGSGGAYSFSLTTFSPSGKLVQIEHALAAVAGGTTSLGIKATNGVVLATEKKSPSLLLDTSVLEKVAPICPNIGFVYSGMGPDFRVLVAKARKIAQAYYKVYGEYPPTKVLVQEVAGVMQKATQSGGVRPYGISLLIAGWDSHRGQSLYQVDPSGSYWAWKASAIGKNMVNGKTFLEKRYNDDLSLEDAIHTALLTLKEGFEGQMTENTIEIGVVTVPTAEQMQEKPGERLPPTFRKLTEQEVRDYLAL

SEQ ID NO: 267 - protein, 346 aa, metagenomes purified from environmentally challenged niches
MLTSAFSTSASKMLGKRAVSSSSALNGKVAVLGAAGGIGQPLSLLVKQNPAVSSLSLYDVRGSPGVAADISHINTPAVTEGFLPDNDGLKQALEGAEVVLIPAGVPRKPGMTRDDLFNTNASIVKMLAEASAKYCPKAMMLIIANPVNSTVPIVAETFKRAGVYDPARLFGVTTLDVVRSSTFVSGITGAKPSDTVVQVIGGHSGATIVPLLSQIPQGDKIVKAGGQQYADLVKRIQFGGDEVVKAKDGTGSATLSMAYAAAVFNDALLKAMDGQKGLVQPAYVESPHFAKEGAKYFASNVELGPNGVEKILDIGNMSSEEQELLKECLPQLAKNIAAGEKFVADN

SEQ ID NO: 268 - protein, 373 aa, metagenomes purified from environmentally challenged niches
MSLFLLFSLALIIIGSNVVGYPLVVSDELLTSSNVLGELGKALLKELLLLRGHVADVEDLLNTVGAELDVGGEVLSTLLGEVGALDVSGLNETLLAVHSLEESVVEDGSGVSHGEGSGASAVLGLDDFVTAKLDALDEVSVLLAASLDNLVALRDLGEQGHDGGARVTTDDLDHGVGGLGTGDARDESGRADNVEGGDTEETGRVVDTSTLEGLSDDRHGGVDGVGNDEHHSLGAVLGRSLSKHLDDGSVGVEKVVTGHAGLARNTSRNEDHLSTLEGLLEAIVVGEEALGDSRGVDVANVSSNTRGAANIVKGEAGDSRVLLDQQGEGLANTASSTEDGNLSVQGAGRRDCSLAEHLGSRCRKGAGQHFGSK

SEQ ID NO: 269 - protein, 435 aa, metagenomes purified from environmentally challenged niches
GASVLLPALHFDEREQRPGRTSSTASLLQRHDRNEPLSLNSHSPTSVDHTPTTAHFTGAEELLASDVGPTATAGLPGDAELESKLKLLEEVKRARESVHSSLERIRAGTPTPSISQGMPSPTPSGAPGYARTPSSVGLSDDVRSRRGSTTSSKVLDAIDKPRVATQSEWDEYVRNRHVISPPPTQFAVLPTSAAMVDRGTSRHSQYALVSDGVAKALDRRERTISMMEPQVAEDWGPRETLDSTPAHVSMGRRAMSFHEIPLASPVAASRPQDRSSYSAGPRQVIGSAAGHTQRPGISQSRSAHGRTMTYDELTERHRQRLSALQAPVSAKIREPMDIASAKASWDKQKRVERDEMKRREAEKLAQAHARERRGPAVDKKEVLKSTDEWRRSVHGGLDGFAVPHLPAHARGSTQPGGSGAKRSSLSQRPSNYFAN

SEQ ID NO: 270 - protein, 225 aa, metagenomes purified from environmentally challenged niches
GQACCFRHCISTSGSNDLDVRLRLQVCCSVTIAMNLYRSTRTRRHLWTTLPLLRISLVLKSCSPPTSDRPRQLGYPVMRSLRASSSCLKRSNVHGNRYIARSRGSEPARLPRLSARECPARHPLVPLVTLELRRLSACRTTCARDEAQRPAPRFLTLSTSLESLPNPNGTSTFATGMSSHLHPLSLPYCPHLLRWSIVVPVDTASMPLFPTALPKRLTGGSELFQ

SEQ ID NO: 271 - protein, 168 aa, metagenomes purified from environmentally challenged niches
MGSPAPHHRHQSSLEGVIDFSTGRGHPLNPYQRDKAESVFTGIINRFEDSSTVEKPYNRAKLVRLTYEYARSEDSRCNFLQAFFGSVNVTMDDSIDFDDEAVEEGIRSSLNSFADFLVENFFLPLKASASRTPPAPQPKFRADVLLWGLWKEWPRSDATASSAIDIVA

SEQ ID NO: 272 - protein, 253 aa, metagenomes purified from environmentally challenged niches
QDAPSPPAQVPSRRPAVGSVERVASLRRDCLIRDRHRCVISRNFDMKEAERRLDDSGYDHASDDEGHLLKDQEHGSFAELEVAHILPHSLMTTTANSELNKSKETALTILNMFDSGIVHLIDGPDIDRPRNALTLSIDLHRQFGNFKVFFEPMPEPHTYRIDSTLRQPFRNPIFPVTRALYLTPERTIDPPSGRLLAVHRAICHILHLSAAGNYIDSILRDMDDGTVQANGSTRLASIVRLKLGGWWDGTVVG

SEQ ID NO: 273 - protein, 106 aa, metagenomes purified from environmentally challenged niches
MVNIPKTRRTYCKGKECKKHTQHKVTQYKAGKASLFAQGKRRYDRKQSGYGGQTKPVFHKKAKTTKKVVLRLECTSCKTKAQLALKRCKHFELGGDKKTKGAALVF

SEQ ID NO: 274 - protein, 84 aa, metagenomes purified from environmentally challenged niches
MILEGSESKLRFSYDRPTRKDMSRHIMACAQHSSRVHQRCPTLPLRCVGCDSSTTAFQYHLFACRSEDDFTTVHITNRKCQQDQ

SEQ ID NO: 275 - protein, 41 aa, metagenomes purified from environmentally challenged niches
MKLTFKDLKQEKFVIEVEPSETVREVKQKLLKKKANMRRNE

SEQ ID NO: 276 - protein, 369 aa, metagenomes purified from environmentally challenged niches
GPEAGEVRNRGRALRDCSRSQAKIAQEKGEYEAERMKVIYSGKILQDDKTVESYNIQEKDFLVCLPSKGPKPAASSSASQAPATPAPRAPVATPAAPAPAAPAPASSTPAVPATPSPAGAQTGPSFGDPSALTMGSAAEGAVTQMEAMGFARSDIDRAMRAAFFNPDRAVDYLLNGIPADVQQEQQQRQQEQQADRAAEQAPVPSAEDAAAAAALGGDEGFNMFEAAAQAGDGRGGGARSGGSEALANLDFLRSNPHFQQLRQLVQQQPHMLEPILQQVAAGNPQISQIIGQNSEQFLQLLSEEGDEEDAALPPGTQAISVTEEERDAIERLCRLGFPRDSVIQAYFACDKNEELAANFLFDQPDDDEE

SEQ ID NO: 277 - protein, 375 aa, metagenomes purified from environmentally challenged niches
MKLTFKDLKQEKFVIEVEPSETVREVKQKIAQEKGEYEAERMKVIYSGKILQDDKTVESYNIQEKDFLVCLPSKGPKPAASSSASQAPATPAPRAPVATPAAPAPAAPAPASSTPAVPATPSPAGAQTGPSFGDPSALTMGSAAEGAVTQMEAMGFARSDIDRAMRAAFFNPDRAVDYLLNGIPADVQQEQQQRQQEQQADRAAEQAPVPSAEDAAAAAALGGDEGFNMFEAAAQAGDGRGGGARSGGSEALANLDFLRSNPHFQQLRQLVQQQPHMLEPILQQVAAGNPQISQIIGQNSEQFLQLLSEEGDEEDAALPPGTQAISVTEEERDAIERLCRLGFPRDSVIQAYFACDKNEELAANFLFDQPDDDEE

SEQ ID NO: 278 - protein, 342 aa, metagenomes purified from environmentally challenged niches
APGDMETADAKNRAMRAAGFIVPDTFEDLPEVLKTTYTGLVQKGVIVPKAEIDPPNIPMDYQWASKLGLIRKPAAFISTISDERGQELMYAGMRISDVFKEEIGIGGVISLLWFKRRLPPFACKFIEMVLQLTADHGPAVSGAMNTIITARAGKDLISSLAAGLLTIGDRFGGALDGAAAEFSRGLNSGATPREFVDSMRKANRLIPGIGHKIKSKTNPDLRVVLVVDYVKKHFPSHKTLDFALAVEDVTTQKSNTLILNVDGAIAASFCDLLSGCGAFTEDEAADYLKNGTLNGLFVLGRSIGFIGHYLDQRLLKQPLYRHPADDIFINMQERVVFQPGSN

SEQ ID NO: 279 - protein, 182 aa, metagenomes purified from environmentally challenged niches
GAYKEGKFTSESIQKSKLRFQDILVELPLRVHNSHLLTSFLHQVPQAPPAKNPLDFPSSLAELSRDSDVSSNPFAPNLDTLDLSIDPFQYWQRALGREQQKITAWQQKRKAENAARAASKQPPLDENEWQKLFKLPTEPSRLEALLVGRQVEQYARQVDGFSATVSAKMFGVRGNLLPNEIE

SEQ ID NO: 280 - protein, 171 aa, metagenomes purified from environmentally challenged niches
MSAPTPSHPTLTPWTSASTPSSTGSAPSAASSRRSPHGNRSARLRMLHAPRASSRPLTRMSGRSCSSCPRSPAGSRLCLSAGRSSSTPARSTDSPPPFPPRCLASGATSSLTRSSRGRILRRRDRRLCIARRSRLGGVEYMRHGYKKKDDVVPPSTSSGQRCIESQKKKGF

SEQ ID NO: 281 - protein, 217 aa, metagenomes purified from environmentally challenged niches
MRRSSKFKNVKILSSFGILCSVALNSSMAEPHHPFFCSHAACTLPHPAENASLCINAGPVSVIFVLYSISLGRRLPLTPNILAETVAENPSTWRAYCSTCLPTSRASSLLGSVGSLNSFCHSFSSRGGCLLAARAAFSALRFCCHAVIFCCSRPRARCQYWKGSMLRSRVSRLGAKGLELTSESRESSARDEGKSRGFFAGGACGTWCRKLVRRWEL

SEQ ID NO: 282 - protein, 150 aa, metagenomes purified from environmentally challenged niches
MYSTPPSRERLAMHKRRSRLRNIRPLLDLVREEVAPDAKHLGGNGGGESVDLAGVLLDLPADKQSLEPAGLRGQLEQLLPLILVKGRLLARGACSILSLALLLPCGDLLLLAAEGALPVLEGVDAEVQGVKVGCEGVGADIGVARKLCKG

SEQ ID NO: 283 - protein, 269 aa, metagenomes purified from environmentally challenged niches
MSNSFIRHLPSTLRAFRSSTAFSLTRSFSSTMASNGTSTNGVQHDARKVFFFDIDNCLYPKSYQIHDKMAVLIDNYFQNHLSLSQEDATTLHQRYYKDYGLAIEGLVRHHKVDPLEYNEKVDDALPLDDIIKPDPKLRKLLQDIDTDKVKLWLFTNAYVNHAKRVTRLLGVDDLFEGMTFCDYAAERLLCKPTTEMYNKAMQEANATDIDQCYFVDDSALNAAAAMKYGWKTAHLVEPTAKPPPQPVSQHQISNLEELRKVFPEVFKTS

SEQ ID NO: 284 - protein, 256 aa, metagenomes purified from environmentally challenged niches
MARIFITGSTDGLGLLSAKLLSEQGHSVFLHARNAERASQAKAAVPKAQGVIIGDLSNVSDVKQLAADANKAGPFDAVVHNAGLGLTTNGQKTAEGVAQIFAVNSMAPYILTALMDKPKRLLYVSSGLHFGGDPSLEDVTWATREFRPSDAYNDTKMQNVMLSKAVAKRWPDVQSGSLDPGWVKTKLGGSAAPGTTDAPAEMIAEYAAGKSCAGDQTGAYLTPRGVEEPHDATKLAEKQDRLMQIYKEVSGVSFPQ

SEQ ID NO: 285 - protein, 201 aa, metagenomes purified from environmentally challenged niches
MKLCLLGERNTRYLLVNLHQTILLLGQLSRIMRLFHATRSQVGTCLIACARFAGSVLSNHLCWSVGGARRGRPAELSLHPAWVKRAALHIRPAFGDCFREHDVLHLCIVVCIRWSELPCGPSDVLEAGVATEVQSGADVQEPLRLVHESGQNVRCHAVNGKNLGYALSSLLAIGGESEASIVNNGVKRSSLVGIGGELLHV

SEQ ID NO: 286 - protein, 192 aa, metagenomes purified from environmentally challenged niches
MAIGQSSQQQADGQNVVTQGNSDKAANPMRELRIQKLVLNISVGESGDRLTRAAKVLEQLSGQTPVYSKARYTVRTFGIRRNEKISVHVTVRGAKAEEILERGLKVKEYELRKRNFSATGNFGFGISEHIDLGIKYDPAIGIYGMDFYVVMSRPGERVARRRRAKTRVGASHKVNAPEVIKWYKNRFEGIVR

SEQ ID NO: 287 - protein, 213 aa, metagenomes purified from environmentally challenged niches
GHTGDVLSVSFSADNRQIVSASRDRTIKLWNTLGECKFNIVDDGHSEWVSCVRFSPNPVIPVIVSAGWDKVVKVWELSKCKLKTNHHGHTGYINTLAVSPDGSLAASGGKDGITMLWDLNDGKHLYSLEAGDIVNSLVFSPNRYWLCAATASSIKIFDLESKSIVDDLKPDFSAEYSDKAQKPQCTSLAWSADGQTLFAGFSDNLVRVWVVTA

SEQ ID NO: 288 - protein, 347 aa, metagenomes purified from environmentally challenged niches
MAPSTQKQWTVKNGEQDFDGLVYGDAPVPTAGDSEVVVKLHGASLNYRDLIIPKGKYPFPLSFPVVPGSDGAGEVVEVGSKVKQFKKGDKVVTLFNQLHQYGPVDAAAASSGLGGAVDGTLRQYGVFNENGVVRAPTNLNFLESSTLTCAGLTSWNALYGLKPLLPGQTVLVQGTGGVSIFALQFAKAAGATVIATTSSEEKGKRLKDLGADHVINYKTQTNWGEIARGLTRDNIGVDHIIEVGGAGTLEQSFKCIKFEGVISIIGFLGGMNPSTIPNVLQTLSNICTVRGVYVGSKALMNDMINAIEANNIHPVVDGTVFTLEKTREAYEYMWAQKHFGKLTIQIA

SEQ ID NO: 289 - protein, 518 aa, metagenomes purified from environmentally challenged niches
MLEQQYQMRKEQQVQFTPMASPSSTPYHMHQDFTVPGDFFSPLTSPALHAQNQPQSRQQFTAHQQGYYTNPSTAASSAAPSPIDANGDVEMGGDGVALPESASQPKKPSRRKPATPRTFAMNKVKQSPIQKPQKRKSVALAHKDADAVVQDAQRSGHIAPKSAGLQMPPPFESSENDSVSPEALNDLPMGPPPRPGSVSQSPAIAPQNQSVSGPAATPKSLLSMKGAQDMNAPASTGISGQMGQASLEDLELPEAAENPGSTATHSQVLNSQEPTPRLMPSRKTPKLGPLSTPSSGKPTSASNSPAHALSPMTASTPAGLLKDKKDNKGGRATSKKRGSVSTTNSAMVSPALRPKVSPSIKPLLPEGTSLNSPTHALLLASKSNYQNLLEGNHLPGISYPDSLSTGLTSKRTSHKVAEQGRRNRINDALKEMQALIPASSGARAEELMTADAGDDDSQETKEKDRDAAVKSNSSKAATVESANRYIRVLKESDAAQKDAIARPNSPGSRSLDPPDLDN

SEQ ID NO: 290 - protein, 126 aa, metagenomes purified from environmentally challenged niches
MRNILLVLASAALAVVAQKPDLDVKGTFGDANPFSKVVNGQSNKLYLTLDNHSPESLVVKSISGSWSEKTSASSGQEKFLKNSTTQEKLTVPIPPKSEGAFQPPTVLTYQFWSEFKPRELLLTVLG

SEQ ID NO: 291 - protein, 91 aa, metagenomes purified from environmentally challenged niches
MVLALVGGAGYLAYNIYFPPARKPRRSANTAPTDAPAAPADPDEWIPVHHKRAKKTSGGGATSGEESEATEGYASEKSASGAKKRGKGGRK

SEQ ID NO: 292 - protein, 252 aa, metagenomes purified from environmentally challenged niches
MSDNNDGNHGGGVGASYYYGGIAIALCLVIVLTLVSRILYRRRVRNRLLRANRQERITLRDRGEAPGLPTYRESRNQPSLPRYTAEADYAPPPGPPPSNSPDNEGHHFHFHFPSLHVPQALHLRPRQADDPADQIPTVPPPSYEPPKYEPPSGAPPEQQQEPVASGSSEHHHQQSALGEHTAAATAAATTPAEHSGESTELRSASPSQPQSQSQPQAPAQPQEQDYGYDDADFIHPEERRRIEAAQRNDPQT

SEQ ID NO: 293 - protein, 161 aa, metagenomes purified from environmentally challenged niches
MSRIGDPTNNPATQQLYSDRPLHLPGPGLKPSRQLTISSAVAFREDSGQTRFNLISSDHREVLHISIRARDNVLVLNTKAPDGDWGKEERHDLKPLFDTPLLPYITVMATKNSYILSVPGKREIIFNKRKGFMEPAVRIEYDYDEMSAFSDPCYITVPSSS

SEQ ID NO: 294 - protein, 84 aa, metagenomes purified from environmentally challenged niches
MPQEIKDIKNLLEIARRKDARSARIKKTKTVGAKGEPAQLTKFKIRCSRYLYTLVVSDGEKAEKLKQSLPPTLNVEEIGKVSKK

SEQ ID NO: 295 - protein, 173 aa, metagenomes purified from environmentally challenged niches
MSHTFYDGTIVVLQGILETFSHILHKAEESPNSSAFPAARLHEDMYPLTDQIRLATQFSEYILAKVTGREPRKFEGNPLTFAEFYERIDTMLKSLKEADKDVVNANADKEELTQVGPTAKIELSNAIYAHRIALPNIYFHLNIAYGILRKEGVPLGKLDYFAGFFPPSMAQGK

SEQ ID NO: 296 - protein, 162 aa, metagenomes purified from environmentally challenged niches
MSRIGDFANNNQATQQLFSDRPMQLPGPGLKPSRQLTVSSAMAFRWDSGQTRFNLISSDRREVLHISIRAKDDVLVLNTKAPDGNWGKEERHELKPLFDTPMLPYITVTATKTSYILSVPGNQEIIFNKRKGFMEPAVKIEYDYDENPAFSDPCYVTVPHLS

SEQ ID NO: 297 - protein, 313 aa, metagenomes purified from environmentally challenged niches
MSEQLHYKGSLAGHGNWVTAIATSAENPDMILTASRDKSVIVWQLTRDDAQYGYPKRILKGHNHFVSDVSISYDGQFALSSSWDKTLRLWDLNTGLTTRRFVGHEADVLSVSFSADNRQIVSGSRDRTIKLWNTLGECKFDIKDEGHSEWVSCVRFSPNPMNPVIVSAGWDKVVKVWELSNCKLKTNHYGHTGYINTVSVSPDGSLAASGGKDGITMLWDLNEGKHLYSLEAGDIVNALVFSPNRYWLCAATASCIKIFDLESKSIVDELKPDFVDVGKNSREPEAVSLSWSADGQTLFAGFTDNAVRVWTVA

SEQ ID NO: 298 - protein, 107 aa, metagenomes purified from environmentally challenged niches
GEGGGIHGTTFNSIMKCDVDVRKDLYGNIVMSGGTTMYPGIADRMQKEITALAPSSMKVKIIAPPERKYSVWIGGSILASLSTFQQMWISKQEYDESGPSIVHRKCF

SEQ ID NO: 299 - protein, 111 aa, metagenomes purified from environmentally challenged niches
MRLSLEALAVDDRRAALVVLLLRDPHLLEGGQRSQDGTTNPHRVFTLRRSNDLDLHRRRSKSGDFLLHTVGNTRVHSSTTRHDNVAIEILTDVNITLHDGVEGGSVDTTTF

SEQ ID NO: 300 - protein, 213 aa, metagenomes purified from environmentally challenged niches; identical to SEQ ID NO: 149

SEQ ID NO: 301 - protein, 161 aa, metagenomes purified from environmentally challenged niches; identical to SEQ ID NO: 293

SEQ ID NO: 302 - protein, 178 aa, metagenomes purified from environmentally challenged niches
MKAYWYDNQPGDQRLPHDSGRPVTESYLESIGVFYRHCPTIDLVDSLAAERGYKNRDEVCVSPQTMGDVYEEKVKTFFSEHLHEDEEIRYIRDGEGYFDVRGQEDEWVRIRLSKDDLIILPAGIYHRFTTDDKNYVKAMRLFQEEPKWTPLNRGPEVDVNPHRKTYLETVPSPAVAAN

SEQ ID NO: 303 - protein, 216 aa, metagenomes purified from environmentally challenged niches
VAAGYTPEALEILSKKKGGKYLVLEMDETYNPPAEETRTLYGVQLTQARNDAVISPQKTFNTIITPKNTESLPESALRDLTVATLALKYTQSNSVCYALNGQVVGLGAGQQSRIHCTRLAGDKTDNWWMRFHERVLNIKWKQGTKRADKSNAIDLLCSGQTPRNDAEKVEYERVFAEVPAPFTQEERDAWLSQLTNVAISSDAFVCLSPLLEHSKF

SEQ ID NO: 304 - protein, 51 aa, metagenomes purified from environmentally challenged niches
FPFIDNVFRAARSGVKYIAAPSGSQNDGPVFETAEKLGISFVEQGTRLFHH

SEQ ID NO: 305 - protein, 255 aa, metagenomes purified from environmentally challenged niches
VAAGYTPEALEILSKKKGGKYLVLEMDETYNPPAEETRTLYGVQLTQARNDAVISPQKTFNTIITPKNTESLPESALRDLTVATLALKYTQSNSVCYALNGQVVGLGAGQQSRIHCTRLAGDKTDNWWMRFHERVLNIKWKQGTKRADKSNAIDLLCSGQTPRNDAEKVEYERVFAEVPAPFTQEERDAWLSQLTNVAISSDAFFPFIDNVFRAARSGVKYIAAPSGSQNDGPVFETAEKLGISFVEQGTRLFHH

SEQ ID NO: 306 - protein, 316 aa, metagenomes purified from environmentally challenged niches
MCDRSRIGPKGWEAVVSTQAVVSTQAVVSTQAVVSTQAVVSTQAVVSTQSAQPGAISAPVAAGKDVELQWTEWPESHHGPVITYLANCNGDCSEVDKSSLEFFKIDQKGLIDDSNVPGTWATDKLISNNNSYTVTIPSDIAAGNYVLRHEIIALHSAGNEDGAQNYPQCLNLKVTGGGNASPSGTLGTKLYNEDDSGILVSIYQQLDSYDIPGPALYSGASSSSNSGSSSSVASATASATSAAASSPSSSQASGTPASQVKAQTASSTPSASSGATSGSLSDYFSSLSAEEFLNVISETLSWLVTDKIHARDLSTA

SEQ ID NO: 307 - protein, 138 aa, metagenomes purified from environmentally challenged niches
MKSLLCTPLATRMVPRTTPSVSTSRLLVVATLLPQVLLVPSSTTRTTRVSLSVSTSSLTPTTSPALLCTLALPRPPTLVLLPALLRPLLLPLLPLLPLPRPLRLPVPPLPRSRLRPLALLLALRPVPLPAVCPTTSAL

SEQ ID NO: 308 - protein, 272 aa, metagenomes purified from environmentally challenged niches
VVSTQSAQPGAISAPVAAGKDVELQWTEWPESHHGPVITYLANCNGDCSEVDKSSLEFFKIDQKGLIDDSNVPGTWATDKLISNNNSYTVTIPSDIAAGNYVLRHEIIALHSAGNEDGAQNYPQCLNLKVTGGGNASPSGTLGTKLYNEDDSGILVSIYQQLDSYDIPGPALYSGASSSSNSGSSSSVASATASATSAAASSPSSSQASGTPASQVKAQTASSTPSASSGATSGSLSDYFSSLSAEEFLNVISETLSWLVTDKIHARDLSTA

SEQ ID NO: 309 - protein, 138 aa, metagenomes purified from environmentally challenged niches; identical to SEQ ID NO: 307

SEQ ID NO: 310 - protein, 305 aa, metagenomes purified from environmentally challenged niches
MLSMFTRVARGQAKVFTRNASTASSKPTNQSSNKAATIAASISGVTAALYAHQYGLIDSVFASGLEEGLHAPHFPWSHNGWLDSFDHNSIRRGYQVYREVCSSCHSLDRIAWRNLVAVSHTSDEARAMAEEQEYTDGPNDQGESFQRPGKLADYMPAPYPNEEASRAANGGALPPDLSLIVKARHGGADYIMALLTGYQDPPAGIQVQEGMNFNPYFPGGGIAMGRVLFDGLVEYDDGTPATTTQMAKDVATFLSWASEPEHDDRKKMGFQAVIILSAMTAISLYVKRLKWSPIKTRKLTYNPPK

SEQ ID NO: 311 - protein, 165 aa, metagenomes purified from environmentally challenged niches
GGSPAKKSLIGAMEAQNLKTFPKQPIFQNSKTRGNKKVTKDRRWYKDVGLGFKTPQEAITGTYIDKKCPWTGEVSIRGRILSGKVVSTKMTRTIVIRREYLHYVPKYNRYEKRHKNLPVHASPAFRIENGDQVVVGQCRPLSKTVRFNVLRVIKNKAAAKAFAKF

SEQ ID NO: 312 - protein, 72 aa, metagenomes purified from environmentally challenged niches
MPPRKPRCSFKECKEQAQRIVGDCSFCSGHFCSKHRMLEAHSCSGLEDCKKESHARNADKLNSERTQVIKGV

SEQ ID NO: 313 - protein, 161 aa, metagenomes purified from environmentally challenged niches
MSRNFGDFSTNQATQQLYSDRPLHLPGNGLKPARQLTISSAVAFRWDSDQTRFNLISSDRREVLHISIRAKDNVLVLNTKAPDGDWGREERHELKKLFDTPMLPYITVTATKMTYNITVPSGQEIIFNKRKGFMEPAVKIEYDYDEHSAFSDPCYITVPSS

SEQ ID NO: 314 - protein, 119 aa, metagenomes purified from environmentally challenged niches
LLASNSRSNELSSPPSTHLHISQSTMVSKILFWSGFGIAVRLWQLGIEMRPILAKQGLWAYPVFAGVGGSFGYWLQGVEDRQLKILAQRREAILDKRRRRDEREGLSNIEKEGTLAATP

SEQ ID NO: 315 - protein, 91 aa, metagenomes purified from environmentally challenged niches
LNWSCNFADCWPRTPDRTNSPLLRQRTFTYRKAQWFPRFSSGVASASPSVSGNSVSKCVPFLPSRVSGPTPSSQVSVEASVTGSRVSRTVS

SEQ ID NO: 316 - protein, 182 aa, metagenomes purified from environmentally challenged niches
MIHAQQCNCRSFSEGSENKQQPTQQIMGSQPKYPPSQCCSDPHARPVSGACRGWLRGAAQESSADGPRHPGASNRSFHRHLRRRGRPRDPAWQEWDAFRYRVARDGRRCRSHSRRESWKPLCFAICEGALTEERRVRSIGSSRPAISEIAGPIQTPATKANTAGDNRESGESTPANKKFSAR

SEQ ID NO: 317 - protein, 127 aa, metagenomes purified from environmentally challenged niches
MPSNAIAGLSPKAVKINNSQRNKSWGRSQSTLLLNVAQTLTLVPSPALVEDGFAALRKNLQLTVLDTLEPVTEASTDTCEDGVGPETLLGKNGTHFDTELPETDGDAEATPEENLGNHCALRYVKVR

SEQ ID NO: 318 - protein, 300 aa, metagenomes purified from environmentally challenged niches
MPFIKEAKSNSYFSRYQVKYRRRREGKTDFYARKRLVTQAKNKYNAPKYRLVVRFTNKDIICQIVSSKLQGDVVLTHARARELPRYGIKHGLTSWSSAYAVGLLVARRALTKLGLADKYEGDVEATGEYNLTEPLGDDEPRPFKVFLDVGLKRTSTGSRVFGALKGASDGGLYIPHSENRFPGYDIESKELDAEILNKYILGGHIAEYMEALEEEDEERFKAQFSTYLEDGIGSEDIEEIFSGAHEAIRADPTFKPSEAAKGTDWKSESKKHRAVRLTKQQREDAIQQRIKYYQQAGDLE

SEQ ID NO: 319 - protein, 212 aa, metagenomes purified from environmentally challenged niches; identical to SEQ ID NO: 164

SEQ ID NO: 320 - protein, 192 aa, metagenomes purified from environmentally challenged niches
MTEKLYTEQVNAFGNELPPLSYKDLDKLPLHQNVIKETLRIHNSIHTLMRKVKNPLPVPGTRFVIPTSHTLLASPGVTTRDDSHFRNAMTWDPHRWETRSEVEDDGETIDYGYGVVSKGTKSPYLPFGAGRHRCIGEKFAYLNLTVIVATLVRNFRFSEPDDREGVPETDYSSLFSRPMRPATARWERRGEY

SEQ ID NO: 321 - protein, 210 aa, metagenomes purified from environmentally challenged niches
MAHWREEYLTALAVRDQREKANLSIYDAYTRLADSTAKLPATIDTSGSPSGDKGPSGTYESEKTAFSQSRTAKKQQTEVEPSVTELLNTTRAELAEAQRSRAELRDRLERATNEAEKLRKQIGKDGRRIHGLENEVAQQQKRRKDVEEELRGKAKLLNEFQDEIAALTLQVNMAERKAKKLGEENDDLVNRWMKRMGQEADAMNDASKFS

SEQ ID NO: 322 - DNA, 53 bp, Artificial Sequence
  poly-A mRNA primer
  misc_feature (52)..(53)
  misc_feature (52)..(52): a,c or g
  misc_feature (53)..(53): n is a, c, g, or t
attctagagcgatcgcacatgttttttttttttttttttttttttttttttvn

SEQ ID NO: 323 - DNA, 34 bp, Artificial Sequence
  poly-A mRNA primer
  Ribonucleotide Guanosine (32)..(33)
  LNA modification (34)..(34)
aagcagtggtatcaacgcagagtggcgcgccggg

SEQ ID NO: 324 - DNA, 34 bp, Artificial Sequence; identical to SEQ ID NO: 323
  oligo-capping rapid amplification of cDNA ends primers
  5' Inverted Dideoxy-T (1)..(1)
  Ribonucleotide (2)..(33)

SEQ ID NO: 325 - DNA, 33 bp, Artificial Sequence
  primer for amplification of prokaryote cDNA library
  5' Inverted Dideoxy-T (1)..(1)
  Ribonucleotide (2)..(33)
taagcagugguaucaacgcagaguggcgcgccg

SEQ ID NO: 326 - DNA, 20 bp, Artificial Sequence
  primer for CaMV 35S promoter
ccactgacgtaagggatgac

SEQ ID NO: 327 - DNA, 20 bp, Artificial Sequence
  primer for CBF3 promoter
cagcatgctctcactccaac

SEQ ID NO: 328 - DNA, 20 bp, Artificial Sequence
  primer for Erd10 promoter
cgtgagaatgacacaaccac

SEQ ID NO: 329 - DNA, 18 bp, Artificial Sequence
  primer for Kin1 promoter
ctcgtggcaccacactcc

SEQ ID NO: 330 - DNA, 19 bp, Artificial Sequence
  primer for NOS/HSP terminator
ggaaattcgcctcgagatc

SEQ ID NO: 331 - DNA, 1391 bp, Arabidopsis thaliana
ataccggagctcagagaatcatatgactaaggacgtggtggttgaaggaaatgagagaatacatgaagaagagaaacttctttgagtgagaaggaagtgcgctggctggagagaaaagagagaaaagagtttcgagtgagagagagggcgttgagattgtgatcaacttaatgtaatatgttcttttattacattttctttttgtcatatactcaaaccttttactattttgtctcataaatctaacacaccccaccatttgttaatgcatgatggtagaaaatattaaatataattaactacttttatgtgatcaaaattaggtttcagactcgtttcgcgatccgatctacaattacaactgcatgcttctaattgatctaaattctaaattttttatacatattaaaaaaacaactttttgttaaattctcaatcatcatttttgtgattaacaattttttataactctaaaccaataatatttgattatttattttatatgtataatgatgattgagaattttaattagcagtctatttagggttttcctaaagttacaatatgttgttacccttctagttaaattttccaaaataccatatttcataacttttcaaactgtttattaattcaaccgtaaaaagcactaaaatgttacatttgatcattcacccaaattaaattcaaaagtttttccgccaaaactacttggtgacttacgtgcttatatacggacgactattattatgttctatacttttttatactttgttgcacaaatatctactctcccaattcatattctagaaggatgtgctataagaatgggagaaattacacaagaagagcatctttaaatatcctctcacaatctttatgtctaatacacgggtgaacaattaacgacaatttctttattcaggaatataataatgaataacggttaccctacacctagtacactaaatccttaacagccacacattcatacgcaaagagtttataaaactcataaaggtataataataacgagtgaataagtcaaaaaaagtcttctctggacacatggcagatcttaatgagtgaatccttaaactactcattttacaattgcttcgctgtgtatagtttacgtggcattaccagagacacaaactccgtcttcgccttttcttttgcctctaaaatatcttccgccattataaaacagcatgctctcactccaacttttatttatctacaaacattaaatccacctgaactagaacagaaagagagagaaactattatttcagcaaaccataccaacaaaaaagacagagatcttttagttaccttatccagtttcttgaaacagagtactcttctgatcaggcgcgccgccata

SEQ ID NO: 332 - DNA, 1215 bp, Arabidopsis thaliana
ataccggagctcgactaggtggacaaaataatttgttaattaaataaaaattagttcaatatagaaatgaaaacgattgctttgtttggtatgtgtcggtacagtgaccatcctaatgcctaatataaaagattcgatcggtatgttacaagttgcgtgtatatgaaaacgtcacattttattaagtggcacgtcgttgtgatgaatctttcaaccgaacacgattcataatctataagcaaaatccgaaaatggtgccttctcaatgccccctatctgttcaatctttttttttttttttttttttgtatatctgttcaatcttatttaaatgtaatgacaaattaaatgaagtttacgttagtaatataagctgacaaacaacaccacattacatacataaaattaaattcttttaagtatttcaataacgtttctttatcttaaaaattaaatttacttcgagagcttcctacttcgtcaaaaataaaattttactttgctgcatgtttttactttctttttgtaacgtcttaaaaaggtgattaacgtcaacttaattcaccgaaagtctctgcaattgatattttctgccgacgtggcataagaagtccgattggcccacatgaccgacatccacgcttaaaccaatcaaaaccggccattcagttccatctgtgggctcctgaaacgttctcttgacacgtgtttaccatatattggcttaatccatccatagtctttctatttactgacaggtagtatttttcctatcaattatttattttcacgtggcatgatggctatggctagttgaacctgtgaataacttggtcatatctactctctatttatttagatgattcattttcttgaaggacttgcaattttatccccttacttttatttctttgagagataacctaaaattctcaaaatgagttggaaacatccctttgaagttcctctacaggctttctatgtgcataagaatctgcttaacattggaaataatatatgcattcttctccaattctcctagttggatacatatatgaagtctataaattacacatatttcccacaaaaattattgtaagagtttatatttcaacatatagtatgcaaacttaaatcgtgagaatgacacaaccactaattcaaaccactacattatatattctaatccattcaaattcatggcgcgccgccata

SEQ ID NO: 333 - DNA, 960 bp, Arabidopsis thaliana
ataccggagctcggtaacttgaattcaaccatgaactgtttggattggcaaacataaactcaaataaaatatctaggtataattgtggttcatacaagaattacttcatactgttgggccaaaggacgtatccttccccgcacctccaaaccatgggcttactactgatccgacatcaaaaccgtgttagttgcaaccaacgaatgataagtcaataagattcaacttgtcaacaaatatacagcttatatgacatgtctggctccaaactgaattttagtagaaagttactaattcataaaattaatttatatacaatttttcaatttttattttataaattaaagaaaaaaacatgaaaaatacgggaggttcggcaaacacaacatttaacttgccaaacgtatcatctaactttcccaccttatacaaggaaccattttttcaataataaagtttttttttttttgtcttcgcaaataagagcacgaaatgtttgccaaacgcatatgcaacaaacccacgttacataattctgtttacagccatagagcaagctatattgttaaagacctaaaaaaaactttactataacatatagaggcttcgagatatttcgaaagactcaacttatatataaataaactcaaaaagaaaacacggaggcgagaggatcatactctcacacagaaagagtcacattattatatcctctaaaaaaccaaactaaaacgacacgtgaagtcttgatcagccgataaatagctaccgacataaggcaaaactgatcgtaccatcaaatgtaatccacgtggttttagattactcgtggcaccacactccctttagcctataaatataaaccattaagcccacatctcttctcatcatcactaaccaaaacacacttcaaaaacgattttacaagaaataaatatctgaaaaaggcgcgccgccata